European Patent Application EP 4 483 899 A1, published January 1, 2025. Title: 抗変異ＣＡＬＲ抗体と他の薬剤とを組み合わせてなる医薬. Applicant: 学校法人順天堂. The sequence listing filed with the application follows.

SEQUENCE LISTING (228 sequences)

SEQ ID NO: 1 - protein, 55 aa, Homo sapiens
EEQRLKEEEEDKKRKEEEEAEDKEDDEDKDEDEEDEEDKEEDEEEDVPGQAKDEL

SEQ ID NO: 2 - protein, 49 aa, Homo sapiens
EEQRTRRMMRTKMRMRRMRRTRRKMRRKMSPARPRTSCREACLQGWTEA

SEQ ID NO: 3 - protein, 68 aa, Homo sapiens
EEQRLKEEEEDKKRKEEEEAEDNCRRMMRTKMRMRRMRRTRRKMRRKMSPARPRTSCREACLQGWTEA

SEQ ID NO: 4 - protein, 13 aa, Homo sapiens
RRMMRTKMRMRRM

SEQ ID NO: 5 - protein, 31 aa, Homo sapiens
RRTRRKMRRKMSPARPRTSCREACLQGWTEA

SEQ ID NO: 6 - protein, 119 aa, Rattus norvegicus
QVQLQQSGAELVKPGSSVKISCKASGYTFTRNFIHWIKQQPGNGLEWIGWIFPGDGDTEYNQKFNGKATLTADKSSSTAYMQLSSLTSEDSAVYFCARGNYNYEYFDYWGQGVMVTVSS

SEQ ID NO: 7 - protein, 107 aa, Rattus norvegicus
DIQMTQSPASLSASLGETVSIECLASEDIYSYLAWYQQKPGKSPQLLIFAANRLQDGVPSRFSGSGSGTQFSLKISGMQPEDEGDYFCLQGSKFPYTFGPGTKLELN

SEQ ID NO: 8 - protein, 121 aa, Rattus norvegicus
QVQLQQSGAELVKPGSSVKISCKASGYTFTSYFVHWIKQQPGDGLEWIGWIYPGDGDTEYNHKFNGKSTLTADRSSSTAYMQLSSLTSEDSAVYFCARGNYYDGREVMDAWGQGASVTVSS

SEQ ID NO: 9 - protein, 112 aa, Rattus norvegicus
DVVLTQTPPTLSATIGQSVSISCRSSQSLLDSDGETYLNWLLQRPGQSPQLLIYSVSNLESGVPNRFSGSGSETDFTLKISGMEAEDLGVYYCMQATHGPYTFGAGTKLELK

SEQ ID NO: 10 - protein, 121 aa, Rattus norvegicus
QVQLQQSGAELVKPGSSVKISCKASGYTFTSYFVHWIKQQPGDGLEWIGWIYPGDGDTEYNQKFNGKATLTADRSSSTAYMQLSSLTSEDSAVYFCARGNYYDGREVMDAWGQGASVTVSS

SEQ ID NO: 11 - protein, 112 aa, Rattus norvegicus
DVVLTQTPPTLSATIGQSVSISCRSSQSLLDSDGETYLNWLLQRPGQCPQLLIYSVSNLESGVPNRFSGSGSETDFTLKISGVEAEDLGVYYCMQGTHGPYTFGAGTKLELK

SEQ ID NO: 12 - protein, 119 aa, synthetic construct
QVQLVQSGGGVVQPGRSLRLSCKASGYTFTRYTMHWVRQAPGKGLEWIGYINPSRGYTNYNQKVKDRFTISRDNSKNTAFLQMDSLRPEDTGVYFCARYYDDHYSLDYWGQGTPVTVSS

SEQ ID NO: 13 - protein, 107 aa, synthetic construct
DIQMTQSPSSLSASVGDRVTITCSASSSVSYMNWYQQTPGKAPKRWIYDTSKLASGVPSRFSGSGSGTDYTFTISSLQPEDIATYYCQQWSSNPFTFGQGTKLQITR

SEQ ID NO: 14 - protein, 10 aa, Rattus norvegicus
GYTFTRNFIH

SEQ ID NO: 15 - protein, 17 aa, Rattus norvegicus
WIFPGDGDTEYNQKFNG

SEQ ID NO: 16 - protein, 10 aa, Rattus norvegicus
GNYNYEYFDY

SEQ ID NO: 17 - protein, 11 aa, Rattus norvegicus
LASEDIYSYLA

SEQ ID NO: 18 - protein, 7 aa, Rattus norvegicus
AANRLQD

SEQ ID NO: 19 - protein, 9 aa, Rattus norvegicus
LQGSKFPYT

SEQ ID NO: 20 - protein, 10 aa, Rattus norvegicus
GYTFTSYFVH

SEQ ID NO: 21 - protein, 17 aa, Rattus norvegicus
WIYPGDGDTEYNHKFNG

SEQ ID NO: 22 - protein, 12 aa, Rattus norvegicus
GNYYDGREVMDA

SEQ ID NO: 23 - protein, 16 aa, Rattus norvegicus
RSSQSLLDSDGETYLN

SEQ ID NO: 24 - protein, 7 aa, Rattus norvegicus
SVSNLES

SEQ ID NO: 25 - protein, 9 aa, Rattus norvegicus
MQATHGPYT

SEQ ID NO: 26 - protein, 10 aa, Rattus norvegicus
GYTFTSYFVH

SEQ ID NO: 27 - protein, 17 aa, Rattus norvegicus
WIYPGDGDTEYNQKFNG

SEQ ID NO: 28 - protein, 12 aa, Rattus norvegicus
GNYYDGREVMDA

SEQ ID NO: 29 - protein, 16 aa, Rattus norvegicus
RSSQSLLDSDGETYLN

SEQ ID NO: 30 - protein, 7 aa, Rattus norvegicus
SVSNLES

SEQ ID NO: 31 - protein, 9 aa, Rattus norvegicus
MQGTHGPYT

SEQ ID NO: 32 - protein, 5 aa, Mus musculus
RYTMH

SEQ ID NO: 33 - protein, 17 aa, Mus musculus
YINPSRGYTNYNQKVKD

SEQ ID NO: 34 - protein, 10 aa, Mus musculus
YYDDHYSLDY

SEQ ID NO: 35 - protein, 10 aa, Mus musculus
SASSSVSYMN

SEQ ID NO: 36 - protein, 7 aa, Mus musculus
DTSKLAS

SEQ ID NO: 37 - protein, 9 aa, Mus musculus
QQWSSNPFT

SEQ ID NO: 38 - protein, 714 aa, synthetic construct
QVQLQQSGAELVKPGSSVKISCKASGYTFTRNFIHWIKQQPGNGLEWIGWIFPGDGDTEYNQKFNGKATLTADKSSSTAYMQLSSLTSEDSAVYFCARGNYNYEYFDYWGQGVMVTVSSGGGGSGGGGSGGGGSDIQMTQSPASLSASLGETVSIECLASEDIYSYLAWYQQKPGKSPQLLIFAANRLQDGVPSRFSGSGSGTQFSLKISGMQPEDEGDYFCLQGSKFPYTFGPGTKLELNGGGGSQVQLVQSGGGVVQPGRSLRLSCKASGYTFTRYTMHWVRQAPGKGLEWIGYINPSRGYTNYNQKVKDRFTISRDNSKNTAFLQMDSLRPEDTGVYFCARYYDDHYSLDYWGQGTPVTVSSGGGGSGGGGSGGGGSDIQMTQSPSSLSASVGDRVTITCSASSSVSYMNWYQQTPGKAPKRWIYDTSKLASGVPSRFSGSGSGTDYTFTISSLQPEDIATYYCQQWSSNPFTFGQGTKLQITRDKTHTCPPCPAPEAAGGPSVFLFPPKPKDTLMISRTPEVTCVVVDVSHEDPEVKFNWYVDGVEVHNAKTKPREEQYNSTYRVVSVLTVLHQDWLNGKEYKCKVSNKALPAPIEKTISKAKGQPREPQVYTLPPSRDELTKNQVSLTCLVKGFYPSDIAVEWESNGQPENNYKTTPPVLDSDGSFFLYSKLTVDKSRWQQGNVFSCSVMHEALHNHYTQKSLSLSPGK

SEQ ID NO: 39 - protein, 722 aa, synthetic construct
DIQMTQSPASLSASLGETVSIECLASEDIYSYLAWYQQKPGKSPQLLIFAANRLQDGVPSRFSGSGSGTQFSLKISGMQPEDEGDYFCLQGSKFPYTFGPGTKLELNGGGGSGGGGSGGGGSQVQLQQSGAELVKPGSSVKISCKASGYTFTRNFIHWIKQQPGNGLEWIGWIFPGDGDTEYNQKFNGKATLTADKSSSTAYMQLSSLTSEDSAVYFCARGNYNYEYFDYWGQGVMVTVSSGGGGSQVQLVQSGGGVVQPGRSLRLSCKASGYTFTRYTMHWVRQAPGKGLEWIGYINPSRGYTNYNQKVKDRFTISRDNSKNTAFLQMDSLRPEDTGVYFCARYYDDHYSLDYWGQGTPVTVSSGGGGSGGGGSGGGGSDIQMTQSPSSLSASVGDRVTITCSASSSVSYMNWYQQTPGKAPKRWIYDTSKLASGVPSRFSGSGSGTDYTFTISSLQPEDIATYYCQQWSSNPFTFGQGTKLQITRLEVLFQGPDKTHTCPPCPAPELLGGPSVFLFPPKPKDTLMISRTPEVTCVVVDVSHEDPEVKFNWYVDGVEVHNAKTKPREEQYNSTYRVVSVLTVLHQDWLNGKEYKCKVSNKALPAPIEKTISKAKGQPREPQVYTLPPSRDELTKNQVSLTCLVKGFYPSDIAVEWESNGQPENNYKTTPPVLDSDGSFFLYSKLTVDKSRWQQGNVFSCSVMHEALHNHYTQKSLSLSPGK

SEQ ID NO: 40 - protein, 714 aa, synthetic construct
QVQLVQSGGGVVQPGRSLRLSCKASGYTFTRYTMHWVRQAPGKGLEWIGYINPSRGYTNYNQKVKDRFTISRDNSKNTAFLQMDSLRPEDTGVYFCARYYDDHYSLDYWGQGTPVTVSSGGGGSGGGGSGGGGSDIQMTQSPSSLSASVGDRVTITCSASSSVSYMNWYQQTPGKAPKRWIYDTSKLASGVPSRFSGSGSGTDYTFTISSLQPEDIATYYCQQWSSNPFTFGQGTKLQITRGGGGSQVQLQQSGAELVKPGSSVKISCKASGYTFTRNFIHWIKQQPGNGLEWIGWIFPGDGDTEYNQKFNGKATLTADKSSSTAYMQLSSLTSEDSAVYFCARGNYNYEYFDYWGQGVMVTVSSGGGGSGGGGSGGGGSDIQMTQSPASLSASLGETVSIECLASEDIYSYLAWYQQKPGKSPQLLIFAANRLQDGVPSRFSGSGSGTQFSLKISGMQPEDEGDYFCLQGSKFPYTFGPGTKLELNDKTHTCPPCPAPEAAGGPSVFLFPPKPKDTLMISRTPEVTCVVVDVSHEDPEVKFNWYVDGVEVHNAKTKPREEQYNSTYRVVSVLTVLHQDWLNGKEYKCKVSNKALPAPIEKTISKAKGQPREPQVYTLPPSRDELTKNQVSLTCLVKGFYPSDIAVEWESNGQPENNYKTTPPVLDSDGSFFLYSKLTVDKSRWQQGNVFSCSVMHEALHNHYTQKSLSLSPGK

SEQ ID NO: 41 - protein, 714 aa, synthetic construct
QVQLVQSGGGVVQPGRSLRLSCKASGYTFTRYTMHWVRQAPGKGLEWIGYINPSRGYTNYNQKVKDRFTISRDNSKNTAFLQMDSLRPEDTGVYFCARYYDDHYSLDYWGQGTPVTVSSGGGGSGGGGSGGGGSDIQMTQSPSSLSASVGDRVTITCSASSSVSYMNWYQQTPGKAPKRWIYDTSKLASGVPSRFSGSGSGTDYTFTISSLQPEDIATYYCQQWSSNPFTFGQGTKLQITRGGGGSDIQMTQSPASLSASLGETVSIECLASEDIYSYLAWYQQKPGKSPQLLIFAANRLQDGVPSRFSGSGSGTQFSLKISGMQPEDEGDYFCLQGSKFPYTFGPGTKLELNGGGGSGGGGSGGGGSQVQLQQSGAELVKPGSSVKISCKASGYTFTRNFIHWIKQQPGNGLEWIGWIFPGDGDTEYNQKFNGKATLTADKSSSTAYMQLSSLTSEDSAVYFCARGNYNYEYFDYWGQGVMVTVSSDKTHTCPPCPAPEAAGGPSVFLFPPKPKDTLMISRTPEVTCVVVDVSHEDPEVKFNWYVDGVEVHNAKTKPREEQYNSTYRVVSVLTVLHQDWLNGKEYKCKVSNKALPAPIEKTISKAKGQPREPQVYTLPPSRDELTKNQVSLTCLVKGFYPSDIAVEWESNGQPENNYKTTPPVLDSDGSFFLYSKLTVDKSRWQQGNVFSCSVMHEALHNHYTQKSLSLSPGK

SEQ ID NO: 42 - protein, 717 aa, synthetic construct
QVQLVQSGGGVVQPGRSLRLSCKASGYTFTRYTMHWVRQAPGKGLEWIGYINPSRGYTNYNQKVKDRFTISRDNSKNTAFLQMDSLRPEDTGVYFCARYYDDHYSLDYWGQGTPVTVSSGGGGSDIQMTQSPASLSASLGETVSIECLASEDIYSYLAWYQQKPGKSPQLLIFAANRLQDGVPSRFSGSGSGTQFSLKISGMQPEDEGDYFCLQGSKFPYTFGPGTKLELNGGGGSGGGGSGGGGSGGGGSQVQLQQSGAELVKPGSSVKISCKASGYTFTRNFIHWIKQQPGNGLEWIGWIFPGDGDTEYNQKFNGKATLTADKSSSTAYMQLSSLTSEDSAVYFCARGNYNYEYFDYWGQGVMVTVSSGGGGSDIQMTQSPSSLSASVGDRVTITCSASSSVSYMNWYQQTPGKAPKRWIYDTSKLASGVPSRFSGSGSGTDYTFTISSLQPEDIATYYCQQWSSNPFTFGQGTKLQITRLEVLFQGPDKTHTCPPCPAPEAAGGPSVFLFPPKPKDTLMISRTPEVTCVVVDVSHEDPEVKFNWYVDGVEVHNAKTKPREEQYNSTYRVVSVLTVLHQDWLNGKEYKCKVSNKALPAPIEKTISKAKGQPREPQVYTLPPSRDELTKNQVSLTCLVKGFYPSDIAVEWESNGQPENNYKTTPPVLDSDGSFFLYSKLTVDKSRWQQGNVFSCSVMHEALHNHYTQKSLSLSPGK

SEQ ID NO: 43 - protein, 709 aa, synthetic construct
DIQMTQSPSSLSASVGDRVTITCSASSSVSYMNWYQQTPGKAPKRWIYDTSKLASGVPSRFSGSGSGTDYTFTISSLQPEDIATYYCQQWSSNPFTFGQGTKLQITRGGGGSQVQLQQSGAELVKPGSSVKISCKASGYTFTRNFIHWIKQQPGNGLEWIGWIFPGDGDTEYNQKFNGKATLTADKSSSTAYMQLSSLTSEDSAVYFCARGNYNYEYFDYWGQGVMVTVSSGGGGSGGGGSGGGGSGGGGSDIQMTQSPASLSASLGETVSIECLASEDIYSYLAWYQQKPGKSPQLLIFAANRLQDGVPSRFSGSGSGTQFSLKISGMQPEDEGDYFCLQGSKFPYTFGPGTKLELNGGGGSQVQLVQSGGGVVQPGRSLRLSCKASGYTFTRYTMHWVRQAPGKGLEWIGYINPSRGYTNYNQKVKDRFTISRDNSKNTAFLQMDSLRPEDTGVYFCARYYDDHYSLDYWGQGTPVTVSSDKTHTCPPCPAPEAAGGPSVFLFPPKPKDTLMISRTPEVTCVVVDVSHEDPEVKFNWYVDGVEVHNAKTKPREEQYNSTYRVVSVLTVLHQDWLNGKEYKCKVSNKALPAPIEKTISKAKGQPREPQVYTLPPSRDELTKNQVSLTCLVKGFYPSDIAVEWESNGQPENNYKTTPPVLDSDGSFFLYSKLTVDKSRWQQGNVFSCSVMHEALHNHYTQKSLSLSPGK

SEQ ID NO: 44 - protein, 709 aa, synthetic construct
QVQLQQSGAELVKPGSSVKISCKASGYTFTRNFIHWIKQQPGNGLEWIGWIFPGDGDTEYNQKFNGKATLTADKSSSTAYMQLSSLTSEDSAVYFCARGNYNYEYFDYWGQGVMVTVSSGGGGSDIQMTQSPSSLSASVGDRVTITCSASSSVSYMNWYQQTPGKAPKRWIYDTSKLASGVPSRFSGSGSGTDYTFTISSLQPEDIATYYCQQWSSNPFTFGQGTKLQITRGGGGSGGGGSGGGGSGGGGSQVQLVQSGGGVVQPGRSLRLSCKASGYTFTRYTMHWVRQAPGKGLEWIGYINPSRGYTNYNQKVKDRFTISRDNSKNTAFLQMDSLRPEDTGVYFCARYYDDHYSLDYWGQGTPVTVSSGGGGSDIQMTQSPASLSASLGETVSIECLASEDIYSYLAWYQQKPGKSPQLLIFAANRLQDGVPSRFSGSGSGTQFSLKISGMQPEDEGDYFCLQGSKFPYTFGPGTKLELNDKTHTCPPCPAPEAAGGPSVFLFPPKPKDTLMISRTPEVTCVVVDVSHEDPEVKFNWYVDGVEVHNAKTKPREEQYNSTYRVVSVLTVLHQDWLNGKEYKCKVSNKALPAPIEKTISKAKGQPREPQVYTLPPSRDELTKNQVSLTCLVKGFYPSDIAVEWESNGQPENNYKTTPPVLDSDGSFFLYSKLTVDKSRWQQGNVFSCSVMHEALHNHYTQKSLSLSPGK

SEQ ID NO: 45 - protein, 717 aa, synthetic construct
DIQMTQSPASLSASLGETVSIECLASEDIYSYLAWYQQKPGKSPQLLIFAANRLQDGVPSRFSGSGSGTQFSLKISGMQPEDEGDYFCLQGSKFPYTFGPGTKLELNGGGGSQVQLVQSGGGVVQPGRSLRLSCKASGYTFTRYTMHWVRQAPGKGLEWIGYINPSRGYTNYNQKVKDRFTISRDNSKNTAFLQMDSLRPEDTGVYFCARYYDDHYSLDYWGQGTPVTVSSGGGGSGGGGSGGGGSGGGGSDIQMTQSPSSLSASVGDRVTITCSASSSVSYMNWYQQTPGKAPKRWIYDTSKLASGVPSRFSGSGSGTDYTFTISSLQPEDIATYYCQQWSSNPFTFGQGTKLQITRGGGGSQVQLQQSGAELVKPGSSVKISCKASGYTFTRNFIHWIKQQPGNGLEWIGWIFPGDGDTEYNQKFNGKATLTADKSSSTAYMQLSSLTSEDSAVYFCARGNYNYEYFDYWGQGVMVTVSSLEVLFQGPDKTHTCPPCPAPEAAGGPSVFLFPPKPKDTLMISRTPEVTCVVVDVSHEDPEVKFNWYVDGVEVHNAKTKPREEQYNSTYRVVSVLTVLHQDWLNGKEYKCKVSNKALPAPIEKTISKAKGQPREPQVYTLPPSRDELTKNQVSLTCLVKGFYPSDIAVEWESNGQPENNYKTTPPVLDSDGSFFLYSKLTVDKSRWQQGNVFSCSVMHEALHNHYTQKSLSLSPGK

SEQ ID NO: 46 - protein, 493 aa, synthetic construct
QVQLQQSGAELVKPGSSVKISCKASGYTFTRNFIHWIKQQPGNGLEWIGWIFPGDGDTEYNQKFNGKATLTADKSSSTAYMQLSSLTSEDSAVYFCARGNYNYEYFDYWGQGVMVTVSSGGGGSGGGGSGGGGSDIQMTQSPASLSASLGETVSIECLASEDIYSYLAWYQQKPGKSPQLLIFAANRLQDGVPSRFSGSGSGTQFSLKISGMQPEDEGDYFCLQGSKFPYTFGPGTKLELNGGGGSQVQLVQSGGGVVQPGRSLRLSCKASGYTFTRYTMHWVRQAPGKGLEWIGYINPSRGYTNYNQKVKDRFTISRDNSKNTAFLQMDSLRPEDTGVYFCARYYDDHYSLDYWGQGTPVTVSSGGGGSGGGGSGGGGSDIQMTQSPSSLSASVGDRVTITCSASSSVSYMNWYQQTPGKAPKRWIYDTSKLASGVPSRFSGSGSGTDYTFTISSLQPEDIATYYCQQWSSNPFTFGQGTKLQITRHHHHHH

SEQ ID NO: 47 - protein, 493 aa, synthetic construct
DIQMTQSPASLSASLGETVSIECLASEDIYSYLAWYQQKPGKSPQLLIFAANRLQDGVPSRFSGSGSGTQFSLKISGMQPEDEGDYFCLQGSKFPYTFGPGTKLELNGGGGSGGGGSGGGGSQVQLQQSGAELVKPGSSVKISCKASGYTFTRNFIHWIKQQPGNGLEWIGWIFPGDGDTEYNQKFNGKATLTADKSSSTAYMQLSSLTSEDSAVYFCARGNYNYEYFDYWGQGVMVTVSSGGGGSQVQLVQSGGGVVQPGRSLRLSCKASGYTFTRYTMHWVRQAPGKGLEWIGYINPSRGYTNYNQKVKDRFTISRDNSKNTAFLQMDSLRPEDTGVYFCARYYDDHYSLDYWGQGTPVTVSSGGGGSGGGGSGGGGSDIQMTQSPSSLSASVGDRVTITCSASSSVSYMNWYQQTPGKAPKRWIYDTSKLASGVPSRFSGSGSGTDYTFTISSLQPEDIATYYCQQWSSNPFTFGQGTKLQITRHHHHHH

SEQ ID NO: 48 - protein, 493 aa, synthetic construct
QVQLVQSGGGVVQPGRSLRLSCKASGYTFTRYTMHWVRQAPGKGLEWIGYINPSRGYTNYNQKVKDRFTISRDNSKNTAFLQMDSLRPEDTGVYFCARYYDDHYSLDYWGQGTPVTVSSGGGGSGGGGSGGGGSDIQMTQSPSSLSASVGDRVTITCSASSSVSYMNWYQQTPGKAPKRWIYDTSKLASGVPSRFSGSGSGTDYTFTISSLQPEDIATYYCQQWSSNPFTFGQGTKLQITRGGGGSQVQLQQSGAELVKPGSSVKISCKASGYTFTRNFIHWIKQQPGNGLEWIGWIFPGDGDTEYNQKFNGKATLTADKSSSTAYMQLSSLTSEDSAVYFCARGNYNYEYFDYWGQGVMVTVSSGGGGSGGGGSGGGGSDIQMTQSPASLSASLGETVSIECLASEDIYSYLAWYQQKPGKSPQLLIFAANRLQDGVPSRFSGSGSGTQFSLKISGMQPEDEGDYFCLQGSKFPYTFGPGTKLELNHHHHHH

SEQ ID NO: 49 - protein, 493 aa, synthetic construct
QVQLVQSGGGVVQPGRSLRLSCKASGYTFTRYTMHWVRQAPGKGLEWIGYINPSRGYTNYNQKVKDRFTISRDNSKNTAFLQMDSLRPEDTGVYFCARYYDDHYSLDYWGQGTPVTVSSGGGGSGGGGSGGGGSDIQMTQSPSSLSASVGDRVTITCSASSSVSYMNWYQQTPGKAPKRWIYDTSKLASGVPSRFSGSGSGTDYTFTISSLQPEDIATYYCQQWSSNPFTFGQGTKLQITRGGGGSDIQMTQSPASLSASLGETVSIECLASEDIYSYLAWYQQKPGKSPQLLIFAANRLQDGVPSRFSGSGSGTQFSLKISGMQPEDEGDYFCLQGSKFPYTFGPGTKLELNGGGGSGGGGSGGGGSQVQLQQSGAELVKPGSSVKISCKASGYTFTRNFIHWIKQQPGNGLEWIGWIFPGDGDTEYNQKFNGKATLTADKSSSTAYMQLSSLTSEDSAVYFCARGNYNYEYFDYWGQGVMVTVSSHHHHHH

SEQ ID NO: 50 - protein, 449 aa, synthetic construct
QVQLQQSGAELVKPGSSVKISCKASGYTFTRNFIHWIKQQPGNGLEWIGWIFPGDGDTEYNQKFNGKATLTADKSSSTAYMQLSSLTSEDSAVYFCARGNYNYEYFDYWGQGVMVTVSSASTKGPSVFPLAPSSKSTSGGTAALGCLVKDYFPEPVTVSWNSGALTSGVHTFPAVLQSSGLYSLSSVVTVPSSSLGTQTYICNVNHKPSNTKVDKRVEPKSCDKTHTCPPCPAPEAAGGPSVFLFPPKPKDTLMISRTPEVTCVVVDVSHEDPEVKFNWYVDGVEVHNAKTKPREEQYNSTYRVVSVLTVLHQDWLNGKEYKCKVSNKALPAPIEKTISKAKGQPREPQVYTLPPCREEMTKNQVSLWCLVKGFYPSDIAVEWESNGQPENNYKTTPPVLDSDGSFFLYSKLTVDKSRWQQGNVFSCSVMHEALHNHYTQKSLSLSPGK

SEQ ID NO: 51 - protein, 695 aa, synthetic construct
QVQLQQSGAELVKPGSSVKISCKASGYTFTRNFIHWIKQQPGNGLEWIGWIFPGDGDTEYNQKFNGKATLTADKSSSTAYMQLSSLTSEDSAVYFCARGNYNYEYFDYWGQGVMVTVSSASTKGPSVFPLAPSSKSTSGGTAALGCLVKDYFPEPVTVSWNSGALTSGVHTFPAVLQSSGLYSLSSVVTVPSSSLGTQTYICNVNHKPSNTKVDKRVEPKSCDKTHTCPPCPAPEAAGGPSVFLFPPKPKDTLMISRTPEVTCVVVDVSHEDPEVKFNWYVDGVEVHNAKTKPREEQYNSTYRVVSVLTVLHQDWLNGKEYKCKVSNKALPAPIEKTISKAKGQPREPQVCTLPPSREEMTKNQVSLSCAVKGFYPSDIAVEWESNGQPENNYKTTPPVLDSDGSFFLVSKLTVDKSRWQQGNVFSCSVMHEALHNHYTQKSLSLSPGKGGGGSQVQLVQSGGGVVQPGRSLRLSCKASGYTFTRYTMHWVRQAPGKGLEWIGYINPSRGYTNYNQKVKDRFTISRDNSKNTAFLQMDSLRPEDTGVYFCARYYDDHYSLDYWGQGTPVTVSSGGGGSGGGGSGGGGSDIQMTQSPSSLSASVGDRVTITCSASSSVSYMNWYQQTPGKAPKRWIYDTSKLASGVPSRFSGSGSGTDYTFTISSLQPEDIATYYCQQWSSNPFTFGQGTKLQITR

SEQ ID NO: 52 - protein, 214 aa, synthetic construct
DIQMTQSPASLSASLGETVSIECLASEDIYSYLAWYQQKPGKSPQLLIFAANRLQDGVPSRFSGSGSGTQFSLKISGMQPEDEGDYFCLQGSKFPYTFGPGTKLELNRTVAAPSVFIFPPSDEQLKSGTASVVCLLNNFYPREAKVQWKVDNALQSGNSQESVTEQDSKDSTYSLSSTLTLSKADYEKHKVYACEVTHQGLSSPVTKSFNRGEC

SEQ ID NO: 53 - protein, 695 aa, synthetic construct
QVQLQQSGAELVKPGSSVKISCKASGYTFTRNFIHWIKQQPGNGLEWIGWIFPGDGDTEYNQKFNGKATLTADKSSSTAYMQLSSLTSEDSAVYFCARGNYNYEYFDYWGQGVMVTVSSASTKGPSVFPLAPSSKSTSGGTAALGCLVKDYFPEPVTVSWNSGALTSGVHTFPAVLQSSGLYSLSSVVTVPSSSLGTQTYICNVNHKPSNTKVDKRVEPKSCDKTHTCPPCPAPEAAGGPSVFLFPPKPKDTLMISRTPEVTCVVVDVSHEDPEVKFNWYVDGVEVHNAKTKPREEQYNSTYRVVSVLTVLHQDWLNGKEYKCKVSNKALPAPIEKTISKAKGQPREPQVYTLPPSREEMTKNQVSLTCLVKGFYPSDIAVEWESNGQPENNYKTTPPVLDSDGSFFLYSKLTVDKSRWQQGNVFSCSVMHEALHNHYTQKSLSLSPGKGGGGSQVQLVQSGGGVVQPGRSLRLSCKASGYTFTRYTMHWVRQAPGKGLEWIGYINPSRGYTNYNQKVKDRFTISRDNSKNTAFLQMDSLRPEDTGVYFCARYYDDHYSLDYWGQGTPVTVSSGGGGSGGGGSGGGGSDIQMTQSPSSLSASVGDRVTITCSASSSVSYMNWYQQTPGKAPKRWIYDTSKLASGVPSRFSGSGSGTDYTFTISSLQPEDIATYYCQQWSSNPFTFGQGTKLQITR

SEQ ID NO: 54 - protein, 473 aa, synthetic construct
QVQLVQSGGGVVQPGRSLRLSCKASGYTFTRYTMHWVRQAPGKGLEWIGYINPSRGYTNYNQKVKDRFTISRDNSKNTAFLQMDSLRPEDTGVYFCARYYDDHYSLDYWGQGTPVTVSSGGGGSGGGGSGGGGSDIQMTQSPSSLSASVGDRVTITCSASSSVSYMNWYQQTPGKAPKRWIYDTSKLASGVPSRFSGSGSGTDYTFTISSLQPEDIATYYCQQWSSNPFTFGQGTKLQITREPKSCDKTHTCPPCPAPEAAGGPSVFLFPPKPKDTLMISRTPEVTCVVVDVSHEDPEVKFNWYVDGVEVHNAKTKPREEQYNSTYRVVSVLTVLHQDWLNGKEYKCKVSNKALPAPIEKTISKAKGQPREPQVCTLPPSREEMTKNQVSLSCAVKGFYPSDIAVEWESNGQPENNYKTTPPVLDSDGSFFLVSKLTVDKSRWQQGNVFSCSVMHEALHNHYTQKSLSLSPGK

SEQ ID NO: 55 - protein, 474 aa, synthetic construct
QVQLQQSGAELVKPGSSVKISCKASGYTFTRNFIHWIKQQPGNGLEWIGWIFPGDGDTEYNQKFNGKATLTADKSSSTAYMQLSSLTSEDSAVYFCARGNYNYEYFDYWGQGVMVTVSSASTKGPSVFPLAPSSKSTSGGTAALGCLVKDYFPEPVTVSWNSGALTSGVHTFPAVLQSSGLYSLSSVVTVPSSSLGTQTYICNVNHKPSNTKVDKRVEPKSCGGGGSQVQLVQSGGGVVQPGRSLRLSCKASGYTFTRYTMHWVRQAPGKGLEWIGYINPSRGYTNYNQKVKDRFTISRDNSKNTAFLQMDSLRPEDTGVYFCARYYDDHYSLDYWGQGTPVTVSSGGGGSGGGGSGGGGSDIQMTQSPSSLSASVGDRVTITCSASSSVSYMNWYQQTPGKAPKRWIYDTSKLASGVPSRFSGSGSGTDYTFTISSLQPEDIATYYCQQWSSNPFTFGQGTKLQITRHHHHHH

SEQ ID NO: 56 - protein, 695 aa, synthetic construct
QVQLQQSGAELVKPGSSVKISCKASGYTFTRNFIHWIKQQPGNGLEWIGWIFPGDGDTEYNQKFNGKATLTADKSSSTAYMQLSSLTSEDSAVYFCARGNYNYEYFDYWGQGVMVTVSSASTKGPSVFPLAPSSKSTSGGTAALGCLVKDYFPEPVTVSWNSGALTSGVHTFPAVLQSSGLYSLSSVVTVPSSSLGTQTYICNVNHKPSNTKVDKRVEPKSCGGGGSQVQLVQSGGGVVQPGRSLRLSCKASGYTFTRYTMHWVRQAPGKGLEWIGYINPSRGYTNYNQKVKDRFTISRDNSKNTAFLQMDSLRPEDTGVYFCARYYDDHYSLDYWGQGTPVTVSSGGGGSGGGGSGGGGSDIQMTQSPSSLSASVGDRVTITCSASSSVSYMNWYQQTPGKAPKRWIYDTSKLASGVPSRFSGSGSGTDYTFTISSLQPEDIATYYCQQWSSNPFTFGQGTKLQITRDKTHTCPPCPAPEAAGGPSVFLFPPKPKDTLMISRTPEVTCVVVDVSHEDPEVKFNWYVDGVEVHNAKTKPREEQYNSTYRVVSVLTVLHQDWLNGKEYKCKVSNKALPAPIEKTISKAKGQPREPQVYTLPPSREEMTKNQVSLTCLVKGFYPSDIAVEWESNGQPENNYKTTPPVLDSDGSFFLYSKLTVDKSRWQQGNVFSCSVMHEALHNHYTQKSLSLSPGK

SEQ ID NO: 57 - protein, 580 aa, synthetic construct
QVQLQQSGAELVKPGSSVKISCKASGYTFTRNFIHWIKQQPGNGLEWIGWIFPGDGDTEYNQKFNGKATLTADKSSSTAYMQLSSLTSEDSAVYFCARGNYNYEYFDYWGQGVMVTVSSASTKGPSVFPLAPSSKSTSGGTAALGCLVKDYFPEPVTVSWNSGALTSGVHTFPAVLQSSGLYSLSSVVTVPSSSLGTQTYICNVNHKPSNTKVDKRVEPKSCGGGGSQVQLVQSGGGVVQPGRSLRLSCKASGYTFTRYTMHWVRQAPGKGLEWIGYINPSRGYTNYNQKVKDRFTISRDNSKNTAFLQMDSLRPEDTGVYFCARYYDDHYSLDYWGQGTPVTVSSGGGGSGGGGSGGGGSDIQMTQSPSSLSASVGDRVTITCSASSSVSYMNWYQQTPGKAPKRWIYDTSKLASGVPSRFSGSGSGTDYTFTISSLQPEDIATYYCQQWSSNPFTFGQGTKLQITRAAAGGGQPREPQVYTLPPSREEMTKNQVSLTCLVKGFYPSDIAVEWESNGQPENNYKTTPPVLDSDGSFFLYSKLTVDKSRWQQGNVFSCSVMHEALHNHYTQKSLSLSPGK

SEQ ID NO: 58 - protein, 701 aa, synthetic construct
QVQLQQSGAELVKPGSSVKISCKASGYTFTRNFIHWIKQQPGNGLEWIGWIFPGDGDTEYNQKFNGKATLTADKSSSTAYMQLSSLTSEDSAVYFCARGNYNYEYFDYWGQGVMVTVSSASTKGPSVFPLAPSSKSTSGGTAALGCLVKDYFPEPVTVSWNSGALTSGVHTFPAVLQSSGLYSLSSVVTVPSSSLGTQTYICNVNHKPSNTKVDKRVEPKSCGGGGSQVQLVQSGGGVVQPGRSLRLSCKASGYTFTRYTMHWVRQAPGKGLEWIGYINPSRGYTNYNQKVKDRFTISRDNSKNTAFLQMDSLRPEDTGVYFCARYYDDHYSLDYWGQGTPVTVSSGGGGSGGGGSGGGGSDIQMTQSPSSLSASVGDRVTITCSASSSVSYMNWYQQTPGKAPKRWIYDTSKLASGVPSRFSGSGSGTDYTFTISSLQPEDIATYYCQQWSSNPFTFGQGTKLQITRGGGGSQVQLQQSGAELVKPGSSVKISCKASGYTFTRNFIHWIKQQPGNGLEWIGWIFPGDGDTEYNQKFNGKATLTADKSSSTAYMQLSSLTSEDSAVYFCARGNYNYEYFDYWGQGVMVTVSSASTKGPSVFPLAPSSKSTSGGTAALGCLVKDYFPEPVTVSWNSGALTSGVHTFPAVLQSSGLYSLSSVVTVPSSSLGTQTYICNVNHKPSNTKVDKRVEPKSCHHHHHH

SEQ ID NO: 59 - protein, 474 aa, synthetic construct
QVQLVQSGGGVVQPGRSLRLSCKASGYTFTRYTMHWVRQAPGKGLEWIGYINPSRGYTNYNQKVKDRFTISRDNSKNTAFLQMDSLRPEDTGVYFCARYYDDHYSLDYWGQGTPVTVSSGGGGSGGGGSGGGGSDIQMTQSPSSLSASVGDRVTITCSASSSVSYMNWYQQTPGKAPKRWIYDTSKLASGVPSRFSGSGSGTDYTFTISSLQPEDIATYYCQQWSSNPFTFGQGTKLQITRGGGGSQVQLQQSGAELVKPGSSVKISCKASGYTFTRNFIHWIKQQPGNGLEWIGWIFPGDGDTEYNQKFNGKATLTADKSSSTAYMQLSSLTSEDSAVYFCARGNYNYEYFDYWGQGVMVTVSSASTKGPSVFPLAPSSKSTSGGTAALGCLVKDYFPEPVTVSWNSGALTSGVHTFPAVLQSSGLYSLSSVVTVPSSSLGTQTYICNVNHKPSNTKVDKRVEPKSCHHHHHH

SEQ ID NO: 60 - protein, 695 aa, synthetic construct
QVQLVQSGGGVVQPGRSLRLSCKASGYTFTRYTMHWVRQAPGKGLEWIGYINPSRGYTNYNQKVKDRFTISRDNSKNTAFLQMDSLRPEDTGVYFCARYYDDHYSLDYWGQGTPVTVSSGGGGSGGGGSGGGGSDIQMTQSPSSLSASVGDRVTITCSASSSVSYMNWYQQTPGKAPKRWIYDTSKLASGVPSRFSGSGSGTDYTFTISSLQPEDIATYYCQQWSSNPFTFGQGTKLQITRGGGGSQVQLQQSGAELVKPGSSVKISCKASGYTFTRNFIHWIKQQPGNGLEWIGWIFPGDGDTEYNQKFNGKATLTADKSSSTAYMQLSSLTSEDSAVYFCARGNYNYEYFDYWGQGVMVTVSSASTKGPSVFPLAPSSKSTSGGTAALGCLVKDYFPEPVTVSWNSGALTSGVHTFPAVLQSSGLYSLSSVVTVPSSSLGTQTYICNVNHKPSNTKVDKRVEPKSCDKTHTCPPCPAPEAAGGPSVFLFPPKPKDTLMISRTPEVTCVVVDVSHEDPEVKFNWYVDGVEVHNAKTKPREEQYNSTYRVVSVLTVLHQDWLNGKEYKCKVSNKALPAPIEKTISKAKGQPREPQVYTLPPSREEMTKNQVSLTCLVKGFYPSDIAVEWESNGQPENNYKTTPPVLDSDGSFFLYSKLTVDKSRWQQGNVFSCSVMHEALHNHYTQKSLSLSPGK

SEQ ID NO: 61 - protein, 580 aa, synthetic construct
QVQLVQSGGGVVQPGRSLRLSCKASGYTFTRYTMHWVRQAPGKGLEWIGYINPSRGYTNYNQKVKDRFTISRDNSKNTAFLQMDSLRPEDTGVYFCARYYDDHYSLDYWGQGTPVTVSSGGGGSGGGGSGGGGSDIQMTQSPSSLSASVGDRVTITCSASSSVSYMNWYQQTPGKAPKRWIYDTSKLASGVPSRFSGSGSGTDYTFTISSLQPEDIATYYCQQWSSNPFTFGQGTKLQITRGGGGSQVQLQQSGAELVKPGSSVKISCKASGYTFTRNFIHWIKQQPGNGLEWIGWIFPGDGDTEYNQKFNGKATLTADKSSSTAYMQLSSLTSEDSAVYFCARGNYNYEYFDYWGQGVMVTVSSASTKGPSVFPLAPSSKSTSGGTAALGCLVKDYFPEPVTVSWNSGALTSGVHTFPAVLQSSGLYSLSSVVTVPSSSLGTQTYICNVNHKPSNTKVDKRVEPKSCAAAGGGQPREPQVYTLPPSREEMTKNQVSLTCLVKGFYPSDIAVEWESNGQPENNYKTTPPVLDSDGSFFLYSKLTVDKSRWQQGNVFSCSVMHEALHNHYTQKSLSLSPGK

SEQ ID NO: 62 - protein, 228 aa, synthetic construct
QVQLQQSGAELVKPGSSVKISCKASGYTFTRNFIHWIKQQPGNGLEWIGWIFPGDGDTEYNQKFNGKATLTADKSSSTAYMQLSSLTSEDSAVYFCARGNYNYEYFDYWGQGVMVTVSSASTKGPSVFPLAPSSKSTSGGTAALGCLVKDYFPEPVTVSWNSGALTSGVHTFPAVLQSSGLYSLSSVVTVPSSSLGTQTYICNVNHKPSNTKVDKRVEPKSCHHHHHH

SEQ ID NO: 63 - protein, 460 aa, synthetic construct
QVQLVQSGGGVVQPGRSLRLSCKASGYTFTRYTMHWVRQAPGKGLEWIGYINPSRGYTNYNQKVKDRFTISRDNSKNTAFLQMDSLRPEDTGVYFCARYYDDHYSLDYWGQGTPVTVSSGGGGSGGGGSGGGGSDIQMTQSPSSLSASVGDRVTITCSASSSVSYMNWYQQTPGKAPKRWIYDTSKLASGVPSRFSGSGSGTDYTFTISSLQPEDIATYYCQQWSSNPFTFGQGTKLQITRGGGGSDIQMTQSPASLSASLGETVSIECLASEDIYSYLAWYQQKPGKSPQLLIFAANRLQDGVPSRFSGSGSGTQFSLKISGMQPEDEGDYFCLQGSKFPYTFGPGTKLELNRTVAAPSVFIFPPSDEQLKSGTASVVCLLNNFYPREAKVQWKVDNALQSGNSQESVTEQDSKDSTYSLSSTLTLSKADYEKHKVYACEVTHQGLSSPVTKSFNRGEC

SEQ ID NO: 64 - protein, 449 aa, synthetic construct
QVQLQQSGAELVKPGSSVKISCKASGYTFTRNFIHWIKQQPGNGLEWIGWIFPGDGDTEYNQKFNGKATLTADKSSSTAYMQLSSLTSEDSAVYFCARGNYNYEYFDYWGQGVMVTVSSASTKGPSVFPLAPSSKSTSGGTAALGCLVKDYFPEPVTVSWNSGALTSGVHTFPAVLQSSGLYSLSSVVTVPSSSLGTQTYICNVNHKPSNTKVDKRVEPKSCDKTHTCPPCPAPEAAGGPSVFLFPPKPKDTLMISRTPEVTCVVVDVSHEDPEVKFNWYVDGVEVHNAKTKPREEQYNSTYRVVSVLTVLHQDWLNGKEYKCKVSNKALPAPIEKTISKAKGQPREPQVYTLPPSREEMTKNQVSLTCLVKGFYPSDIAVEWESNGQPENNYKTTPPVLDSDGSFFLYSKLTVDKSRWQQGNVFSCSVMHEALHNHYTQKSLSLSPGK

SEQ ID NO: 65 - protein, 334 aa, synthetic construct
QVQLQQSGAELVKPGSSVKISCKASGYTFTRNFIHWIKQQPGNGLEWIGWIFPGDGDTEYNQKFNGKATLTADKSSSTAYMQLSSLTSEDSAVYFCARGNYNYEYFDYWGQGVMVTVSSASTKGPSVFPLAPSSKSTSGGTAALGCLVKDYFPEPVTVSWNSGALTSGVHTFPAVLQSSGLYSLSSVVTVPSSSLGTQTYICNVNHKPSNTKVDKRVEPKSCAAAGGGQPREPQVYTLPPSREEMTKNQVSLTCLVKGFYPSDIAVEWESNGQPENNYKTTPPVLDSDGSFFLYSKLTVDKSRWQQGNVFSCSVMHEALHNHYTQKSLSLSPGK

SEQ ID NO: 66 - DNA, 2142 bp, synthetic construct
  source 1..2142: mol_type = other DNA
caggtgcaactgcagcagtccggggctgagctggtgaagcctggtagctctgtaaagatctcttgcaaggcaagcggctacacttttacccgaaacttcatccattggatcaaacagcaaccaggcaatggactagagtggattggatggatctttcctggcgatggggacaccgaatacaatcagaaattcaacgggaaagccaccttaactgctgataagtcttcctcaaccgcatacatgcagttaagcagcctgacatccgaggattcagccgtgtacttttgtgctagaggcaactacaattacgagtatttcgattattggggccagggcgttatggtcaccgtgtcatccggtggtggcgggagtggcggaggtggctctggtggtggaggatctgatatacagatgacgcagagtcccgccagcttatctgcgtccctgggggaaaccgtgtcgattgaatgcctagcaagtgaggacatctatagctaccttgcatggtaccaacagaaacccggtaaaagtcctcagttgttgatatttgccgccaaccggttacaggacggagtccccagcaggttttctgggtcagggagcggtacacagttttccctgaagatctcagggatgcagccagaagacgagggcgattacttctgtctgcagggttctaagttcccgtacaccttcggacctggcactaagctggaactcaatggcggcggcggtagccaggtccagcttgttcagtctgggggaggggtagtgcaaccaggaagatccctgaggctgtcatgcaaagcctccgggtatacattcacccgctatacgatgcattgggtgagacaggcaccgggaaaggggcttgaatggatcggctatattaacccatcaagaggctacactaactataaccagaaagtgaaagaccggtttactatctcgcgtgataacagcaaaaacactgccttcttgcagatggatagcctgaggccagaggacacaggcgtgtatttttgtgcgcggtattatgacgaccattactcgctcgactattgggggcaaggcactcctgtcaccgtcagctctggaggcgggggaagtggaggaggagggtccggtggcgggggatcagacatccaaatgactcagagcccctcaagtctgtcagcttcggtgggcgatcgcgtcacgattacttgtagcgccagtagtagcgttagctacatgaactggtatcagcaaacaccaggtaaagcccccaaacgctggatttatgacaccagcaaattggcttctggagtgcctagtcgttttagcggatctggatcaggcacagactacaccttcaccatttcctcccttcaacccgaggacatagcgacatactactgtcagcagtggagttccaatccattcacgtttggtcaaggaacgaagctgcagataaccagagacaagactcacacttgccctccttgtcctgcccccgaagccgccggcggcccttcagtatttctctttccaccgaaacctaaggacacattgatgatctcacgcactccagaagtgacctgcgtggtggttgatgtctcacacgaagatcctgaggtgaaattcaactggtacgtagatggcgtggaagtccataacgcgaagacaaagcccagagaggagcagtataattcgacctatcgggtggtttcggtactgaccgtcctgcatcaggactggcttaacggcaaggagtacaagtgcaaggtttctaataaagccctcccagctcccatcgagaaaacaatcagcaaggctaagggccaacccagggaaccccaagtctacactttgccaccgagtcgtgacgagctcacaaaaaatcaggtgtctttaacttgcctcgtaaagggcttttatcccagcgacattgccgtcgagtgggaatcgaatggccagccagaaaacaactacaagactactccacccgtgctcgactcagacggctcctttttcctgtactccaaacttactgtggataagagtagatggcagcagggcaatgtgttctcctgttcagtgatgcatgaagcccttcacaaccattacacacagaaatccttgtctctgtccccaggcaag

SEQ ID NO: 67 - DNA, 2166 bp, synthetic construct
  source 1..2166: mol_type = other DNA
gatatccagatgacgcagagccctgcttccctgtccgccagcttgggcgaaacagtgagcatcgaatgtctggcgtccgaggatatctacagctacctggcttggtaccagcagaaacccgggaagtcacctcagttgctgatatttgccgctaacaggctccaggatggggtgccaagcagattttcagggtccgggagtgggacgcagttcagcctcaaaatctccgggatgcagcccgaagacgaaggggactacttttgcctccaaggatctaagtttccgtacactttcggacctggaaccaaacttgagctgaatggcggcggcggctccggcggcggtggatccggggggggcgggagccaggtccaactgcagcagtctggcgccgaactcgtcaagccgggcagtagtgtgaagatctcttgtaaagcaagcggctatacctttacccggaattttattcactggattaagcagcaaccaggcaatggcctagagtggataggatggatctttccaggcgatggtgacacagaatacaatcagaagttcaatggcaaagcaacactgactgccgacaaaagcagtagcactgcctacatgcagctctcatccttaacctcagaggactcagccgtctacttctgcgctagaggaaactacaactacgagtacttcgactactggggccaaggcgtaatggtgactgtgtcttcgggagggggaggttcacaggttcagctggtgcagtctggaggcggagtggtccaaccaggtcgctccctgaggctgagttgcaaggcatccggttataccttcacccgctacactatgcactgggttcgacaagctccaggtaaagggctcgaatggattgggtatatcaacccttctcgggggtataccaactataaccagaaggttaaagaccggttcaccattagccgggataactctaagaacactgcatttctgcagatggattccctcagacccgaagatacgggtgtgtacttctgtgccagatactacgatgaccactacagcttggactattgggggcaaggaactcctgtaaccgtgagcagtggaggagggggctctggtggaggtggatctggcggaggaggctccgacatacagatgacccagtctccctcgtccttgtccgcctccgtaggagatcgggtgactatcacctgttcagcatcctcgtcagtgagctatatgaactggtatcaacaaacaccagggaaagctccgaagcgctggatctacgataccagcaagttagcgtcaggcgtcccctctcgatttagtggctctgggtcagggacagactatacatttacgatctcaagccttcaacctgaggacattgccacgtattattgccagcagtggtcttctaatccattcacctttggtcaggggactaaactgcagattactaggttggaggtactcttccaaggtcctgacaagacacatacttgtcccccatgtcccgctccagaattgcttggtggtccaagcgtattcctatttcccccgaaacccaaggatactctcatgatatcacgtacacccgaagtgacatgcgttgtcgtagacgttagtcatgaggatcctgaggtgaaattcaactggtatgtggacggcgttgaagtgcacaatgccaagacaaagccacgtgaggaacagtacaatagcacctatagggtggtttcagtgttaacagtcctgcatcaggattggcttaatggcaaggagtacaagtgcaaagtctcgaacaaggcactgcctgctccgattgagaagacaatctcgaaagcgaagggacagcctagagaaccacaggtgtacacactccctcccagtagggacgagctaacaaagaatcaggtgagcttaacctgcctcgtgaaaggcttttatccctccgatattgcagtcgagtgggagtccaacggtcaacccgagaacaactataagacaactccccctgtgttggacagtgacggatccttcttcctgtatagcaaacttaccgtcgataaaagtcgctggcagcagggaaatgttttcagttgcagcgtgatgcatgaggccctgcacaatcactatacccagaagagtctttctctatctcctggcaaa

SEQ ID NO: 68 - DNA, 2142 bp, synthetic construct
  source 1..2142: mol_type = other DNA
caggttcaactggtgcagtccggcggtggcgtggtgcaacctggcagatccttacggctgtcttgtaaggcatctggctacactttcacccggtatacgatgcattgggtgaggcaggcaccaggaaaggggttggagtggatcggttacattaatcccagccgaggctataccaactataaccagaaggtcaaagacaggtttacaatcagccgagacaatagcaagaataccgcctttcttcagatggactccctaagacctgaggacactggcgtgtatttctgcgcccgttattacgatgaccactactccctggactattggggccaggggaccccggtaacagtgtcttccggaggcggcggatctggcggaggtggatccggcggcggtgggtccgatatccaaatgactcagtcaccgagcagtctgtccgccagcgttggggacagagtgaccatcacatgcagtgctagttcctccgtctcttacatgaattggtatcagcagactccgggtaaggcgcctaaaaggtggatttacgatacctccaagctcgcatccggtgttccttccagatttagcgggtccggctctgggactgactacacattcaccataagtagcctacaacccgaagatatcgcaacctattactgtcagcagtggtcttcgaatccttttacgtttggacagggaaccaaactgcagattacacggggagggggcggctctcaagtgcagttacaacagtcgggcgctgaacttgtgaaaccaggctcttcagtcaagatcagttgcaaagcctctggctatacattcactcgcaatttcatccactggataaagcagcaacctggaaatggcctggaatggataggatggattttccccggtgatggcgatacagagtacaaccagaagttcaacgggaaagctaccctcactgccgataagtccagttctaccgcatacatgcagcttagtagcttgacaagtgaagatagcgctgtctacttttgcgccagaggaaactacaattacgagtattttgactactggggccaaggggtcatggtcacagttagctcagggggaggcgggtcaggagggggagggagcggaggcggtggcagcgacattcagatgactcagagccccgcttctctttccgcctcactcggggagactgtgagcatcgagtgtctcgcaagcgaggatatctattcctatctggcttggtaccagcagaaacccggcaaatcgccacagctcttgattttcgccgcgaaccggctgcaggatggggttcctagccgcttcagcggttccgggagcggaacacagttctcactgaaaatttcagggatgcagcccgaggacgaaggtgactacttttgtctgcaagggtcgaagttcccctatacgttcggtccaggaaccaagctggagctcaacgacaagactcacacttgccctccttgtcctgcccccgaagccgccggcggcccttcagtatttctctttccaccgaaacctaaggacacattgatgatctcacgcactccagaagtgacctgcgtggtggttgatgtctcacacgaagatcctgaggtgaaattcaactggtacgtagatggcgtggaagtccataacgcgaagacaaagcccagagaggagcagtataattcgacctatcgggtggtttcggtactgaccgtcctgcatcaggactggcttaacggcaaggagtacaagtgcaaggtttctaataaagccctcccagctcccatcgagaaaacaatcagcaaggctaagggccaacccagggaaccccaagtctacactttgccaccgagtcgtgacgagctcacaaaaaatcaggtgtctttaacttgcctcgtaaagggcttttatcccagcgacattgccgtcgagtgggaatcgaatggccagccagaaaacaactacaagactactccacccgtgctcgactcagacggctcctttttcctgtactccaaacttactgtggataagagtagatggcagcagggcaatgtgttctcctgttcagtgatgcatgaagcccttcacaaccattacacacagaaatccttgtctctgtccccaggcaag

SEQ ID NO: 69 - DNA, 2142 bp, synthetic construct
  source 1..2142: mol_type = other DNA
caagtgcaactcgtccagtccggtggaggcgtagtacagccaggcagatcattgagactgagctgcaaggccagcgggtacacttttacgcgctacactatgcattgggtgagacaggcaccaggcaaggggttggaatggatagggtacatcaatcccagccgcggatataccaattacaatcagaaggtcaaagatcggttcaccatttctagggataacagcaagaacactgccttcctgcagatggactctctgcggcctgaggatactggggtgtacttctgtgctcgctactacgacgaccactattccctagattactggggacagggcaccccagtcacagtttcgtcaggaggaggtgggtccggcggagggggtagcgggggcggaggctcagatatccagatgactcagagtccctcgagcctttctgcttccgtaggcgatcgggtgaccatcacttgttctgcgtccagcagtgtcagttacatgaactggtatcaacagactccagggaaagctcccaaaaggtggatctatgacacaagtaagttggccagcggcgtcccctcgcgcttcagtgggtctggctccggcaccgactatacctttacaatctcaagccttcagcccgaagacattgctacatactactgtcagcagtggtcaagtaacccattcaccttcgggcagggcacaaagctccagattacacgagggggaggaggcagcgacatccaaatgacccagagccccgctagcttgagcgccagtcttggcgagactgtgtctatagagtgcttagcctctgaggatatctactcttatctggcatggtatcagcagaagcctgggaaatcccctcagctgctgatctttgccgcgaatcggctacaggatggagtcccttctcgttttagtggctctggcagtggtacgcaattttccctgaagatctcaggcatgcagccggaagacgagggcgactatttctgcttacagggcagcaaatttccctataccttcggtccgggtacaaaacttgagctgaatggtggggggggctccgggggtggcgggtcaggcggcggcggatcccaggttcagctgcagcagtcaggagctgaactggtgaaacccggatcgagcgttaagatttcttgcaaagcatcagggtatacgtttacgcgaaacttcatccactggattaagcagcagccaggtaacggcttggagtggataggctggatttttcccggagacggagacaccgagtataaccagaagttcaatggcaaggcaacactgacagctgacaagtccagtagcacagcctacatgcaactgtcttcactgactagcgaagattcagccgtctacttttgcgcacgggggaattacaactacgagtacttcgactattggggtcaaggcgttatggtgactgtgagttccgataagacacatacctgtcctccatgccctgctcctgaagctgctggaggtcccagcgtctttttgtttcctccaaaaccgaaagacacactgatgatttcccgtaccccggaagttacctgtgtggtggtggatgtttctcacgaggatccggaagtgaagttcaactggtatgttgatggtgtagaggtccacaatgcgaagaccaaacctagggaggagcaatacaactccacctatagggtggtcagcgtgctaactgtgctccatcaggactggctgaatgggaaggagtacaagtgcaaagtctccaataaagcattacctgcaccaatcgagaaaaccatctccaaggccaaaggacaaccaagagaacctcaggtgtacacactgcccccatccagagatgagctcaccaaaaaccaggtgtctctgacttgcctcgtaaagggattctatcccagtgacattgccgtggaatgggagtccaatggacaacccgaaaacaactacaagacaaccccacctgtgctggactcggatggtagcttcttcctgtattctaagctcacggtggataaatctaggtggcagcaggggaatgtgtttagttgtagcgtaatgcatgaagccttacacaaccactatacgcagaaatccctttcactgtcacctggtaag

SEQ ID NO: 70 - DNA, 2151 bp, synthetic construct
  source 1..2151: mol_type = other DNA
caggtccagttggtccaatctggaggcggtgtagttcagcctgggaggtctttacgcctgagctgtaaagcaagcggatatacattcacccggtacaccatgcactgggtgagacaggctcccggaaagggacttgagtggatagggtatatcaacccgtctcgtggttataccaactacaaccagaaggtgaaagacagattcaccatctctagggacaactccaagaacacagcgtttctgcagatggatagcttacggccagaggatactggcgtgtatttctgcgccagatactacgatgaccactacagcctggattattggggccagggtacccctgtgactgtctcgtcaggcgggggaggtagtgatatccagatgacccagtccccagcttctctatccgcttcattgggagaaaccgtttccattgaatgtctggcttctgaggacatttacagctacctggcgtggtatcagcagaaacccgggaaatcccctcagctcctcattttcgctgccaatcgcctgcaagatggggttccatcccggtttagcgggagcgggtctggaacccagttctccctgaagatctccggcatgcaacctgaggatgagggggactacttttgcctgcaggggagcaaattcccctatacatttggtccgggtacgaaactggagctcaatggaggtgggggatccggaggcggaggaagcggcggagggggcagcggggggggtggtagtcaggtgcagctacaacagagtggagctgagctggtcaagcccgggagtagtgtcaagatttcctgcaaagccagtggatatacgttcacgcgaaatttcattcactggattaagcagcagccaggcaacggcttagagtggatcggatggatctttcctggggatggtgataccgagtataaccagaaattcaatggtaaagccactctaacagccgataagagcagtagcactgcctatatgcaattgtcatccctaacctctgaagacagtgcagtgtacttctgtgcacgagggaattacaattatgagtacttcgactattgggggcagggagttatggtaaccgtgagcagtggaggtggtgggagcgacatacagatgactcaatctcctagctctctgtcagcaagtgtgggagatcgagtgaccataacgtgcagcgcctccagctcagtctcatacatgaactggtaccaacagacgccaggaaaagcacccaaacggtggatttacgacacatcgaagctggccagtggggtgccgtctcgcttctccgggtctggctcaggcaccgactacacctttacaatctcatctctgcagcccgaagatatagccacatattattgtcaacagtggagcagcaatccctttacatttggccaaggcaccaagctccagattacgaggctggaagtgctgtttcaaggccctgacaagactcacacttgccctccttgtcctgcccccgaagccgccggcggcccttcagtatttctctttccaccgaaacctaaggacacattgatgatctcacgcactccagaagtgacctgcgtggtggttgatgtctcacacgaagatcctgaggtgaaattcaactggtacgtagatggcgtggaagtccataacgcgaagacaaagcccagagaggagcagtataattcgacctatcgggtggtttcggtactgaccgtcctgcatcaggactggcttaacggcaaggagtacaagtgcaaggtttctaataaagccctcccagctcccatcgagaaaacaatcagcaaggctaagggccaacccagggaaccccaagtctacactttgccaccgagtcgtgacgagctcacaaaaaatcaggtgtctttaacttgcctcgtaaagggcttttatcccagcgacattgccgtcgagtgggaatcgaatggccagccagaaaacaactacaagactactccacccgtgctcgactcagacggctcctttttcctgtactccaaacttactgtggataagagtagatggcagcagggcaatgtgttctcctgttcagtgatgcatgaagcccttcacaaccattacacacagaaatccttgtctctgtccccaggcaag

SEQ ID NO: 71 - DNA, 2127 bp, synthetic construct
  source 1..2127: mol_type = other DNA
gatatccagatgactcaaagtccctcctctcttagcgcaagcgtaggagatcgggtgaccattacatgctctgcatcgagctcagtatcatacatgaattggtaccagcagacaccaggaaaagccccgaagcggtggatttatgacactagtaaactcgcttctggagtcccaagccgcttcagtgggtctggaagtgggacagactatactttcacaatcagcagtctacagccagaggacattgctacttactactgccaacagtggtcttccaaccctttcacctttggccagggcactaaattgcagattaccagaggtggaggtggatcccaggtgcagttacagcagtctggcgctgaactggtgaaacccgggtcatctgtgaagatatcctgcaaggctagcggatatacattcacccgaaacttcatccactggataaagcagcagcctgggaatggcttggagtggattggttggatttttcccggcgacggggatactgagtacaatcagaagttcaacggcaaagccaccttaaccgcggataagtcgagtagcacagcttacatgcagttgtcatccctaacatctgaggatagcgccgtgtatttctgcgcaagagggaattataactacgaatacttcgattattgggggcaaggagttatggtgacagtgagctctggcggcgggggatccggtgggggaggctcaggaggaggaggcagcggaggagggggaagcgacatccaaatgactcagtcccctgcctcactcagtgccagtttgggagaaacggtgtccatcgaatgtttggcctctgaggacatatacagctacctcgcctggtatcagcagaagcctggcaagtcccctcaactgctcatttttgctgccaatcgcttacaggacggcgtacctagccggttttcaggttctggctcaggtactcaattcagtttaaagatatccggcatgcagccagaagatgagggcgattatttctgcttgcagggtagcaagtttccctacaccttcggtcccggcactaagctcgaactcaatggaggcggcgggtcacaggtccaactagtccagtccggtggcggcgtggttcagcctgggcgttcccttagactgagctgtaaggccagcgggtacaccttcaccagatacaccatgcactgggtgcgccaagcaccagggaaaggccttgagtggatcggttacatcaatccatcgaggggatacacgaactataaccagaaagtcaaagatcggtttacaatcagtcgggacaactctaagaacacggcctttctacaaatggactcacttagacccgaggatacaggggtctacttttgtgcacgctactatgacgaccactattccctggattactgggggcagggcacacccgtcaccgtgtcctcggacaaaacacacacgtgtccaccatgtccagcccctgaagccgccggtgggccgagcgtgtttctgtttccccccaaaccgaaagacaccctcatgatcagtcgaacacctgaagtaacctgtgtggttgtggacgtgtcccatgaggacccggaagtcaagtttaactggtatgtagacggtgttgaggttcacaacgccaagaccaaacccagggaagagcagtataacagcacgtatcgtgtcgtgagcgtcctgacagtcctgcatcaggattggctgaatggtaaggagtataagtgcaaagtgagcaacaaggctctgccagcgcccatcgaaaaaaccatttccaaggcaaaagggcagccaagggaaccccaagtgtacacgctgccaccttctagggacgagctgactaaaaatcaggtgtcactgacctgcctggttaagggcttctatcccagtgatattgcggttgagtgggagtctaatggccagccggaaaataactacaagacaactcctcctgttctggactccgatgggtcattcttcctgtattccaaactgactgtggataagagcaggtggcaacagggcaatgtcttctcatgctcggtgatgcatgaggcactgcataaccactacactcagaagtctctgagtctgtctcctgggaaa

SEQ ID NO: 72 - DNA, 2127 bp, synthetic construct
  source 1..2127: mol_type = other DNA
caagtacagctccagcagtcaggagctgagctggtaaaacctgggagtagcgtgaagattagctgcaaagctagtggatacacctttacccgtaacttcatccattggatcaagcaacagcctgggaatgggctcgaatggataggctggatctttccgggggatggggataccgagtacaatcagaagttcaatggcaaggccacactgaccgcagataagtcttcttccaccgcatacatgcagctgtccagccttacaagcgaggattctgccgtttatttttgcgccagaggaaactacaactatgagtactttgactattggggtcaaggtgtgatggtgaccgtctcctccgggggtgggggttcggacattcagatgactcagtcgccttcctcattaagtgcctcagttggggaccgggtaaccattacctgcagcgcatcttcaagcgtctcatacatgaactggtaccaacaaacgccaggcaaagcacccaaacgctggatctatgacacttcaaagctggcttccggggttccttcgcgattttctgggagtggctctggcactgattacaccttcacaatatcctcactgcaacccgaggatatcgccacttattactgccagcagtggtctagcaatcctttcacttttgggcaggggacaaaactccagattacccgaggtggcggcggatcaggtggcggtggcagcggaggcggagggtctgggggaggcgggagccaggtacagcttgtccagtctggcggaggcgttgtccagccaggcaggagtcttcgcttgagctgtaaggcttcaggctacactttcacccggtatactatgcactgggttagacaagccccagggaagggtctggagtggatcggctatatcaatcctagtagggggtacacgaattacaaccagaaagtgaaggaccggtttacaataagcagggacaattcgaaaaacaccgcttttctgcaaatggacagtctgcgacccgaagacacaggcgtgtatttctgtgccagatactatgatgaccactactcgctggattactgggggcagggaacacccgtgaccgtgagtagcggaggagggggctctgacatacaaatgactcagagtcctgcctccttgagcgcatctctgggagaaactgtgtccattgaatgccttgcgagtgaggacatctacagctatctagcctggtatcagcagaagcccggtaaatcacctcaattgctcatttttgccgcgaatcgcctacaggatggagtcccttccaggttcagcggctccggatctggaacacaattcagcctcaagatttcaggcatgcagccggaagatgaaggagattacttctgcctacagggaagcaaattcccctacacattcggacccggtacaaaacttgaactgaacgataagacacacacctgtccaccatgtcctgcaccagaagccgccggcggccctagtgtcttcctgtttcccccgaaaccgaaggacacactcatgatcagcaggactcccgaggtgacatgcgtggtggtcgacgtttcccatgaggacccagaagtcaaattcaattggtatgtggacggggtggaggtgcacaatgcgaagacgaagccacgcgaagagcagtataatagcacctatcgggttgtgtccgtcctcacagtcctgcatcaggattggctgaacggtaaagagtacaagtgcaaggtgagtaacaaggcattgcccgctcccattgagaagacaatctctaaggccaaaggtcagccacgggaaccgcaggtatatacgctcccacccagcagagatgagctgactaagaaccaggtatcactcacgtgtctggtgaaaggcttttatccatccgatattgctgttgaatgggagtcaaatggccagcctgaaaacaactacaagactacgcctccagtgttagactctgatggatccttctttctatattctaaactgaccgtggacaaatcccgttggcagcagggcaacgtgttttcctgttccgtgatgcatgaggctctgcacaaccactacacccagaagagtctgtctctgtcccccggtaaa

SEQ ID NO: 73 - DNA, 2151 bp, synthetic construct
  source 1..2151: mol_type = other DNA
gacattcagatgacacagagtccagcaagtctgtccgcaagccttggtgagactgtaagcatcgagtgcctggccagcgaagacatttattcctatctggcgtggtaccagcagaagccagggaagtcaccccagctcctcatttttgccgctaatcgcttacaggacggcgtgccctcacgattcagcgggagcggaagtggcactcagttttccctgaagatttccggaatgcagccagaagacgaaggggattatttctgcctacaaggatcaaagttcccgtatacgtttggccctggtactaaactggaactgaatggggggggagggtcccaggttcagctggtgcagtcaggagggggagtggttcaaccgggcagatctctgaggttatcctgcaaagctagtggctatacctttacacggtacacaatgcactgggtgaggcaggcacctggtaaggggctggagtggatagggtatatcaatcccagcagaggctatacgaattacaatcagaaggtgaaagaccgctttactataagccgtgacaacagtaagaacaccgcctttctccagatggactcgttgcgaccagaagatacaggggtctatttctgcgccagatactatgacgaccattactccctagactactggggtcaaggaacaccagtcaccgtcagtagcggcggaggaggctctggcggtggcgggtccggtggcggtggttccgggggaggaggatccgatatccagatgacccaaagcccttcttcactctcggcatccgtaggcgatagagtcaccataacatgcagtgcttcaagctccgtgtcctacatgaactggtatcagcaaactcctggtaaagcacccaagaggtggatttacgatacctcaaagctggcctctggcgtaccctccaggttttctggctcgggctccgggacagactatacgttcacgatcagttctctccagcctgaggatattgccacttactactgtcagcagtggagcagcaatccctttaccttcggccagggaacaaagttacagatcacgagaggtggcggcgggagtcaagtgcagctccaacagtctggcgccgaactcgtgaaacccggatctagcgtgaaaatctcatgcaaggccagcggctatacattcacccggaacttcatccactggattaagcaacagcctggaaatggtctagaatggatcggttggatttttccgggagatggagacaccgagtacaaccaaaaattcaacgggaaagcgactctgaccgccgataaatcgagctctacggcttacatgcagctgtcttctctcacttcagaggactcagccgtttacttttgtgctcgcggcaactacaactacgagtactttgattattggggtcagggcgtaatggtgaccgtctcctctctcgaagtgctgttccagggaccagacaaaactcacacatgtccaccttgtcccgctcctgaggccgccgggggcccatcggtctttctgttcccccctaaaccaaaagacaccctgatgatctctcgtacacccgaggtgacctgtgtcgttgtggacgttagccacgaggaccccgaagtgaagttcaactggtatgtggatggcgtggaggttcataatgccaaaacaaagcctcgggaagagcagtataattctacataccgcgttgtatcagtattgaccgtcctgcatcaggattggttgaatggaaaggagtacaagtgcaaggtgtctaacaaggcactgcctgcgcctatagagaagaccatctccaaggctaaagggcaaccacgggaaccacaagtctacacacttccccccagcagggatgaactcaccaaaaaccaggtgagtctgacttgcttggttaaaggcttctacccgtccgatattgccgtcgaatgggagagcaacggacagccggagaacaactataagaccacacctccagtgttggatagcgatgggagcttcttcctttacagtaagctgactgtcgacaagtctcgatggcaacaggggaatgtgtttagctgtagtgtgatgcatgaggcattacacaatcactatactcagaaatccttgagtctatcacccgggaaa

SEQ ID NO: 74 - DNA, 1479 bp, synthetic construct
  source 1..1479: mol_type = other DNA
caggtacagctgcaacagtctggggctgagttagtcaaaccagggtcctcggtgaagatctcttgcaaggcatcaggctacacattcacccgtaatttcattcactggattaagcagcagccaggaaatggcctcgagtggattgggtggatatttcccggggatggagataccgagtacaatcagaagtttaatggaaaggccacactgaccgctgacaagtcgagttcaactgcctatatgcagctgagttccctgaccagcgaggatagcgccgtttatttctgcgcaagagggaactacaactacgagtacttcgactattggggacagggtgtcatggtcacagtgagttctggggggggaggttcaggcggcggagggtctggcggaggcggctctgacattcagatgacacagagtcctgcaagtctgagtgcgtcccttggcgagactgtgtccatcgaatgtctcgcatctgaagacatctactcctatttggcgtggtaccagcaaaagccagggaaatcccctcagttactgatcttcgccgctaataggctgcaagatggagtgcctagccgattttctggtagcggatccggcacccagttctcgctcaagatctccggtatgcagcccgaagatgaaggagactacttctgcttgcagggcagcaagttcccctatacctttggaccggggaccaagttggagctcaatgggggcggaggtagccaggttcagctagttcagtcaggtgggggcgtagtgcaacccggaaggtcccttagactgagttgcaaagcttccggctatacatttacccggtatacgatgcattgggtgagacaagcgccaggcaaaggcttggaatggattggctacatcaacccttctcggggttatacaaactacaaccagaaggtgaaagatcggtttactatcagtcgcgacaacagcaaaaacaccgcatttctgcagatggacagccttagacccgaagacacaggcgtctatttctgtgccaggtattacgacgatcactacagcctagattactggggtcaaggcactcccgtcacagtgtctagcggaggtggaggctcagggggtggcgggtctggtggaggaggcagcgacatacagatgactcagtctcctagctccctttcagccagcgtaggcgatcgcgtgacaatcacttgtagcgccagcagctcagtgtcgtacatgaactggtatcagcagactcctgggaaagcccccaaacgatggatttatgacacatcaaagctggcatcaggggttccaagccgcttttccggcagtggtagtggaaccgactatacgttcacgatctcttccctccaaccagaggatattgccacttactactgtcaacagtggtcatctaatccgtttacctttggccaggggacgaaactccaaattaccaggcaccatcaccaccatcac

SEQ ID NO: 75 - DNA, 1479 bp, synthetic construct
  source 1..1479: mol_type = other DNA
gatatacagatgacccaatcaccagcatctctttccgctagccttggcgaaactgtgtccatcgaatgccttgcctccgaagacatctatagctatctggcctggtatcagcagaaacccggcaagtcacctcagctgctaatcttcgcggccaatagactccaggacggggtaccatctcgttttagcgggtccggctcgggaacacagtttagcctgaagatttcagggatgcagcctgaggacgaaggggactacttctgtctccagggatccaagttcccctacacatttggcccaggtaccaaactggagctgaatggtggggggggctctggaggcggtgggtctgggggcggtggcagtcaagtccagctacagcaaagtggggccgaattggtgaaaccaggcagcagcgtgaaaatctcctgcaaagccagtgggtatacgttcacaaggaacttcatccactggatcaaacagcagcctggcaatggcttagaatggattggctggatttttcccggggatggagacaccgagtataatcagaagttcaacgggaaggccactctcactgcggataagtcatcgagtactgcctatatgcagctgtcctcgctgacttctgaggatagcgctgtgtacttttgtgctcgcggcaactacaactacgagtactttgactactggggacagggtgtaatggtcacagtgtcgtccggcgggggaggatctcaggtacagctggttcaatccggaggaggagtggtgcaaccgggtagatctttgaggctgtcatgcaaggcctccgggtacacatttacccggtataccatgcattgggtgcgacaagcaccgggaaagggtttagagtggatcggatatatcaatcccagcagaggttacaccaattacaaccagaaagtcaaggacagattcaccatcagccgcgataactcaaagaacacggcttttctccagatggattccctgcgaccagaggatactggcgtgtatttctgtgctcggtattacgatgatcactatagtctcgactattggggccagggcacaccagtcaccgtgtctagtgggggagggggctcaggaggagggggatcaggcggcggtggttctgacattcagatgacgcaatctccttctagcttgagtgcttccgttggcgatcgcgtcactattacctgtagcgcaagcagcagtgtgtcctacatgaattggtaccagcaaacgcctggcaaagcaccgaaacggtggatttacgacactagcaagctcgcatcaggagttcccagcaggttttccggaagtggttctggcacagactacacattcaccataagctcccttcagcccgaggacattgccacctactattgccaacagtggtcaagtaaccctttcactttcgggcagggaaccaagctgcaaattaccaggcatcaccaccatcaccat

SEQ ID NO: 76 - DNA, 1479 bp, synthetic construct
  source 1..1479: mol_type = other DNA
caggtgcagctggttcagtctggtggcggagttgtgcagcctggcagatctctgagactgagctgtaaagccagcggctacaccttcaccagatacaccatgcactgggtccgacaggcccctggaaaaggactggaatggatcggctacatcaaccccagccggggctacaccaactacaaccagaaagtgaaggaccggttcaccatcagccgggacaacagcaagaataccgccttcctgcagatggacagcctgaggcctgaagataccggcgtgtacttctgcgcccggtactacgatgaccactacagcctggattactggggccagggcacacctgtgacagtttctagcggaggcggaggaagtggcggcggaggatctggcggtggtggttctgatatccagatgacacagagccctagcagcctgtctgcctctgtgggcgatagagtgaccatcacatgtagcgccagcagcagcgtgtcctacatgaactggtatcagcagacccctggcaaggcccctaagagatggatctacgataccagcaagctggcctccggcgtgccaagcagattttctggctctggcagcggaaccgattacacgttcaccattagctccctgcagccagaggatatcgccacctactactgccagcagtggtccagcaatcccttcacctttggacagggcaccaagctgcagatcacaagaggtggtggtggcagccaggttcagctgcaacaatctggcgccgagctggttaagcctggctctagcgtgaagatctcttgcaaggcctccggatacacattcacccggaacttcatccactggatcaagcagcagcccggcaatggactcgagtggatcggatggattttccccggcgacggcgacaccgagtacaatcagaagttcaacggcaaggccacactgaccgccgataagagcagcagcacagcctacatgcagctgagcagcctgacaagcgaggacagcgccgtgtatttctgtgccagaggcaactacaattacgagtacttcgactattggggacagggcgtgatggttaccgtttcatctggcggaggcggaagcggtggtggtggaagcggaggtggcggctcagatattcagatgacccagtctcctgccagcctgagcgcttctctgggagagacagtgtctatcgagtgcctggccagcgaggatatctacagctacctggcttggtatcaacagaagccaggcaagagccctcagctgctgatcttcgccgccaatagactgcaggatggcgtgccatctagattcagcggctctggctccggcacacagttcagcctgaaaatctctggcatgcagcccgaggacgagggcgattacttttgcctgcaaggcagcaagttcccctacacatttggccctggcacaaagctggaactgaaccaccatcatcaccaccac

SEQ ID NO: 77 - DNA, 1479 bp, synthetic construct
  source 1..1479: mol_type = other DNA
caggtccagctggtgcaatcgggtgggggagtggtgcaacctgggagatccttacggcttagttgcaaagcctccgggtatacgtttactaggtacaccatgcattgggtaagacaggcacctggaaagggactggaatggattggctacatcaaccccagtcgaggatataccaactacaatcagaaggtgaaggataggttcacaattagccgtgacaacagcaagaacaccgcctttctgcagatggattctctaagaccggaggatactggcgtctacttctgtgctcgctattatgacgaccactattccctggattattgggggcaaggcactccagtgaccgttagctctggaggagggggtagcggcggaggaggctctgggggaggggggtctgacatacagatgactcaatcccctagctcactgtcagcatcggttggcgacagagtgaccattacctgtagcgccagctctagtgtcagctacatgaactggtatcagcagacaccaggtaaagccccaaaaaggtggatctacgacacgagcaagttggcctctggtgtgcccagtcgcttctcagggtcaggttccgggactgattacacattcacaatcagctctctccaaccggaagacatagcgacttactattgccagcagtggtcatcgaatccattcacctttggccagggcactaagctacagattacacgggggggaggtggctcagacattcagatgacacaaagtcccgcttctctgagtgcttccctgggagaaaccgtgtctatcgagtgtctcgcgagtgaggacatttactcctatctggcatggtatcaacagaaacctgggaaatccccccagttgctgatctttgccgctaatcgactccaggatggcgtaccttcacgcttcagcggcagcggatccggaacgcagtttagtctcaagatatctgggatgcagccggaagatgagggggactatttctgcttacagggatctaaattcccctatacattcggccctggcaccaagctggagcttaatggcggtgggggtagtggtggtggcggttcgggaggcggtgggtcacaggtgcagcttcagcaatctggcgcagagttggtgaagccaggatcctcagtcaagatcagctgcaaggcttccggctatacctttaccaggaatttcattcactggatcaaacagcaacccggcaatggcctcgaatggatcgggtggatctttcccggggatggcgataccgagtacaaccagaagtttaacggcaaagccactcttacagccgacaaaagcagcagcacagcctacatgcagctctcctcactgacctccgaagactccgctgtgtacttttgcgcacggggaaactacaattacgagtacttcgattactggggccaaggcgtcatggttacggtatccagtcaccatcaccaccatcat

SEQ ID NO: 78 - DNA, 1347 bp, synthetic construct
  source 1..1347: mol_type = other DNA
caggtacagttgcagcaatctggggcagaactggtcaaacccgggagttctgtgaaaatctcctgtaaggccagtggatataccttcacccgtaatttcatccactggatcaaacaacagcctggcaatggcctcgaatggatcggatggatttttcccggtgatggcgataccgagtataaccagaagttcaatgggaaggcaacactaacagccgacaaatcctcatccacagcctatatgcaacttagtagcctcacatctgaagatagcgccgtgtacttttgcgcaaggggcaactataactacgagtatttcgactactggggtcagggggtgatggtgaccgtatcttccgctagtactaaaggacccagcgtgtttccactggcaccatcctctaaatctacaagcggaggcactgccgcacttggctgcctggtcaaagactattttcctgaacccgtcactgtgtcttggaactctggagctttgacatctggcgttcacacttttcccgcagtactccagtcatctggcctgtattctctgtcaagtgttgtgactgttcccagcagtagtctgggaacccagacctacatatgcaacgtcaaccataaacccagcaacacaaaggtggataagcgcgtcgagcctaagagctgcgataagacccatacatgcccaccatgtcccgctccagaggccgccggaggtccatccgtattcttgtttcctcccaaacccaaggataccctgatgatcagccggacacctgaagtcacttgtgtggttgtggacgtatcccatgaagatccagaggtgaagttcaactggtacgtcgacggtgtcgaagtccataatgccaaaaccaaacctagggaggaacagtacaacagtacctaccgagtagtgtcagtcctgactgtgttgcaccaggactggctgaatggtaaggagtacaagtgtaaggtgtccaataaggcccttcctgctcccattgaaaagaccatctccaaagcaaaagggcagccaagagagccccaggtgtatacactgcctccatgcagagaggagatgaccaagaatcaggttagtctgtggtgcctggttaaggggttttatccctcagatattgccgtggagtgggagtccaatggccaacccgagaataactacaagaccacgcctcccgtgcttgacagcgacgggagtttcttcctgtattccaagctgactgttgacaagtcccgttggcagcagggaaacgtgtttagctgttccgtgatgcacgaagccctgcacaaccactacacccagaaaagcctctctctctctccagggaag

SEQ ID NO: 79 - DNA, 2085 bp, synthetic construct
  source 1..2085: mol_type = other DNA
caggtccagttgcagcagagcggcgcggagctggtgaagcctggcagtagcgtcaagatctcttgcaaggcgagtggctataccttcacacggaacttcatccactggataaagcagcaacccggcaatggactagagtggattgggtggattttcccgggagatggcgataccgagtataaccagaagttcaatggtaaggcgacattaaccgccgataagtccagtagtaccgcctatatgcagttgtcttcattgacatctgaagactcagccgtgtatttttgcgctaggggcaactacaactatgagtactttgactactggggacaaggggtgatggtgactgtatcctccgcttccacaaagggtccatccgtatttccccttgctccaagcagcaaatcaacctctggtggtacagctgcccttggatgtcttgttaaggactattttcccgaaccggttacggtaagctggaacagtggcgcactgacatccggcgttcacacctttcctgccgtgcttcaaagtagcggactctattcactgagctccgtagtgaccgtaccatcctcctcccttgggacccagacttacatctgcaatgtgaaccataagccctctaataccaaggtcgacaagcgggtcgaacccaaatcgtgtgataagacccacacttgtcccccgtgtcctgctcctgaagccgcaggcgggccatccgtcttcctcttccctcccaaaccgaaggacacactgatgatctcccgtacgcctgaggtgacatgtgtggttgtcgatgtgagccatgaagatcctgaagtgaagtttaattggtatgttgacggagtcgaagtacacaacgcaaagaccaaacctagggaggagcagtataactccacataccgcgtcgtctcggtcttaactgtcctgcatcaggattggctgaatggcaaagagtacaagtgcaaggtttccaataaggcactacccgccccaatcgagaaaaccatcagcaaagccaaagggcagcctagagagccccaggtgtgcactttgcctcccagtagggaggaaatgaccaaaaatcaagtgtccctcagctgtgccgttaaaggcttttacccatctgacatagctgtggaatgggagtcaaacggacaaccagagaacaactataagacaacaccacccgtgctggactctgacgggtcattctttctggtgagcaaactcaccgtggacaaatctcgctggcaacaggggaatgtgttcagctgcagtgtgatgcatgaagcactgcacaaccactacacgcagaaaagcctctctctgtcacctgggaaagggggaggcggctcccaagttcagctcgttcagtccggagggggagtagtgcagccagggagaagccttcggctgagctgcaaagctagcggctacacttttacgcgatacaccatgcactgggttcgtcaggctcctggcaagggcctggagtggatcggctacatcaatccgagtcgagggtataccaactacaatcagaaagtcaaagatcgcttcacgatctcacgggacaactctaagaatacagcatttctccagatggattctttacggcctgaggatactggcgtgtacttttgcgccagatactatgacgatcactatagcctggactattggggtcaaggcactcccgtgacagtgtcctcagggggaggaggtagtggaggagggggttctgggggtggaggctcagatattcaaatgactcagtcaccctcctctctgagcgcgagcgtcggggacagagtgaccattacatgctctgcctctagtagcgtgagttacatgaactggtatcagcagacccccggaaaagccccaaagaggtggatctacgacacttcaaaactggcttcgggagtcccaagcagattctcaggttcgggctctggtacggattacaccttcaccataagcagtctacagccagaagacattgccacatactactgtcagcaatggtcctctaatcccttcacttttggtcagggcactaagctccagattacaagg

SEQ ID NO: 80 - DNA, 642 bp, synthetic construct
  source 1..642: mol_type = other DNA
gatatacagatgacacagagccccgcaagcctatccgcctccctgggggagacagtgtctatagagtgcttagcttccgaggacatctatagctacttggcttggtatcagcaaaagcctgggaaatcaccacagctgttgatctttgcggccaacaggcttcaggacggagtccctagccggtttagtggatctggctcaggtacacagttcagtctgaagatctccgggatgcagcccgaagacgaaggagactacttctgcttgcagggatctaaattcccatacacttttggccctggcacgaaactggagttaaatcgcactgttgcagctccctcagtgttcatcttccctcccagcgatgagcagctgaaaagtggaactgccagtgttgtgtgcttgctgaacaacttttaccccagggaagccaaggtgcagtggaaggtagacaatgctcttcagtcagggaactctcaggaatccgtgactgagcaagacagcaaggattccacctacagtctcagcagcacactgaccctctccaaagcagactacgagaagcacaaggtgtatgcctgtgaggtaacccatcaagggcttagctccccagtcaccaagagtttcaataggggcgagtgt

SEQ ID NO: 81 - DNA, 2085 bp, synthetic construct
  source 1..2085: mol_type = other DNA
caagttcagcttcaacaaagtggtgcggagctagtgaaacccggatctagtgtcaagatctcttgtaaggcaagcggctatacgtttacccgcaacttcatacactggatcaaacagcaacctggtaatgggctggagtggatcgggtggatttttccgggagatggagacacagagtataatcagaaattcaatggcaaagctactctgacggccgataaaagctccagcacagcctacatgcagttatcttccctgacaagtgaggatagcgccgtgtacttttgcgcaagagggaactacaactacgagtatttcgactattggggccaaggcgtaatggtaaccgtatcctccgccagtacaaagggcccaagtgtgtttccactggcaccgtcttcaaagagcacatcaggtgggactgctgccttgggctgtctggtgaaggactactttccagaacccgtgaccgtgtcctggaatagtggggctttgacaagtggcgttcacacttttcccgctgtactgcagagttcagggctgtatagcttgtcgtccgttgtcactgttcctagcagcagcctaggaacccagacctacatttgcaatgtgaatcacaagccatctaataccaaggtggacaagagggtcgagccaaagtcttgcgacaagactcatacttgtcccccatgtccagcgcctgaagccgctggcggaccctctgtgtttctgttccctccaaagcccaaagatactctcatgatcagccggactccggaggtcacttgtgtcgttgtcgacgtgtcacatgaggatcctgaagtgaagttcaactggtatgtcgatggagtcgaggtgcacaatgccaagaccaaaccccgagaagagcagtacaacagcacataccgggtagtgtccgtgctgaccgtgctccatcaggattggttgaacggtaaggagtacaaatgcaaggtgagcaacaaagctctgccagcacccattgagaagaccatctccaaggccaaagggcagcctagagaaccccaagtgtacaccctccctccaagccgggaagagatgacaaagaatcaggttagcctcacatgccttgtcaagggcttttatccctccgacattgccgtagaatgggagtccaatggccaacccgaaaacaattacaaaaccacaccacccgtcctcgatagcgatggctccttctttctctactccaagttaacggttgacaaaagccggtggcagcaggggaatgtgttcagctgctccgtaatgcacgaggcccttcacaatcactatacccagaaatcgctgtctctttctcccgggaaaggcgggggcggatcacaggtgcaactcgtccagtctgggggaggtgtggtgcaacctggccggagtttacgactgagttgcaaggcatcgggctatacttttaccaggtatactatgcattgggtgagacaggcacccggcaaaggcctagaatggattggctacatcaacccttcaagggggtatactaactacaaccagaaggtgaaagacaggtttaccatatcgcgtgataacagcaaaaacacagccttcctgcagatggactcccttagacctgaagacacaggggtgtatttctgtgctcgttactacgacgaccactatagtctggactactgggggcagggtacaccggttaccgtttctagtggtggaggtggatcaggcggagggggatccggtggaggcggatccgatattcagatgacacagagcccctcttccctttccgcgtcagtgggagacagggtcaccattacctgttccgcctctagctccgtctcatacatgaactggtatcagcagacccctgggaaagcaccaaagcgctggatctatgatacgtcgaagttggcttctggagttccgtcacgcttctcaggatcaggttcaggtaccgactacacttttacgatctcttctctccagcctgaagatatagcgacgtactattgccagcagtggtctagtaaccctttcacattcggccaagggaccaaactgcagatcactcgc

SEQ ID NO: 82 - DNA, 1419 bp, synthetic construct
  source 1..1419: mol_type = other DNA
caggtccagttggtgcaatcgggcggcggcgttgtccagccgggtcgctctctacggctcagctgcaaagcaagtgggtatacctttactcgctatactatgcattgggtacgacaggctcccggtaaaggactggaatggattggctacatcaatcccagtcgcggctatacaaactacaaccaaaaggtcaaagacaggtttacgatttcccgggataactctaagaatacagcctttttgcagatggacagtctgaggccagaggatacaggcgtctacttttgtgccagatactatgacgatcactactcactcgactattggggccaagggacccccgtgactgtgagctcaggaggaggtggatctggcggcggagggagtgggggagggggttccgatatccagatgacccagtcccccagttcactgagcgcttctgtgggcgatcgggtcaccattacatgcagtgccagcagctccgtttcctacatgaattggtaccagcagacacccggaaaagcgccaaaacggtggatctatgacaccagtaaactggcaagcggcgtgcccagtcgattctcgggaagtgggtcaggtaccgactacacatttacgataagcagcctgcagcctgaggacatagccacatactactgccagcagtggtcgtcgaacccgtttactttcggccagggtacgaaactgcagattactcgagagcctaagagctgcgataagacccatacatgcccaccatgtcccgctccagaggccgccggaggtccatccgtattcttgtttcctcccaaacccaaggataccctgatgatcagccggacacctgaagtcacttgtgtggttgtggacgtatcccatgaagatccagaggtgaagttcaactggtacgtcgacggtgtcgaagtccataatgccaaaaccaaacctagggaggaacagtacaacagtacctaccgagtagtgtcagtcctgactgtgttgcaccaggactggctgaatggtaaggagtacaagtgtaaggtgtccaataaggcccttcctgctcccattgaaaagaccatctccaaagcaaaagggcagccaagagagccccaggtgtgtacactgcctccatctagagaggagatgaccaagaatcaggttagtctgagttgcgccgttaaggggttttatccctcagatattgccgtggagtgggagtccaatggccaacccgagaataactacaagaccacgcctcccgtgcttgacagcgacgggagtttcttcctggtttccaagctgactgttgacaagtcccgttggcagcagggaaacgtgtttagctgttccgtgatgcacgaagccctgcacaaccactacacccagaaaagcctctctctctctccagggaag

SEQ ID NO: 83 - DNA, 1422 bp, synthetic construct
  source 1..1422: mol_type = other DNA
caggtacagttgcagcaatctggggcagaactggtcaaacccgggagttctgtgaaaatctcctgtaaggccagtggatataccttcacccgtaatttcatccactggatcaaacaacagcctggcaatggcctcgaatggatcggatggatttttcccggtgatggcgataccgagtataaccagaagttcaatgggaaggcaacactaacagccgacaaatcctcatccacagcctatatgcaacttagtagcctcacatctgaagatagcgccgtgtacttttgcgcaaggggcaactataactacgagtatttcgactactggggtcagggggtgatggtgaccgtatcttccgctagtactaaaggacccagcgtgtttccactggcaccatcctctaaatctacaagcggaggcactgccgcacttggctgcctggtcaaagactattttcctgaacccgtcactgtgtcttggaactctggagctttgacatctggcgttcacacttttcccgcagtactccagtcatctggcctgtattctctgtcaagtgttgtgactgttcccagcagtagtctgggaacccagacctacatatgcaacgtcaaccataaacccagcaacacaaaggtggataagcgcgtcgagcctaagagctgcggaggtggaggctcacaggttcagctagttcagtcaggtgggggcgtagtgcaacccggaaggtcccttagactgagttgcaaagcttccggctatacatttacccggtatacgatgcattgggtgagacaagcgccaggcaaaggcttggaatggattggctacatcaacccttctcggggttatacaaactacaaccagaaggtgaaagatcggtttactatcagtcgcgacaacagcaaaaacaccgcatttctgcagatggacagccttagacccgaagacacaggcgtctatttctgtgccaggtattacgacgatcactacagcctagattactggggtcaaggcactcccgtcacagtgtctagcggaggtggaggctcagggggtggcgggtctggtggaggaggcagcgacatacagatgactcagtctcctagctccctttcagccagcgtaggcgatcgcgtgacaatcacttgtagcgccagcagctcagtgtcgtacatgaactggtatcagcagactcctgggaaagcccccaaacgatggatttatgacacatcaaagctggcatcaggggttccaagccgcttttccggcagtggtagtggaaccgactatacgttcacgatctcttccctccaaccagaggatattgccacttactactgtcaacagtggtcatctaatccgtttacctttggccaggggacgaaactccaaattaccaggcaccatcaccaccatcac

SEQ ID NO: 84 - DNA, 2085 bp, synthetic construct
  source 1..2085: mol_type = other DNA
caggtacagttgcagcaatctggggcagaactggtcaaacccgggagttctgtgaaaatctcctgtaaggccagtggatataccttcacccgtaatttcatccactggatcaaacaacagcctggcaatggcctcgaatggatcggatggatttttcccggtgatggcgataccgagtataaccagaagttcaatgggaaggcaacactaacagccgacaaatcctcatccacagcctatatgcaacttagtagcctcacatctgaagatagcgccgtgtacttttgcgcaaggggcaactataactacgagtatttcgactactggggtcagggggtgatggtgaccgtatcttccgctagtactaaaggacccagcgtgtttccactggcaccatcctctaaatctacaagcggaggcactgccgcacttggctgcctggtcaaagactattttcctgaacccgtcactgtgtcttggaactctggagctttgacatctggcgttcacacttttcccgcagtactccagtcatctggcctgtattctctgtcaagtgttgtgactgttcccagcagtagtctgggaacccagacctacatatgcaacgtcaaccataaacccagcaacacaaaggtggataagcgcgtcgagcctaagagctgcggaggtggaggctcacaggttcagctagttcagtcaggtgggggcgtagtgcaacccggaaggtcccttagactgagttgcaaagcttccggctatacatttacccggtatacgatgcattgggtgagacaagcgccaggcaaaggcttggaatggattggctacatcaacccttctcggggttatacaaactacaaccagaaggtgaaagatcggtttactatcagtcgcgacaacagcaaaaacaccgcatttctgcagatggacagccttagacccgaagacacaggcgtctatttctgtgccaggtattacgacgatcactacagcctagattactggggtcaaggcactcccgtcacagtgtctagcggaggtggaggctcagggggtggcgggtctggtggaggaggcagcgacatacagatgactcagtctcctagctccctttcagccagcgtaggcgatcgcgtgacaatcacttgtagcgccagcagctcagtgtcgtacatgaactggtatcagcagactcctgggaaagcccccaaacgatggatttatgacacatcaaagctggcatcaggggttccaagccgcttttccggcagtggtagtggaaccgactatacgttcacgatctcttccctccaaccagaggatattgccacttactactgtcaacagtggtcatctaatccgtttacctttggccaggggacgaaactccaaattaccagggataagacccatacatgcccaccatgtcccgctccagaggccgccggaggtccatccgtattcttgtttcctcccaaacccaaggataccctgatgatcagccggacacctgaagtcacttgtgtggttgtggacgtatcccatgaagatccagaggtgaagttcaactggtacgtcgacggtgtcgaagtccataatgccaaaaccaaacctagggaggaacagtacaacagtacctaccgagtagtgtcagtcctgactgtgttgcaccaggactggctgaatggtaaggagtacaagtgtaaggtgtccaataaggcccttcctgctcccattgaaaagaccatctccaaagcaaaagggcagccaagagagccccaggtgtatacactgcctccatctagagaggagatgaccaagaatcaggttagtctgacatgcctggttaaggggttttatccctcagatattgccgtggagtgggagtccaatggccaacccgagaataactacaagaccacgcctcccgtgcttgacagcgacgggagtttcttcctgtattccaagctgactgttgacaagtcccgttggcagcagggaaacgtgtttagctgttccgtgatgcacgaagccctgcacaaccactacacccagaaaagcctctctctctctccagggaag

SEQ ID NO: 85 - DNA, 1740 bp, synthetic construct
  source 1..1740: mol_type = other DNA
caggtacagttgcagcaatctggggcagaactggtcaaacccgggagttctgtgaaaatctcctgtaaggccagtggatataccttcacccgtaatttcatccactggatcaaacaacagcctggcaatggcctcgaatggatcggatggatttttcccggtgatggcgataccgagtataaccagaagttcaatgggaaggcaacactaacagccgacaaatcctcatccacagcctatatgcaacttagtagcctcacatctgaagatagcgccgtgtacttttgcgcaaggggcaactataactacgagtatttcgactactggggtcagggggtgatggtgaccgtatcttccgctagtactaaaggacccagcgtgtttccactggcaccatcctctaaatctacaagcggaggcactgccgcacttggctgcctggtcaaagactattttcctgaacccgtcactgtgtcttggaactctggagctttgacatctggcgttcacacttttcccgcagtactccagtcatctggcctgtattctctgtcaagtgttgtgactgttcccagcagtagtctgggaacccagacctacatatgcaacgtcaaccataaacccagcaacacaaaggtggataagcgcgtcgagcctaagagctgcggaggtggaggctcacaggttcagctagttcagtcaggtgggggcgtagtgcaacccggaaggtcccttagactgagttgcaaagcttccggctatacatttacccggtatacgatgcattgggtgagacaagcgccaggcaaaggcttggaatggattggctacatcaacccttctcggggttatacaaactacaaccagaaggtgaaagatcggtttactatcagtcgcgacaacagcaaaaacaccgcatttctgcagatggacagccttagacccgaagacacaggcgtctatttctgtgccaggtattacgacgatcactacagcctagattactggggtcaaggcactcccgtcacagtgtctagcggaggtggaggctcagggggtggcgggtctggtggaggaggcagcgacatacagatgactcagtctcctagctccctttcagccagcgtaggcgatcgcgtgacaatcacttgtagcgccagcagctcagtgtcgtacatgaactggtatcagcagactcctgggaaagcccccaaacgatggatttatgacacatcaaagctggcatcaggggttccaagccgcttttccggcagtggtagtggaaccgactatacgttcacgatctcttccctccaaccagaggatattgccacttactactgtcaacagtggtcatctaatccgtttacctttggccaggggacgaaactccaaattaccagggccgctgcaggcggtgggcagccaagagagccccaggtgtatacactgcctccatctagagaggagatgaccaagaatcaggttagtctgacatgcctggttaaggggttttatccctcagatattgccgtggagtgggagtccaatggccaacccgagaataactacaagaccacgcctcccgtgcttgacagcgacgggagtttcttcctgtattccaagctgactgttgacaagtcccgttggcagcagggaaacgtgtttagctgttccgtgatgcacgaagccctgcacaaccactacacccagaaaagcctctctctctctccagggaag

SEQ ID NO: 86 - DNA, 2103 bp, synthetic construct
  source 1..2103: mol_type = other DNA
caggtacagttgcagcaatctggggcagaactggtcaaacccgggagttctgtgaaaatctcctgtaaggccagtggatataccttcacccgtaatttcatccactggatcaaacaacagcctggcaatggcctcgaatggatcggatggatttttcccggtgatggcgataccgagtataaccagaagttcaatgggaaggcaacactaacagccgacaaatcctcatccacagcctatatgcaacttagtagcctcacatctgaagatagcgccgtgtacttttgcgcaaggggcaactataactacgagtatttcgactactggggtcagggggtgatggtgaccgtatcttccgctagtactaaaggacccagcgtgtttccactggcaccatcctctaaatctacaagcggaggcactgccgcacttggctgcctggtcaaagactattttcctgaacccgtcactgtgtcttggaactctggagctttgacatctggcgttcacacttttcccgcagtactccagtcatctggcctgtattctctgtcaagtgttgtgactgttcccagcagtagtctgggaacccagacctacatatgcaacgtcaaccataaacccagcaacacaaaggtggataagcgcgtcgagcctaagagctgcggaggtggaggctcacaggttcagctagttcagtcaggtgggggcgtagtgcaacccggaaggtcccttagactgagttgcaaagcttccggctatacatttacccggtatacgatgcattgggtgagacaagcgccaggcaaaggcttggaatggattggctacatcaacccttctcggggttatacaaactacaaccagaaggtgaaagatcggtttactatcagtcgcgacaacagcaaaaacaccgcatttctgcagatggacagccttagacccgaagacacaggcgtctatttctgtgccaggtattacgacgatcactacagcctagattactggggtcaaggcactcccgtcacagtgtctagcggaggtggaggctcagggggtggcgggtctggtggaggaggcagcgacatacagatgactcagtctcctagctccctttcagccagcgtaggcgatcgcgtgacaatcacttgtagcgccagcagctcagtgtcgtacatgaactggtatcagcagactcctgggaaagcccccaaacgatggatttatgacacatcaaagctggcatcaggggttccaagccgcttttccggcagtggtagtggaaccgactatacgttcacgatctcttccctccaaccagaggatattgccacttactactgtcaacagtggtcatctaatccgtttacctttggccaggggacgaaactccaaattaccaggggaggtggaggctcacaggtacagttgcagcaatctggggcagaactggtcaaacccgggagttctgtgaaaatctcctgtaaggccagtggatataccttcacccgtaatttcatccactggatcaaacaacagcctggcaatggcctcgaatggatcggatggatttttcccggtgatggcgataccgagtataaccagaagttcaatgggaaggcaacactaacagccgacaaatcctcatccacagcctatatgcaacttagtagcctcacatctgaagatagcgccgtgtacttttgcgcaaggggcaactataactacgagtatttcgactactggggtcagggggtgatggtgaccgtatcttccgctagtactaaaggacccagcgtgtttccactggcaccatcctctaaatctacaagcggaggcactgccgcacttggctgcctggtcaaagactattttcctgaacccgtcactgtgtcttggaactctggagctttgacatctggcgttcacacttttcccgcagtactccagtcatctggcctgtattctctgtcaagtgttgtgactgttcccagcagtagtctgggaacccagacctacatatgcaacgtcaaccataaacccagcaacacaaaggtggataagcgcgtcgagcctaagagctgccaccatcaccaccatcac

SEQ ID NO: 87 - DNA, 1422 bp, synthetic construct
  source 1..1422: mol_type = other DNA
caggttcaactcgtccagagtggaggcggggttgtacagccagggagaagcctcaggcttagttgtaaagcatctggctataccttcacacgctataccatgcactgggtgagacaggctccagggaagggactggagtggatagggtatatcaatccctctcgtggttatacaaactataaccagaaggtgaaggatcggttcactatcagccgagataattcaaagaacacagcatttctgcagatggatagcctgcgacctgaagataccggtgtctacttttgcgccaggtattacgacgatcattatagcttggactactggggccaaggcacccctgtgacggtttccagcggcggaggaggcagtggaggaggaggctccggaggtggcggatctgacatccaaatgacccaaagccccagttctttgagcgcctcagttggagatcgggtgaccattacttgcagcgccagcagtagcgtgtcttacatgaactggtatcagcagaccccggggaaggctccaaagcgctggatctacgatacgtccaagctggcttccggcgtgccctctagattctcagggtctggcagtggtactgactacactttcacgatctcctctttgcagccagaggatatagcgacctactactgtcagcagtggtcctctaatcccttcacttttggtcaaggtaccaagctgcagattacaagaggcggtggaggcagccaggtgcagctccagcagtcaggggccgagctggtaaaaccgggttcatcagtgaagattagctgcaaagcctccggttacacctttacaaggaacttcattcactggatcaagcagcaacccgggaatgggctcgagtggattgggtggatattcccaggggacggagacacagagtacaaccagaaatttaacggcaaagctacactgacagccgacaaatcatcaagtacagcatacatgcagctctcctcactgacttccgaggacagcgcggtgtacttctgtgcgcgcggaaattataactacgaatactttgactattggggtcaaggcgtgatggtaacagtcagttctgcatcaacgaaaggccctagcgtctttcctctggcccctagctctaagtctacttccggcggaacagccgctctggggtgtcttgtcaaggactatttccctgaacccgtcacagtgagctggaatagcggggcccttacttcaggcgtccacacctttcctgctgtgcttcagagttccggcctgtattccctgagttctgtggtcactgttccaagctccagcctggggacccagacctacatctgcaatgtgaatcataaaccgtccaacacgaaagtggataaacgggttgaacccaagagctgccaccatcaccatcatcac

SEQ ID NO: 88 - DNA, 2085 bp, synthetic construct
  source 1..2085: mol_type = other DNA
caggttcaactcgtccagagtggaggcggggttgtacagccagggagaagcctcaggcttagttgtaaagcatctggctataccttcacacgctataccatgcactgggtgagacaggctccagggaagggactggagtggatagggtatatcaatccctctcgtggttatacaaactataaccagaaggtgaaggatcggttcactatcagccgagataattcaaagaacacagcatttctgcagatggatagcctgcgacctgaagataccggtgtctacttttgcgccaggtattacgacgatcattatagcttggactactggggccaaggcacccctgtgacggtttccagcggcggaggaggcagtggaggaggaggctccggaggtggcggatctgacatccaaatgacccaaagccccagttctttgagcgcctcagttggagatcgggtgaccattacttgcagcgccagcagtagcgtgtcttacatgaactggtatcagcagaccccggggaaggctccaaagcgctggatctacgatacgtccaagctggcttccggcgtgccctctagattctcagggtctggcagtggtactgactacactttcacgatctcctctttgcagccagaggatatagcgacctactactgtcagcagtggtcctctaatcccttcacttttggtcaaggtaccaagctgcagattacaagaggcggtggaggcagccaggtgcagctccagcagtcaggggccgagctggtaaaaccgggttcatcagtgaagattagctgcaaagcctccggttacacctttacaaggaacttcattcactggatcaagcagcaacccgggaatgggctcgagtggattgggtggatattcccaggggacggagacacagagtacaaccagaaatttaacggcaaagctacactgacagccgacaaatcatcaagtacagcatacatgcagctctcctcactgacttccgaggacagcgcggtgtacttctgtgcgcgcggaaattataactacgaatactttgactattggggtcaaggcgtgatggtaacagtcagttctgcatcaacgaaaggccctagcgtctttcctctggcccctagctctaagtctacttccggcggaacagccgctctggggtgtcttgtcaaggactatttccctgaacccgtcacagtgagctggaatagcggggcccttacttcaggcgtccacacctttcctgctgtgcttcagagttccggcctgtattccctgagttctgtggtcactgttccaagctccagcctggggacccagacctacatctgcaatgtgaatcataaaccgtccaacacgaaagtggataaacgggttgaacccaagagctgcgataagacccatacatgcccaccatgtcccgctccagaggccgccggaggtccatccgtattcttgtttcctcccaaacccaaggataccctgatgatcagccggacacctgaagtcacttgtgtggttgtggacgtatcccatgaagatccagaggtgaagttcaactggtacgtcgacggtgtcgaagtccataatgccaaaaccaaacctagggaggaacagtacaacagtacctaccgagtagtgtcagtcctgactgtgttgcaccaggactggctgaatggtaaggagtacaagtgtaaggtgtccaataaggcccttcctgctcccattgaaaagaccatctccaaagcaaaagggcagccaagagagccccaggtgtatacactgcctccatctagagaggagatgaccaagaatcaggttagtctgacatgcctggttaaggggttttatccctcagatattgccgtggagtgggagtccaatggccaacccgagaataactacaagaccacgcctcccgtgcttgacagcgacgggagtttcttcctgtattccaagctgactgttgacaagtcccgttggcagcagggaaacgtgtttagctgttccgtgatgcacgaagccctgcacaaccactacacccagaaaagcctctctctctctccagggaag

SEQ ID NO: 89 - DNA, 1740 bp, synthetic construct
  source 1..1740: mol_type = other DNA
caggttcaactcgtccagagtggaggcggggttgtacagccagggagaagcctcaggcttagttgtaaagcatctggctataccttcacacgctataccatgcactgggtgagacaggctccagggaagggactggagtggatagggtatatcaatccctctcgtggttatacaaactataaccagaaggtgaaggatcggttcactatcagccgagataattcaaagaacacagcatttctgcagatggatagcctgcgacctgaagataccggtgtctacttttgcgccaggtattacgacgatcattatagcttggactactggggccaaggcacccctgtgacggtttccagcggcggaggaggcagtggaggaggaggctccggaggtggcggatctgacatccaaatgacccaaagccccagttctttgagcgcctcagttggagatcgggtgaccattacttgcagcgccagcagtagcgtgtcttacatgaactggtatcagcagaccccggggaaggctccaaagcgctggatctacgatacgtccaagctggcttccggcgtgccctctagattctcagggtctggcagtggtactgactacactttcacgatctcctctttgcagccagaggatatagcgacctactactgtcagcagtggtcctctaatcccttcacttttggtcaaggtaccaagctgcagattacaagaggcggtggaggcagccaggtgcagctccagcagtcaggggccgagctggtaaaaccgggttcatcagtgaagattagctgcaaagcctccggttacacctttacaaggaacttcattcactggatcaagcagcaacccgggaatgggctcgagtggattgggtggatattcccaggggacggagacacagagtacaaccagaaatttaacggcaaagctacactgacagccgacaaatcatcaagtacagcatacatgcagctctcctcactgacttccgaggacagcgcggtgtacttctgtgcgcgcggaaattataactacgaatactttgactattggggtcaaggcgtgatggtaacagtcagttctgcatcaacgaaaggccctagcgtctttcctctggcccctagctctaagtctacttccggcggaacagccgctctggggtgtcttgtcaaggactatttccctgaacccgtcacagtgagctggaatagcggggcccttacttcaggcgtccacacctttcctgctgtgcttcagagttccggcctgtattccctgagttctgtggtcactgttccaagctccagcctggggacccagacctacatctgcaatgtgaatcataaaccgtccaacacgaaagtggataaacgggttgaacccaagagctgcgctgcagccggaggcgggcagccaagagagccccaggtgtatacactgcctccatctagagaggagatgaccaagaatcaggttagtctgacatgcctggttaaggggttttatccctcagatattgccgtggagtgggagtccaatggccaacccgagaataactacaagaccacgcctcccgtgcttgacagcgacgggagtttcttcctgtattccaagctgactgttgacaagtcccgttggcagcagggaaacgtgtttagctgttccgtgatgcacgaagccctgcacaaccactacacccagaaaagcctctctctctctccagggaag

SEQ ID NO: 90 - DNA, 684 bp, synthetic construct
  source 1..684: mol_type = other DNA
caggttcagcttcagcagtccggtgcagagctggtgaaaccagggtcatctgtgaagattagctgcaaagcctctggctatacctttacacgcaatttcatccactggatcaagcaacagcctggaaatggcctcgaatggattggctggatctttcctggagatggggataccgagtacaaccagaagttcaatggcaaagccacattgacagccgacaaatcctccagtaccgcctatatgcagctcagctctctgacttcagaggattccgctgtatacttctgtgcgagagggaactacaactatgagtacttcgattattggggtcaaggcgtcatggtgaccgtgagttcagccagcaccaagggaccatctgtgtttccactggcaccctccagcaagagtactagcggtggaactgctgcgttgggatgtctggtgaaggactactttcccgaaccggttactgtgagttggaactcaggcgcccttacgtccggcgtccacacctttcctgctgttctgcaaagctctgggctgtatagcctgtcaagcgtcgtgactgtgccttcctccagtctggggacacagacgtacatttgcaacgtcaatcacaaacccagcaataccaaggtcgacaaacgggttgaacccaagagctgccatcatcaccatcaccat

SEQ ID NO: 91 - DNA, 1380 bp, synthetic construct
  source 1..1380: mol_type = other DNA
caggtgcagctcgtccaaagcggcggaggtgtggtccaaccagggagatccctgaggctgtcctgcaaagccagtgggtacacattcacccgatatacaatgcactgggtacggcaagctcctggcaaaggcctggagtggataggctacatcaatccttcccgtggctatacgaactacaaccagaaagtgaaggaccggtttacgattagcagagacaactctaagaataccgcctttctgcagatggacagtctgcgaccagaggatactggcgtctatttctgtgctcgctattacgatgaccactattccctggattattggggccagggaacacctgtgacagtgagtagcggtggaggtgggtcaggaggtggagggagtggaggcggcggcagcgatatccagatgacgcagagtccttcatctttgtcagcctccgttggggacagggtcaccattacttgctcagccagcagctccgtgtcatacatgaattggtatcaacagactcccggcaaggctccaaaacggtggatttacgatacatccaaactggcaagcggtgtaccctccaggttttctggcagcgggtctggaacagactacaccttcaccattagctccttgcagccagaagatattgcaacctactactgtcagcagtggtctagcaacccctttaccttcgggcagggaaccaagctgcagataactcggggcggcggtggatctgacatccaaatgactcagtccccagctagcctgagtgctagccttggagagactgtgtcaatcgagtgtcttgcctctgaggacatctacagctatctcgcctggtaccaacagaagcccggaaagagccctcagctgctgatctttgccgccaatcgcctccaggatggcgtacctagccgtttctccggatcaggttcagggactcagttttcactgaagatatcaggtatgcagcccgaggacgaaggcgattacttttgcctgcaagggtctaagttcccgtatacttttgggcccggcaccaaattggagctgaacaggacagtcgcggcacctagtgtctttatcttcccacccagcgatgaacagctgaagtctgggaccgcaagcgttgtgtgcctgctgaataacttctatccgagagaagccaaggttcagtggaaagttgacaatgcgttgcagagtggcaatagccaggaatccgtgaccgagcaggattccaaagactccacatactctcttagtagcacactcaccctcagtaaagctgattacgagaagcacaaggtgtatgcctgtgaagtgacccatcaagggctttcttctccggtgacaaaatccttcaacagaggggaatgc

SEQ ID NO: 92 - DNA, 1347 bp, synthetic construct
  source 1..1347: mol_type = other DNA
caggtacagttgcagcaatctggggcagaactggtcaaacccgggagttctgtgaaaatctcctgtaaggccagtggatataccttcacccgtaatttcatccactggatcaaacaacagcctggcaatggcctcgaatggatcggatggatttttcccggtgatggcgataccgagtataaccagaagttcaatgggaaggcaacactaacagccgacaaatcctcatccacagcctatatgcaacttagtagcctcacatctgaagatagcgccgtgtacttttgcgcaaggggcaactataactacgagtatttcgactactggggtcagggggtgatggtgaccgtatcttccgctagtactaaaggacccagcgtgtttccactggcaccatcctctaaatctacaagcggaggcactgccgcacttggctgcctggtcaaagactattttcctgaacccgtcactgtgtcttggaactctggagctttgacatctggcgttcacacttttcccgcagtactccagtcatctggcctgtattctctgtcaagtgttgtgactgttcccagcagtagtctgggaacccagacctacatatgcaacgtcaaccataaacccagcaacacaaaggtggataagcgcgtcgagcctaagagctgcgataagacccatacatgcccaccatgtcccgctccagaggccgccggaggtccatccgtattcttgtttcctcccaaacccaaggataccctgatgatcagccggacacctgaagtcacttgtgtggttgtggacgtatcccatgaagatccagaggtgaagttcaactggtacgtcgacggtgtcgaagtccataatgccaaaaccaaacctagggaggaacagtacaacagtacctaccgagtagtgtcagtcctgactgtgttgcaccaggactggctgaatggtaaggagtacaagtgtaaggtgtccaataaggcccttcctgctcccattgaaaagaccatctccaaagcaaaagggcagccaagagagccccaggtgtatacactgcctccatctagagaggagatgaccaagaatcaggttagtctgacatgcctggttaaggggttttatccctcagatattgccgtggagtgggagtccaatggccaacccgagaataactacaagaccacgcctcccgtgcttgacagcgacgggagtttcttcctgtattccaagctgactgttgacaagtcccgttggcagcagggaaacgtgtttagctgttccgtgatgcacgaagccctgcacaaccactacacccagaaaagcctctctctctctccagggaag

SEQ ID NO: 93 - DNA, 1002 bp, synthetic construct
  source 1..1002: mol_type = other DNA
caggtacagttgcagcaatctggggcagaactggtcaaacccgggagttctgtgaaaatctcctgtaaggccagtggatataccttcacccgtaatttcatccactggatcaaacaacagcctggcaatggcctcgaatggatcggatggatttttcccggtgatggcgataccgagtataaccagaagttcaatgggaaggcaacactaacagccgacaaatcctcatccacagcctatatgcaacttagtagcctcacatctgaagatagcgccgtgtacttttgcgcaaggggcaactataactacgagtatttcgactactggggtcagggggtgatggtgaccgtatcttccgctagtactaaaggacccagcgtgtttccactggcaccatcctctaaatctacaagcggaggcactgccgcacttggctgcctggtcaaagactattttcctgaacccgtcactgtgtcttggaactctggagctttgacatctggcgttcacacttttcccgcagtactccagtcatctggcctgtattctctgtcaagtgttgtgactgttcccagcagtagtctgggaacccagacctacatatgcaacgtcaaccataaacccagcaacacaaaggtggataagcgcgtcgagcctaagagctgcgctgcagccggaggcgggcagccaagagagccccaggtgtatacactgcctccatctagagaggagatgaccaagaatcaggttagtctgacatgcctggttaaggggttttatccctcagatattgccgtggagtgggagtccaatggccaacccgagaataactacaagaccacgcctcccgtgcttgacagcgacgggagtttcttcctgtattccaagctgactgttgacaagtcccgttggcagcagggaaacgtgtttagctgttccgtgatgcacgaagccctgcacaaccactacacccagaaaagcctctctctctctccagggaag

SEQ ID NO: 94 - protein, 119 aa, synthetic construct
QVQLVQSGAEVKKPGASVKVSCKASGYTFTRNFIHWVRQAPGQGLEWMGWIFPGDGDTEYNQKFNGRVTMTRDTSISTAYMELSRLRSDDTAVYYCARGNYNYEYFDYWGQGTMVTVSS

SEQ ID NO: 95 - protein, 119 aa, synthetic construct
QVQLQESGAEVKKPGASVKVSCKASGYTFTRNFIHWVRQAPGQRLEWMGWIFPGDGDTEYNQKFNGRVTITRDTSASTAYMELSSLRSEDTAVYYCARGNYNYEYFDYWGQGTLVTVSS

SEQ ID NO: 96 - protein, 119 aa, synthetic construct
QVQLVQSGAEVKKPGASVKISCKASGYTFTRNFIHWVRQAPGQSLEWVGWIFPGDGDTEYNQKFNGRITITRDTSANTAYMELSSLKSEDTAVYYCARGNYNYEYFDYWGQGTLVTVSS

SEQ ID NO: 97 - protein, 119 aa, synthetic construct
QMQLVQSGAEVKKTGSSVKVSCKASGYTFTRNFIHWVRQAPGQALEWMGWIFPGDGDTEYNQKFNGRVTITRDRSMSTAYMELSSLRSEDTAMYYCARGNYNYEYFDYWGQGTLVTVSS

SEQ ID NO: 98 - protein, 119 aa, synthetic construct
QVQLVQSGAEVKKPGSSVKVSCKASGYTFTRNFIHWVRQQPGQGLEWMGWIFPGDGDTEYNQKFNGRVTITADKSTSTAYMQLSSLTSEDTAVYFCARGNYNYEYFDYWGQGVMVTVSS

SEQ ID NO: 99 - protein, 107 aa, synthetic construct
DIQMTQSPSFVSASVGDRVTITCLASEDIYSYLAWYQQKPGKAPKLLIFAANRLQDGVPSRFSGGGSGTGFTLTISSLQPEDFATYFCLQGSKFPYTFGQGTKLEIN

SEQ ID NO: 100 - protein, 107 aa, synthetic construct
DIQLTQSPAFLSASLGDRVTITCLASEDIYSYLAWYQQKPGKAPKLLISAANRLQDGVPSRFSGSGSGTEFTLTISSLQPEDFATYSCLQGSKFPYTFGQGTKLEIK

SEQ ID NO: 101 - protein, 107 aa, synthetic construct
DIQLTQSPSSLSASVGDRVTITCLASEDIYSYLAWYQQKPGKGPKLLIYAANRLQDGVPSRFSGSGSGTDFSLTISSLQPEDLATYYCLQGSKFPYTFGGGTKVEIK

SEQ ID NO: 102 - protein, 107 aa, synthetic construct
DIQMTQSPSSLSASVGDTVTIACLASEDIYSYLAWYQQKPGKAPKLLIYAANRLQDGVPSRFSGSGSFTDFTLTINSLQPDDSATYYCLQGSKFPYTFGGGTKVDIK

SEQ ID NO: 103 - protein, 107 aa, synthetic construct
DIQMTQSPSSVSASVGDSVTIECLASEDIYSYLAWYQQKPGKSPKLLIFAANRLQDGVPSRFSGSGSGTQFTLKISSLQPEDFAEYFCLQASKFPYTFGPGTKLELN

SEQ ID NO: 104 - DNA, 357 bp, synthetic construct
  source 1..357: mol_type = other DNA
caggttcagctcgttcagtctggcgcggaagtcaagaaaccaggagcgtctgtgaaagtgagttgcaaagcatccggttacacgtttacccgcaacttcattcactgggttaggcaagcacctggccaagggttggagtggatgggatggatttttcctggagatggcgacactgagtacaaccagaagttcaatggcagagtgacaatgacacgcgatacatccatcagtacagcctacatggagctatcccggttacggtccgatgacactgccgtgtactactgtgccagagggaattacaactacgagtacttcgactattggggacaggggactatggtaaccgtgtcctca

SEQ ID NO: 105 - DNA, 357 bp, synthetic construct
  source 1..357: mol_type = other DNA
caggttcagctgcaagaatcaggcgccgaagtcaagaaaccgggagcaagcgttaaggtgagttgtaaagcgtctggctatacattcacccgtaattttatccattgggtgagacaggcccctggccagcgcttagagtggatgggctggattttccccggcgacggcgatacggagtataaccagaagttcaatggacgggtgacaatcacaagagacactagcgcctcaaccgcgtacatggagctgagttccctccgatcagaggatacagccgtttactactgcgcaagggggaattacaactacgagtacttcgactattgggggcaggggactcttgtgacggtttcgtcc

SEQ ID NO: 106 - DNA, 357 bp, synthetic construct
  source 1..357: mol_type = other DNA
caagtccagctggtacagtccggtgctgaagtaaagaaaccaggcgcctcagttaagatcagctgcaaggcttctggttacaccttcactcgcaacttcatccactgggtgagacaagcccctgggcagtctctcgaatgggttggctggatatttcccggggacggagatactgaatacaaccaaaagttcaatggccggattaccataacacgagatacttctgcgaatactgcctatatggaactgagctctcttaaaagcgaggacactgcagtctactattgcgctagagggaattacaattacgagtactttgactactggggacagggaacactggtgacagttagctcc

SEQ ID NO: 107 - DNA, 357 bp, synthetic construct
  source 1..357: mol_type = other DNA
cagatgcagctcgtacagagcggtgccgaggtgaagaaaaccgggagcagcgttaaagtctcctgtaaagcctccggctacacctttacccggaatttcatccattgggtacggcaggcacccggccaagcactggaatggatggggtggatattcccgggtgacggagatactgagtacaaccagaagttcaatggaagagtgactattacgagagatcgctcaatgagtactgcgtatatggaactgtcctcattgcgcagcgaagatacggcgatgtattactgtgcacgcgggaactacaactacgagtacttcgattactggggccaagggacccttgtcacggtttcatcc

SEQ ID NO: 108 - DNA, 357 bp, synthetic construct
  source 1..357: mol_type = other DNA
caggttcaactggttcagtcaggtgcagaggtaaagaagccagggagctcagtgaaagtctcatgcaaagccagcggatacacctttactcggaactttatccactgggtgagacagcagcctgggcaaggcttggagtggatgggctggatctttccaggcgatggagacaccgagtataaccagaagttcaatggcagagtgactattaccgccgataaaagcacatctacagcctatatgcagctgagcagcctgacaagtgaagataccgccgtctacttctgtgccagaggcaactacaactacgagtatttcgactactggggtcagggggtaatggtcacggtgagcagt

SEQ ID NO: 109 - DNA, 321 bp, synthetic construct
  source 1..321: mol_type = other DNA
gacatccagatgacccaatccccttcattcgtgagtgcctcagtgggcgacagagtcaccattacgtgtcttgcttcagaggacatttacagctatctcgcatggtatcagcagaaacctgggaaagcacccaaactgctgatattcgctgccaatcggctgcaagatggcgtaccatccaggttttctggaggaggatctggtactgggtttaccctgactatcagctcccttcagcccgaggattttgccacatacttctgcctccaaggcagcaaattcccgtacacatttgggcagggtaccaagctggagatcaac

SEQ ID NO: 110 - DNA, 321 bp, synthetic construct
  source 1..321: mol_type = other DNA
gacattcagctcactcagagtcctgcgtttctgtccgcatcacttggcgacagagtcaccatcacttgcttggccagtgaggacatctacagctatctggcttggtaccagcagaaacccggaaaagccccgaagctgttgatctctgctgcgaatcggttgcaggatggagtaccatcacgcttctcaggctctggaagcggtacagagttcacccttaccattagctctctccaacccgaagattttgccacctactcttgcctgcaagggagcaaattcccctatacctttggccaagggaccaaactggagattaag

SEQ ID NO: 111 - DNA, 321 bp, synthetic construct
  source 1..321: mol_type = other DNA
gacattcagctgacccagtcaccaagctcactgagtgcttctgtgggtgatcgtgtgacgattacttgcctggctagtgaggacatctacagctacttggcctggtatcagcagaaacctgggaaaggccccaagctgctgatctacgctgccaataggctgcaagacggggtacctagccgcttttccggatctggctcaggcacagacttcagccttaccatatccagcctccaaccagaggatcttgccacctattactgccttcagggctccaagtttccctacacgtttggaggtggtactaaggtggagatcaaa

SEQ ID NO: 112 - DNA, 321 bp, synthetic construct
  source 1..321: mol_type = other DNA
gacatccagatgactcaatccccaagcagtctgagcgcctctgtaggcgataccgtgacgattgcgtgtctggcttccgaggacatctacagttacctcgcatggtatcagcagaaaccggggaaagcacctaagctgctgatttatgcggctaacagactgcaggatggcgtacccagtcgcttctcaggttccggcagctttaccgactttaccctgaccatcaacagccttcagcccgatgatagcgccacttactactgtctgcaaggctctaagttcccctatacgtttggaggaggcactaaggtcgacataaag

SEQ ID NO: 113 - DNA, 321 bp, synthetic construct
  source 1..321: mol_type = other DNA
gatatccagatgacacagagccctagcagcgttagcgcatcagtaggggacagtgtgaccattgaatgccttgcaagcgaggacatctacagctatttggcgtggtatcagcaaaagccaggcaaatctcccaaactgctcattttcgccgccaataggctccaagatggtgtcccttcccgattttccgggtcaggctcaggaacccagttcacactgaagatttcctctcttcagccagaggactttgcagagtacttctgtctccaggccagtaagtttccctacacctttgggcctggaacgaaactggaactgaat

SEQ ID NO: 114 - protein, 472 aa, synthetic construct
QVTLKESGPVLVKPTETLTLTCTVSGYSITSDYAWNWIRQPPGKALEWLAYISYSGSTSYNPSLKSRLSITKDTSKSQVVLTMTNMDPVDTATYYCARDPPYYYGSWGQGTTVTVSSASTKGPSVFPLAPSSKSTSGGTAALGCLVKDYFPEPVTVSWNSGALTSGVHTFPAVLQSSGLYSLSSVVTVPSSSLGTQTYICNVNHKPSNTKVDKRVEPKSCGGGGSQVQLVQSGGGVVQPGRSLRLSCKASGYTFTRYTMHWVRQAPGKGLEWIGYINPSRGYTNYNQKVKDRFTISRDNSKNTAFLQMDSLRPEDTGVYFCARYYDDHYSLDYWGQGTPVTVSSGGGGSGGGGSGGGGSDIQMTQSPSSLSASVGDRVTITCSASSSVSYMNWYQQTPGKAPKRWIYDTSKLASGVPSRFSGSGSGTDYTFTISSLQPEDIATYYCQQWSSNPFTFGQGTKLQITRHHHHHH

SEQ ID NO: 115 - protein, 219 aa, synthetic construct
DVVMTQSPLSLPVTLGQPASISCKSSQSLLDSDGKTYLNWLQQRPGQSPRRLIYLVSKLDSGVPDRFSGSGSGTDFTLKISRVEAEDVGVYHCWQGTHFPYTFGGGTKVEIKRTVAAPSVFIFPPSDEQLKSGTASVVCLLNNFYPREAKVQWKVDNALQSGNSQESVTEQDSKDSTYSLSSTLTLSKADYEKHKVYACEVTHQGLSSPVTKSFNRGEC

SEQ ID NO: 116 - protein, 468 aa, synthetic construct
QVQLVQSGAEVKKPGASVKVSCKASGYSFTGYYIHWVRQAPGQGLEWIGYISAYNGASSYNQKFKGRATFTVDTSISTAYMELSRLRSDDTAVYYCASSMDYWGQGTLVTVSSASTKGPSVFPLAPSSKSTSGGTAALGCLVKDYFPEPVTVSWNSGALTSGVHTFPAVLQSSGLYSLSSVVTVPSSSLGTQTYICNVNHKPSNTKVDKRVEPKSCGGGGSQVQLVQSGGGVVQPGRSLRLSCKASGYTFTRYTMHWVRQAPGKGLEWIGYINPSRGYTNYNQKVKDRFTISRDNSKNTAFLQMDSLRPEDTGVYFCARYYDDHYSLDYWGQGTPVTVSSGGGGSGGGGSGGGGSDIQMTQSPSSLSASVGDRVTITCSASSSVSYMNWYQQTPGKAPKRWIYDTSKLASGVPSRFSGSGSGTDYTFTISSLQPEDIATYYCQQWSSNPFTFGQGTKLQITRHHHHHH

SEQ ID NO: 117 - protein, 219 aa, synthetic construct
DVVMTQSPLSLPVTLGQPASISCKSSQSLLDSDGKTYLNWLQQRPGQSPKRLIYLVSKLDSGVPDRFSGSGSGTDFTLKISRVEAEDVGVYHCWQGTHFPYTFGQGTKLEIKRTVAAPSVFIFPPSDEQLKSGTASVVCLLNNFYPREAKVQWKVDNALQSGNSQESVTEQDSKDSTYSLSSTLTLSKADYEKHKVYACEVTHQGLSSPVTKSFNRGEC

SEQ ID NO: 118 - protein, 471 aa, synthetic construct
DVQLKLQESGPGLVKNSQSLSLTCTVTGYSITSDYAWNWIRQFPGNKLEWMGYISYSGSTSYNPSLKSRISITRDTSKNQFFLQLNSVTPEDTATYYCARDPPYYYGSNGTLTVSSASTKGPSVFPLAPSSKSTSGGTAALGCLVKDYFPEPVTVSWNSGALTSGVHTFPAVLQSSGLYSLSSVVTVPSSSLGTQTYICNVNHKPSNTKVDKRVEPKSCGGGGSQVQLVQSGGGVVQPGRSLRLSCKASGYTFTRYTMHWVRQAPGKGLEWIGYINPSRGYTNYNQKVKDRFTISRDNSKNTAFLQMDSLRPEDTGVYFCARYYDDHYSLDYWGQGTPVTVSSGGGGSGGGGSGGGGSDIQMTQSPSSLSASVGDRVTITCSASSSVSYMNWYQQTPGKAPKRWIYDTSKLASGVPSRFSGSGSGTDYTFTISSLQPEDIATYYCQQWSSNPFTFGQGTKLQITRHHHHHH

SEQ ID NO: 119 - protein, 219 aa, synthetic construct
DVVMTQTPLTLSVTIGQPASISCKSSQSLLDSDGKTYLNWLLQRPGQSPKRLIYLVSKLDSGVPDRFTGSGSGTDFTLKISRVEAEDLGVYHCWQGTHFPYTFGGGTKLEIKRTVAAPSVFIFPPSDEQLKSGTASVVCLLNNFYPREAKVQWKVDNALQSGNSQESVTEQDSKDSTYSLSSTLTLSKADYEKHKVYACEVTHQGLSSPVTKSFNRGEC

SEQ ID NO: 120 - protein, 474 aa, synthetic construct
QVQLVQSGAEVKKPGASVKVSCKASGYTFTRNFIHWVRQAPGQGLEWMGWIFPGDGDTEYNQKFNGRVTMTRDTSISTAYMELSRLRSDDTAVYYCARGNYNYEYFDYWGQGTMVTVSSASTKGPSVFPLAPSSKSTSGGTAALGCLVKDYFPEPVTVSWNSGALTSGVHTFPAVLQSSGLYSLSSVVTVPSSSLGTQTYICNVNHKPSNTKVDKRVEPKSCGGGGSQVQLVQSGGGVVQPGRSLRLSCKASGYTFTRYTMHWVRQAPGKGLEWIGYINPSRGYTNYNQKVKDRFTISRDNSKNTAFLQMDSLRPEDTGVYFCARYYDDHYSLDYWGQGTPVTVSSGGGGSGGGGSGGGGSDIQMTQSPSSLSASVGDRVTITCSASSSVSYMNWYQQTPGKAPKRWIYDTSKLASGVPSRFSGSGSGTDYTFTISSLQPEDIATYYCQQWSSNPFTFGQGTKLQITRHHHHHH

SEQ ID NO: 121 - protein, 474 aa, synthetic construct
QVQLQESGAEVKKPGASVKVSCKASGYTFTRNFIHWVRQAPGQRLEWMGWIFPGDGDTEYNQKFNGRVTITRDTSASTAYMELSSLRSEDTAVYYCARGNYNYEYFDYWGQGTLVTVSSASTKGPSVFPLAPSSKSTSGGTAALGCLVKDYFPEPVTVSWNSGALTSGVHTFPAVLQSSGLYSLSSVVTVPSSSLGTQTYICNVNHKPSNTKVDKRVEPKSCGGGGSQVQLVQSGGGVVQPGRSLRLSCKASGYTFTRYTMHWVRQAPGKGLEWIGYINPSRGYTNYNQKVKDRFTISRDNSKNTAFLQMDSLRPEDTGVYFCARYYDDHYSLDYWGQGTPVTVSSGGGGSGGGGSGGGGSDIQMTQSPSSLSASVGDRVTITCSASSSVSYMNWYQQTPGKAPKRWIYDTSKLASGVPSRFSGSGSGTDYTFTISSLQPEDIATYYCQQWSSNPFTFGQGTKLQITRHHHHHH

SEQ ID NO: 122 - protein, 474 aa, synthetic construct
QVQLVQSGAEVKKPGASVKISCKASGYTFTRNFIHWVRQAPGQSLEWVGWIFPGDGDTEYNQKFNGRITITRDTSANTAYMELSSLKSEDTAVYYCARGNYNYEYFDYWGQGTLVTVSSASTKGPSVFPLAPSSKSTSGGTAALGCLVKDYFPEPVTVSWNSGALTSGVHTFPAVLQSSGLYSLSSVVTVPSSSLGTQTYICNVNHKPSNTKVDKRVEPKSCGGGGSQVQLVQSGGGVVQPGRSLRLSCKASGYTFTRYTMHWVRQAPGKGLEWIGYINPSRGYTNYNQKVKDRFTISRDNSKNTAFLQMDSLRPEDTGVYFCARYYDDHYSLDYWGQGTPVTVSSGGGGSGGGGSGGGGSDIQMTQSPSSLSASVGDRVTITCSASSSVSYMNWYQQTPGKAPKRWIYDTSKLASGVPSRFSGSGSGTDYTFTISSLQPEDIATYYCQQWSSNPFTFGQGTKLQITRHHHHHH

SEQ ID NO: 123 - protein, 474 aa, synthetic construct
QMQLVQSGAEVKKTGSSVKVSCKASGYTFTRNFIHWVRQAPGQALEWMGWIFPGDGDTEYNQKFNGRVTITRDRSMSTAYMELSSLRSEDTAMYYCARGNYNYEYFDYWGQGTLVTVSSASTKGPSVFPLAPSSKSTSGGTAALGCLVKDYFPEPVTVSWNSGALTSGVHTFPAVLQSSGLYSLSSVVTVPSSSLGTQTYICNVNHKPSNTKVDKRVEPKSCGGGGSQVQLVQSGGGVVQPGRSLRLSCKASGYTFTRYTMHWVRQAPGKGLEWIGYINPSRGYTNYNQKVKDRFTISRDNSKNTAFLQMDSLRPEDTGVYFCARYYDDHYSLDYWGQGTPVTVSSGGGGSGGGGSGGGGSDIQMTQSPSSLSASVGDRVTITCSASSSVSYMNWYQQTPGKAPKRWIYDTSKLASGVPSRFSGSGSGTDYTFTISSLQPEDIATYYCQQWSSNPFTFGQGTKLQITRHHHHHH

SEQ ID NO: 124 - protein, 474 aa, synthetic construct
QVQLVQSGAEVKKPGSSVKVSCKASGYTFTRNFIHWVRQQPGQGLEWMGWIFPGDGDTEYNQKFNGRVTITADKSTSTAYMQLSSLTSEDTAVYFCARGNYNYEYFDYWGQGVMVTVSSASTKGPSVFPLAPSSKSTSGGTAALGCLVKDYFPEPVTVSWNSGALTSGVHTFPAVLQSSGLYSLSSVVTVPSSSLGTQTYICNVNHKPSNTKVDKRVEPKSCGGGGSQVQLVQSGGGVVQPGRSLRLSCKASGYTFTRYTMHWVRQAPGKGLEWIGYINPSRGYTNYNQKVKDRFTISRDNSKNTAFLQMDSLRPEDTGVYFCARYYDDHYSLDYWGQGTPVTVSSGGGGSGGGGSGGGGSDIQMTQSPSSLSASVGDRVTITCSASSSVSYMNWYQQTPGKAPKRWIYDTSKLASGVPSRFSGSGSGTDYTFTISSLQPEDIATYYCQQWSSNPFTFGQGTKLQITRHHHHHH

SEQ ID NO: 125 - protein, 214 aa, synthetic construct
DIQMTQSPSFVSASVGDRVTITCLASEDIYSYLAWYQQKPGKAPKLLIFAANRLQDGVPSRFSGGGSGTGFTLTISSLQPEDFATYFCLQGSKFPYTFGQGTKLEINRTVAAPSVFIFPPSDEQLKSGTASVVCLLNNFYPREAKVQWKVDNALQSGNSQESVTEQDSKDSTYSLSSTLTLSKADYEKHKVYACEVTHQGLSSPVTKSFNRGEC

SEQ ID NO: 126 - protein, 214 aa, synthetic construct
DIQLTQSPAFLSASLGDRVTITCLASEDIYSYLAWYQQKPGKAPKLLISAANRLQDGVPSRFSGSGSGTEFTLTISSLQPEDFATYSCLQGSKFPYTFGQGTKLEIKRTVAAPSVFIFPPSDEQLKSGTASVVCLLNNFYPREAKVQWKVDNALQSGNSQESVTEQDSKDSTYSLSSTLTLSKADYEKHKVYACEVTHQGLSSPVTKSFNRGEC

SEQ ID NO: 127 - protein, 214 aa, synthetic construct
DIQLTQSPSSLSASVGDRVTITCLASEDIYSYLAWYQQKPGKGPKLLIYAANRLQDGVPSRFSGSGSGTDFSLTISSLQPEDLATYYCLQGSKFPYTFGGGTKVEIKRTVAAPSVFIFPPSDEQLKSGTASVVCLLNNFYPREAKVQWKVDNALQSGNSQESVTEQDSKDSTYSLSSTLTLSKADYEKHKVYACEVTHQGLSSPVTKSFNRGEC

SEQ ID NO: 128 - protein, 214 aa, synthetic construct
DIQMTQSPSSLSASVGDTVTIACLASEDIYSYLAWYQQKPGKAPKLLIYAANRLQDGVPSRFSGSGSFTDFTLTINSLQPDDSATYYCLQGSKFPYTFGGGTKVDIKRTVAAPSVFIFPPSDEQLKSGTASVVCLLNNFYPREAKVQWKVDNALQSGNSQESVTEQDSKDSTYSLSSTLTLSKADYEKHKVYACEVTHQGLSSPVTKSFNRGEC

SEQ ID NO: 129 - protein, 214 aa, synthetic construct
DIQMTQSPSSVSASVGDSVTIECLASEDIYSYLAWYQQKPGKSPKLLIFAANRLQDGVPSRFSGSGSGTQFTLKISSLQPEDFAEYFCLQASKFPYTFGPGTKLELNRTVAAPSVFIFPPSDEQLKSGTASVVCLLNNFYPREAKVQWKVDNALQSGNSQESVTEQDSKDSTYSLSSTLTLSKADYEKHKVYACEVTHQGLSSPVTKSFNRGEC

SEQ ID NO: 130 - protein, 17 aa, synthetic construct
WIFPGDADTEYNQKFSG

SEQ ID NO: 131 - protein, 7 aa, synthetic construct
AANRLQS

SEQ ID NO: 132 - protein, 17 aa, synthetic construct
YINPSMGATNYNQKVKD

SEQ ID NO: 133 - protein, 10 aa, synthetic construct
YYNDHYSLDY

SEQ ID NO: 134 - protein, 10 aa, synthetic construct
YYDDHFSLDY

SEQ ID NO: 135 - protein, 10 aa, synthetic construct
SASSSVAYMN

SEQ ID NO: 136 - protein, 7 aa, synthetic construct
NTSKLAS

SEQ ID NO: 137 - protein, 119 aa, synthetic construct
QMQLVQSGAEVKKTGSSVKVSCKASGYTFTRNFIHWVRQAPGQALEWMGWIFPGDADTEYNQKFSGRVTITRDRSMSTAYMELSSLRSEDTAMYYCARGNYNYEYFDYWGQGTLVTVSS

SEQ ID NO: 138 - protein, 119 aa, synthetic construct
QVQLVQSGAEVKKPGSSVKVSCKASGYTFTRNFIHWIRQAPGQGLEWIGWIFPGDADTEYNQKFSGRATITADKSTSTAYMELSSLRSEDTAVYYCARGNYNYEYFDYWGQGTMVTVSS

SEQ ID NO: 139 - protein, 119 aa, synthetic construct
QVQLVQSGAEVKKPGSSVKVSCKASGYTFTRNFIHWIRQAPGQGLEWIGWIFPGDADTEYNQKFSGRVTITADKSTSTAYMELSSLRSEDTAVYYCARGNYNYEYFDYWGQGTMVTVSS

SEQ ID NO: 140 - protein, 119 aa, synthetic construct
QVQLVQSGAEVKKPGSSVKVSCKASGYTFTRNFIHWIRQAPGQGLEWIGWIFPGDGDTEYNQKFNGRATITADKSTSTAYMELSSLRSEDTAVYYCARGNYNYEYFDYWGQGTMVTVSS

SEQ ID NO: 141 - protein, 107 aa, synthetic construct
DIQMTQSPSFVSASVGDRVTITCLASEDIYSYLAWYQQKPGKAPKLLIFAANRLQSGVPSRFSGGGSGTGFTLTISSLQPEDFATYFCLQGSKFPYTFGQGTKLEIN

SEQ ID NO: 142 - protein, 107 aa, synthetic construct
DIQMTQSPSFVSASVGDRVTITCLASEDIYSYLAWYQQKPGKAPKLLIFAANRLQSGVPSRFSGGGSGTGFTLTISSLQPEDFATYFCLQGSKFPYTFGQGTKLEIK

SEQ ID NO: 143 - protein, 107 aa, synthetic construct
DIQMTQSPSFVSASVGDRVTITCLASEDIYSYLAWYQQKPGKAPKLLIFAANRLQDGVPSRFSGGGSGTGFTLTISSLQPEDFATYFCLQGSKFPYTFGQGTKLEIK

SEQ ID NO: 144 - protein, 107 aa, synthetic construct
DIQMTQSPSSLSASVGDRVTITCLASEDIYSYLAWYQQKPGKAPKLLIFAANRLQDGVPSRFSGSGSGTDFTLTISSLQPEDFATYYCLQGSKFPYTFGPGTKVDIK

SEQ ID NO: 145 - protein, 107 aa, synthetic construct
DIQMTQSPSSLSASVGDRVTITCLASEDIYSYLAWYQQKPGKAPKLLIFAANRLQSGVPSRFSGSGSGTDFTLTISSLQPEDFATYYCLQGSKFPYTFGPGTKVDIK

SEQ ID NO: 146 - DNA, 357 bp, synthetic construct
  source 1..357: mol_type = other DNA
caaatgcagctcgtacagtcgggagcagaagtcaagaagaccggcagctcagttaaggtgtcgtgcaaagcctctggatatacattcacgcggaatttcattcactgggtgagacaggcaccaggccaggccttggaatggatgggctggatttttcctggggatgccgacacagagtataaccagaaattctcgggcagggtaacaattactcgggatagatcaatgtctacggcgtatatggagctcagcagcctgagatccgaagatacagccatgtattactgtgccagaggcaattacaattatgagtacttcgactattggggccaagggacactggtcaccgtttcatcc

SEQ ID NO: 147 - DNA, 357 bp, synthetic construct
  source 1..357: mol_type = other DNA
caagttcagctggttcaatctggggctgaagtcaagaagcctgggtcctcagtgaaagtttcctgcaaggcttctggctacaccttcacccgtaactttatccactggatcagacaggcacctggacaaggccttgagtggattgggtggatttttcctggagatgcagatacagagtacaatcaaaagttcagtgggagagcaacaatcacagcagacaaatcaaccagcacagcctatatggagctcagcagcctgagatctgaggacactgcagtctattactgtgcaagaggaaattacaactacgagtactttgattactggggccaaggaaccatggtcacagtctcctca

SEQ ID NO: 148 - DNA, 357 bp, synthetic construct
  source 1..357: mol_type = other DNA
caagttcagctggttcaatctggggctgaagtcaagaagcctgggtcctcagtgaaagtttcctgcaaggcttctggctacaccttcacccgtaactttatccactggatcagacaggcacctggacaaggccttgagtggattgggtggatttttcctggagatgcagatacagagtacaatcaaaagttcagtgggagagtgacaatcacagcagacaaatcaaccagcacagcctatatggagctcagcagcctgagatctgaggacactgcagtctattactgtgcaagaggaaattacaactacgagtactttgattactggggccaaggaaccatggtcacagtctcctca

SEQ ID NO: 149 - DNA, 357 bp, synthetic construct
  source 1..357: mol_type = other DNA
caagttcagctggttcaatctggggctgaagtcaagaagcctgggtcctcagtgaaagtttcctgcaaggcttctggctacaccttcacccgtaactttatccactggatcagacaggcacctggacaaggccttgagtggattgggtggatttttcctggagatggagatacagagtacaatcaaaagttcaatgggagagcaacaatcacagcagacaaatcaaccagcacagcctatatggagctcagcagcctgagatctgaggacactgcagtctattactgtgcaagaggaaattacaactacgagtactttgattactggggccaaggaaccatggtcacagtctcctca

SEQ ID NO: 150 - DNA, 321 bp, synthetic construct
  source 1..321: mol_type = other DNA
gacatccagatgacccaatccccttcattcgtgagtgcctcagtgggcgacagagtcaccattacgtgtcttgcttcagaggacatttacagctatctcgcatggtatcagcagaaacctgggaaagcacccaaactgctgatattcgctgccaatcggctgcaaagcggcgtaccatccaggttttctggaggaggatctggtactgggtttaccctgactatcagctcccttcagcccgaggattttgccacatacttctgcctccaaggcagcaaattcccgtacacatttgggcagggtaccaagctggagatcaac

SEQ ID NO: 151 - DNA, 321 bp, synthetic construct
  source 1..321: mol_type = other DNA
gacatccagatgacccaatccccttcattcgtgagtgcctcagtgggcgacagagtcaccattacgtgtcttgcttcagaggacatttacagctatctcgcatggtatcagcagaaacctgggaaagcacccaaactgctgatattcgctgccaatcggctgcaaagcggcgtaccatccaggttttctggaggaggatctggtactgggtttaccctgactatcagctcccttcagcccgaggattttgccacatacttctgcctccaaggcagcaaattcccgtacacatttgggcagggtaccaagctggagatcaag

SEQ ID NO: 152 - DNA, 321 bp, synthetic construct
  source 1..321: mol_type = other DNA
gacatccagatgacccaatccccttcattcgtgagtgcctcagtgggcgacagagtcaccattacgtgtcttgcttcagaggacatttacagctatctcgcatggtatcagcagaaacctgggaaagcacccaaactgctgatattcgctgccaatcggctgcaagatggcgtaccatccaggttttctggaggaggatctggtactgggtttaccctgactatcagctcccttcagcccgaggattttgccacatacttctgcctccaaggcagcaaattcccgtacacatttgggcagggtaccaagctggagatcaag

SEQ ID NO: 153 - DNA, 321 bp, synthetic construct
  source 1..321: mol_type = other DNA
gacatccagatgacacagtctccatcttccctgtctgcatctgtgggagacagagtcaccatcacttgtctggcaagcgaggacatttacagttatcttgcatggtatcaacagaagccagggaaagctcctaagctcctgatctttgctgcaaataggctgcaagatggggtcccatcacggttcagtggcagtggatctggcacagactttactctcaccatcagcagtctgcaacctgaagatttcgcaacttattactgtcttcagggttccaagtttccctacacctttggacctgggaccaaggtggacatcaaa

SEQ ID NO: 154 - DNA, 321 bp, synthetic construct
  source 1..321: mol_type = other DNA
gacatccagatgacacagtctccatcttccctgtctgcatctgtgggagacagagtcaccatcacttgtctggcaagcgaggacatttacagttatcttgcatggtatcaacagaagccagggaaagctcctaagctcctgatctttgctgcaaataggctgcaaagcggggtcccatcacggttcagtggcagtggatctggcacagactttactctcaccatcagcagtctgcaacctgaagatttcgcaacttattactgtcttcagggttccaagtttccctacacctttggacctgggaccaaggtggacatcaaa

SEQ ID NO: 155 - protein, 695 aa, synthetic construct
QMQLVQSGAEVKKTGSSVKVSCKASGYTFTRNFIHWVRQAPGQALEWMGWIFPGDGDTEYNQKFNGRVTITRDRSMSTAYMELSSLRSEDTAMYYCARGNYNYEYFDYWGQGTLVTVSSASTKGPSVFPLAPSSKSTSGGTAALGCLVKDYFPEPVTVSWNSGALTSGVHTFPAVLQSSGLYSLSSVVTVPSSSLGTQTYICNVNHKPSNTKVDKRVEPKSCGGGGSQVQLVQSGGGVVQPGRSLRLSCKASGYTFTRYTMHWVRQAPGKGLEWIGYINPSRGYTNYNQKVKDRFTISRDNSKNTAFLQMDSLRPEDTGVYFCARYYDDHYSLDYWGQGTPVTVSSGGGGSGGGGSGGGGSDIQMTQSPSSLSASVGDRVTITCSASSSVSYMNWYQQTPGKAPKRWIYDTSKLASGVPSRFSGSGSGTDYTFTISSLQPEDIATYYCQQWSSNPFTFGQGTKLQITRDKTHTCPPCPAPEAAGGPSVFLFPPKPKDTLMISRTPEVTCVVVDVSHEDPEVKFNWYVDGVEVHNAKTKPREEQYNSTYRVVSVLTVLHQDWLNGKEYKCKVSNKALPAPIEKTISKAKGQPREPQVYTLPPSREEMTKNQVSLTCLVKGFYPSDIAVEWESNGQPENNYKTTPPVLDSDGSFFLYSKLTVDKSRWQQGNVFSCSVMHEALHNHYTQKSLSLSPGK

SEQ ID NO: 156 - protein, 695 aa, synthetic construct
QMQLVQSGAEVKKTGSSVKVSCKASGYTFTRNFIHWVRQAPGQALEWMGWIFPGDGDTEYNQKFNGRVTITRDRSMSTAYMELSSLRSEDTAMYYCARGNYNYEYFDYWGQGTLVTVSSASTKGPSVFPLAPSSKSTSGGTAALGCLVKDYFPEPVTVSWNSGALTSGVHTFPAVLQSSGLYSLSSVVTVPSSSLGTQTYICNVNHKPSNTKVDKRVEPKSCGGGGSQVQLVQSGGGVVQPGRSLRLSCKASGYTFTRYTMHWVRQAPGKGLEWIGYINPSRGYTNYNQKVKDRFTISRDNSKNTAFLQMDSLRPEDTGVYFCARYYDDHYSLDYWGQGTPVTVSSGGGGSGGGGSGGGGSDIQMTQSPSSLSASVGDRVTITCSASSSVAYMNWYQQTPGKAPKRWIYDTSKLASGVPSRFSGSGSGTDYTFTISSLQPEDIATYYCQQWSSNPFTFGQGTKLQITRDKTHTCPPCPAPEAAGGPSVFLFPPKPKDTLMISRTPEVTCVVVDVSHEDPEVKFNWYVDGVEVHNAKTKPREEQYNSTYRVVSVLTVLHQDWLNGKEYKCKVSNKALPAPIEKTISKAKGQPREPQVYTLPPSREEMTKNQVSLTCLVKGFYPSDIAVEWESNGQPENNYKTTPPVLDSDGSFFLYSKLTVDKSRWQQGNVFSCSVMHEALHNHYTQKSLSLSPGK

SEQ ID NO: 157 - protein, 695 aa, synthetic construct
QMQLVQSGAEVKKTGSSVKVSCKASGYTFTRNFIHWVRQAPGQALEWMGWIFPGDGDTEYNQKFNGRVTITRDRSMSTAYMELSSLRSEDTAMYYCARGNYNYEYFDYWGQGTLVTVSSASTKGPSVFPLAPSSKSTSGGTAALGCLVKDYFPEPVTVSWNSGALTSGVHTFPAVLQSSGLYSLSSVVTVPSSSLGTQTYICNVNHKPSNTKVDKRVEPKSCGGGGSQVQLVQSGGGVVQPGRSLRLSCKASGYTFTRYTMHWVRQAPGKGLEWIGYINPSRGYTNYNQKVKDRFTISRDNSKNTAFLQMDSLRPEDTGVYFCARYYDDHYSLDYWGQGTPVTVSSGGGGSGGGGSGGGGSDIQMTQSPSSLSASVGDRVTITCSASSSVSYMNWYQQTPGKAPKRWIYNTSKLASGVPSRFSGSGSGTDYTFTISSLQPEDIATYYCQQWSSNPFTFGQGTKLQITRDKTHTCPPCPAPEAAGGPSVFLFPPKPKDTLMISRTPEVTCVVVDVSHEDPEVKFNWYVDGVEVHNAKTKPREEQYNSTYRVVSVLTVLHQDWLNGKEYKCKVSNKALPAPIEKTISKAKGQPREPQVYTLPPSREEMTKNQVSLTCLVKGFYPSDIAVEWESNGQPENNYKTTPPVLDSDGSFFLYSKLTVDKSRWQQGNVFSCSVMHEALHNHYTQKSLSLSPGK

SEQ ID NO: 158 - protein, 695 aa, synthetic construct
QMQLVQSGAEVKKTGSSVKVSCKASGYTFTRNFIHWVRQAPGQALEWMGWIFPGDGDTEYNQKFNGRVTITRDRSMSTAYMELSSLRSEDTAMYYCARGNYNYEYFDYWGQGTLVTVSSASTKGPSVFPLAPSSKSTSGGTAALGCLVKDYFPEPVTVSWNSGALTSGVHTFPAVLQSSGLYSLSSVVTVPSSSLGTQTYICNVNHKPSNTKVDKRVEPKSCGGGGSQVQLVQSGGGVVQPGRSLRLSCKASGYTFTRYTMHWVRQAPGKGLEWIGYINPSRGYTNYNQKVKDRFTISRDNSKNTAFLQMDSLRPEDTGVYFCARYYNDHYSLDYWGQGTPVTVSSGGGGSGGGGSGGGGSDIQMTQSPSSLSASVGDRVTITCSASSSVSYMNWYQQTPGKAPKRWIYDTSKLASGVPSRFSGSGSGTDYTFTISSLQPEDIATYYCQQWSSNPFTFGQGTKLQITRDKTHTCPPCPAPEAAGGPSVFLFPPKPKDTLMISRTPEVTCVVVDVSHEDPEVKFNWYVDGVEVHNAKTKPREEQYNSTYRVVSVLTVLHQDWLNGKEYKCKVSNKALPAPIEKTISKAKGQPREPQVYTLPPSREEMTKNQVSLTCLVKGFYPSDIAVEWESNGQPENNYKTTPPVLDSDGSFFLYSKLTVDKSRWQQGNVFSCSVMHEALHNHYTQKSLSLSPGK

SEQ ID NO: 159 - protein, 695 aa, synthetic construct
QMQLVQSGAEVKKTGSSVKVSCKASGYTFTRNFIHWVRQAPGQALEWMGWIFPGDGDTEYNQKFNGRVTITRDRSMSTAYMELSSLRSEDTAMYYCARGNYNYEYFDYWGQGTLVTVSSASTKGPSVFPLAPSSKSTSGGTAALGCLVKDYFPEPVTVSWNSGALTSGVHTFPAVLQSSGLYSLSSVVTVPSSSLGTQTYICNVNHKPSNTKVDKRVEPKSCGGGGSQVQLVQSGGGVVQPGRSLRLSCKASGYTFTRYTMHWVRQAPGKGLEWIGYINPSRGYTNYNQKVKDRFTISRDNSKNTAFLQMDSLRPEDTGVYFCARYYDDHFSLDYWGQGTPVTVSSGGGGSGGGGSGGGGSDIQMTQSPSSLSASVGDRVTITCSASSSVSYMNWYQQTPGKAPKRWIYDTSKLASGVPSRFSGSGSGTDYTFTISSLQPEDIATYYCQQWSSNPFTFGQGTKLQITRDKTHTCPPCPAPEAAGGPSVFLFPPKPKDTLMISRTPEVTCVVVDVSHEDPEVKFNWYVDGVEVHNAKTKPREEQYNSTYRVVSVLTVLHQDWLNGKEYKCKVSNKALPAPIEKTISKAKGQPREPQVYTLPPSREEMTKNQVSLTCLVKGFYPSDIAVEWESNGQPENNYKTTPPVLDSDGSFFLYSKLTVDKSRWQQGNVFSCSVMHEALHNHYTQKSLSLSPGK

SEQ ID NO: 160 - protein, 695 aa, synthetic construct
QMQLVQSGAEVKKTGSSVKVSCKASGYTFTRNFIHWVRQAPGQALEWMGWIFPGDGDTEYNQKFNGRVTITRDRSMSTAYMELSSLRSEDTAMYYCARGNYNYEYFDYWGQGTLVTVSSASTKGPSVFPLAPSSKSTSGGTAALGCLVKDYFPEPVTVSWNSGALTSGVHTFPAVLQSSGLYSLSSVVTVPSSSLGTQTYICNVNHKPSNTKVDKRVEPKSCGGGGSQVQLVQSGGGVVQPGRSLRLSCKASGYTFTRYTMHWVRQAPGKGLEWIGYINPSMGATNYNQKVKDRFTISRDNSKNTAFLQMDSLRPEDTGVYFCARYYDDHYSLDYWGQGTPVTVSSGGGGSGGGGSGGGGSDIQMTQSPSSLSASVGDRVTITCSASSSVSYMNWYQQTPGKAPKRWIYDTSKLASGVPSRFSGSGSGTDYTFTISSLQPEDIATYYCQQWSSNPFTFGQGTKLQITRDKTHTCPPCPAPEAAGGPSVFLFPPKPKDTLMISRTPEVTCVVVDVSHEDPEVKFNWYVDGVEVHNAKTKPREEQYNSTYRVVSVLTVLHQDWLNGKEYKCKVSNKALPAPIEKTISKAKGQPREPQVYTLPPSREEMTKNQVSLTCLVKGFYPSDIAVEWESNGQPENNYKTTPPVLDSDGSFFLYSKLTVDKSRWQQGNVFSCSVMHEALHNHYTQKSLSLSPGK

SEQ ID NO: 161 - protein, 695 aa, synthetic construct
QMQLVQSGAEVKKTGSSVKVSCKASGYTFTRNFIHWVRQAPGQALEWMGWIFPGDADTEYNQKFSGRVTITRDRSMSTAYMELSSLRSEDTAMYYCARGNYNYEYFDYWGQGTLVTVSSASTKGPSVFPLAPSSKSTSGGTAALGCLVKDYFPEPVTVSWNSGALTSGVHTFPAVLQSSGLYSLSSVVTVPSSSLGTQTYICNVNHKPSNTKVDKRVEPKSCGGGGSQVQLVQSGGGVVQPGRSLRLSCKASGYTFTRYTMHWVRQAPGKGLEWIGYINPSRGYTNYNQKVKDRFTISRDNSKNTAFLQMDSLRPEDTGVYFCARYYDDHYSLDYWGQGTPVTVSSGGGGSGGGGSGGGGSDIQMTQSPSSLSASVGDRVTITCSASSSVSYMNWYQQTPGKAPKRWIYDTSKLASGVPSRFSGSGSGTDYTFTISSLQPEDIATYYCQQWSSNPFTFGQGTKLQITRDKTHTCPPCPAPEAAGGPSVFLFPPKPKDTLMISRTPEVTCVVVDVSHEDPEVKFNWYVDGVEVHNAKTKPREEQYNSTYRVVSVLTVLHQDWLNGKEYKCKVSNKALPAPIEKTISKAKGQPREPQVYTLPPSREEMTKNQVSLTCLVKGFYPSDIAVEWESNGQPENNYKTTPPVLDSDGSFFLYSKLTVDKSRWQQGNVFSCSVMHEALHNHYTQKSLSLSPGK

SEQ ID NO: 162 - protein, 695 aa, synthetic construct
QMQLVQSGAEVKKTGSSVKVSCKASGYTFTRNFIHWVRQAPGQALEWMGWIFPGDADTEYNQKFSGRVTITRDRSMSTAYMELSSLRSEDTAMYYCARGNYNYEYFDYWGQGTLVTVSSASTKGPSVFPLAPSSKSTSGGTAALGCLVKDYFPEPVTVSWNSGALTSGVHTFPAVLQSSGLYSLSSVVTVPSSSLGTQTYICNVNHKPSNTKVDKRVEPKSCGGGGSQVQLVQSGGGVVQPGRSLRLSCKASGYTFTRYTMHWVRQAPGKGLEWIGYINPSRGYTNYNQKVKDRFTISRDNSKNTAFLQMDSLRPEDTGVYFCARYYDDHYSLDYWGQGTPVTVSSGGGGSGGGGSGGGGSDIQMTQSPSSLSASVGDRVTITCSASSSVAYMNWYQQTPGKAPKRWIYDTSKLASGVPSRFSGSGSGTDYTFTISSLQPEDIATYYCQQWSSNPFTFGQGTKLQITRDKTHTCPPCPAPEAAGGPSVFLFPPKPKDTLMISRTPEVTCVVVDVSHEDPEVKFNWYVDGVEVHNAKTKPREEQYNSTYRVVSVLTVLHQDWLNGKEYKCKVSNKALPAPIEKTISKAKGQPREPQVYTLPPSREEMTKNQVSLTCLVKGFYPSDIAVEWESNGQPENNYKTTPPVLDSDGSFFLYSKLTVDKSRWQQGNVFSCSVMHEALHNHYTQKSLSLSPGK

SEQ ID NO: 163 - protein, 695 aa, synthetic construct
QMQLVQSGAEVKKTGSSVKVSCKASGYTFTRNFIHWVRQAPGQALEWMGWIFPGDADTEYNQKFSGRVTITRDRSMSTAYMELSSLRSEDTAMYYCARGNYNYEYFDYWGQGTLVTVSSASTKGPSVFPLAPSSKSTSGGTAALGCLVKDYFPEPVTVSWNSGALTSGVHTFPAVLQSSGLYSLSSVVTVPSSSLGTQTYICNVNHKPSNTKVDKRVEPKSCGGGGSQVQLVQSGGGVVQPGRSLRLSCKASGYTFTRYTMHWVRQAPGKGLEWIGYINPSRGYTNYNQKVKDRFTISRDNSKNTAFLQMDSLRPEDTGVYFCARYYDDHYSLDYWGQGTPVTVSSGGGGSGGGGSGGGGSDIQMTQSPSSLSASVGDRVTITCSASSSVSYMNWYQQTPGKAPKRWIYNTSKLASGVPSRFSGSGSGTDYTFTISSLQPEDIATYYCQQWSSNPFTFGQGTKLQITRDKTHTCPPCPAPEAAGGPSVFLFPPKPKDTLMISRTPEVTCVVVDVSHEDPEVKFNWYVDGVEVHNAKTKPREEQYNSTYRVVSVLTVLHQDWLNGKEYKCKVSNKALPAPIEKTISKAKGQPREPQVYTLPPSREEMTKNQVSLTCLVKGFYPSDIAVEWESNGQPENNYKTTPPVLDSDGSFFLYSKLTVDKSRWQQGNVFSCSVMHEALHNHYTQKSLSLSPGK

SEQ ID NO: 164 - protein, 695 aa, synthetic construct
QMQLVQSGAEVKKTGSSVKVSCKASGYTFTRNFIHWVRQAPGQALEWMGWIFPGDADTEYNQKFSGRVTITRDRSMSTAYMELSSLRSEDTAMYYCARGNYNYEYFDYWGQGTLVTVSSASTKGPSVFPLAPSSKSTSGGTAALGCLVKDYFPEPVTVSWNSGALTSGVHTFPAVLQSSGLYSLSSVVTVPSSSLGTQTYICNVNHKPSNTKVDKRVEPKSCGGGGSQVQLVQSGGGVVQPGRSLRLSCKASGYTFTRYTMHWVRQAPGKGLEWIGYINPSRGYTNYNQKVKDRFTISRDNSKNTAFLQMDSLRPEDTGVYFCARYYNDHYSLDYWGQGTPVTVSSGGGGSGGGGSGGGGSDIQMTQSPSSLSASVGDRVTITCSASSSVSYMNWYQQTPGKAPKRWIYDTSKLASGVPSRFSGSGSGTDYTFTISSLQPEDIATYYCQQWSSNPFTFGQGTKLQITRDKTHTCPPCPAPEAAGGPSVFLFPPKPKDTLMISRTPEVTCVVVDVSHEDPEVKFNWYVDGVEVHNAKTKPREEQYNSTYRVVSVLTVLHQDWLNGKEYKCKVSNKALPAPIEKTISKAKGQPREPQVYTLPPSREEMTKNQVSLTCLVKGFYPSDIAVEWESNGQPENNYKTTPPVLDSDGSFFLYSKLTVDKSRWQQGNVFSCSVMHEALHNHYTQKSLSLSPGK

SEQ ID NO: 165 - protein, 695 aa, synthetic construct
QMQLVQSGAEVKKTGSSVKVSCKASGYTFTRNFIHWVRQAPGQALEWMGWIFPGDADTEYNQKFSGRVTITRDRSMSTAYMELSSLRSEDTAMYYCARGNYNYEYFDYWGQGTLVTVSSASTKGPSVFPLAPSSKSTSGGTAALGCLVKDYFPEPVTVSWNSGALTSGVHTFPAVLQSSGLYSLSSVVTVPSSSLGTQTYICNVNHKPSNTKVDKRVEPKSCGGGGSQVQLVQSGGGVVQPGRSLRLSCKASGYTFTRYTMHWVRQAPGKGLEWIGYINPSRGYTNYNQKVKDRFTISRDNSKNTAFLQMDSLRPEDTGVYFCARYYDDHFSLDYWGQGTPVTVSSGGGGSGGGGSGGGGSDIQMTQSPSSLSASVGDRVTITCSASSSVSYMNWYQQTPGKAPKRWIYDTSKLASGVPSRFSGSGSGTDYTFTISSLQPEDIATYYCQQWSSNPFTFGQGTKLQITRDKTHTCPPCPAPEAAGGPSVFLFPPKPKDTLMISRTPEVTCVVVDVSHEDPEVKFNWYVDGVEVHNAKTKPREEQYNSTYRVVSVLTVLHQDWLNGKEYKCKVSNKALPAPIEKTISKAKGQPREPQVYTLPPSREEMTKNQVSLTCLVKGFYPSDIAVEWESNGQPENNYKTTPPVLDSDGSFFLYSKLTVDKSRWQQGNVFSCSVMHEALHNHYTQKSLSLSPGK

SEQ ID NO: 166 - protein, 695 aa, synthetic construct
QMQLVQSGAEVKKTGSSVKVSCKASGYTFTRNFIHWVRQAPGQALEWMGWIFPGDADTEYNQKFSGRVTITRDRSMSTAYMELSSLRSEDTAMYYCARGNYNYEYFDYWGQGTLVTVSSASTKGPSVFPLAPSSKSTSGGTAALGCLVKDYFPEPVTVSWNSGALTSGVHTFPAVLQSSGLYSLSSVVTVPSSSLGTQTYICNVNHKPSNTKVDKRVEPKSCGGGGSQVQLVQSGGGVVQPGRSLRLSCKASGYTFTRYTMHWVRQAPGKGLEWIGYINPSMGATNYNQKVKDRFTISRDNSKNTAFLQMDSLRPEDTGVYFCARYYDDHYSLDYWGQGTPVTVSSGGGGSGGGGSGGGGSDIQMTQSPSSLSASVGDRVTITCSASSSVSYMNWYQQTPGKAPKRWIYDTSKLASGVPSRFSGSGSGTDYTFTISSLQPEDIATYYCQQWSSNPFTFGQGTKLQITRDKTHTCPPCPAPEAAGGPSVFLFPPKPKDTLMISRTPEVTCVVVDVSHEDPEVKFNWYVDGVEVHNAKTKPREEQYNSTYRVVSVLTVLHQDWLNGKEYKCKVSNKALPAPIEKTISKAKGQPREPQVYTLPPSREEMTKNQVSLTCLVKGFYPSDIAVEWESNGQPENNYKTTPPVLDSDGSFFLYSKLTVDKSRWQQGNVFSCSVMHEALHNHYTQKSLSLSPGK

SEQ ID NO: 167 - protein, 449 aa, synthetic construct
QMQLVQSGAEVKKTGSSVKVSCKASGYTFTRNFIHWVRQAPGQALEWMGWIFPGDGDTEYNQKFNGRVTITRDRSMSTAYMELSSLRSEDTAMYYCARGNYNYEYFDYWGQGTLVTVSSASTKGPSVFPLAPSSKSTSGGTAALGCLVKDYFPEPVTVSWNSGALTSGVHTFPAVLQSSGLYSLSSVVTVPSSSLGTQTYICNVNHKPSNTKVDKRVEPKSCDKTHTCPPCPAPEAAGGPSVFLFPPKPKDTLMISRTPEVTCVVVDVSHEDPEVKFNWYVDGVEVHNAKTKPREEQYNSTYRVVSVLTVLHQDWLNGKEYKCKVSNKALPAPIEKTISKAKGQPREPQVYTLPPSREEMTKNQVSLTCLVKGFYPSDIAVEWESNGQPENNYKTTPPVLDSDGSFFLYSKLTVDKSRWQQGNVFSCSVMHEALHNHYTQKSLSLSPGK

SEQ ID NO: 168 - protein, 449 aa, synthetic construct
QMQLVQSGAEVKKTGSSVKVSCKASGYTFTRNFIHWVRQAPGQALEWMGWIFPGDADTEYNQKFSGRVTITRDRSMSTAYMELSSLRSEDTAMYYCARGNYNYEYFDYWGQGTLVTVSSASTKGPSVFPLAPSSKSTSGGTAALGCLVKDYFPEPVTVSWNSGALTSGVHTFPAVLQSSGLYSLSSVVTVPSSSLGTQTYICNVNHKPSNTKVDKRVEPKSCDKTHTCPPCPAPEAAGGPSVFLFPPKPKDTLMISRTPEVTCVVVDVSHEDPEVKFNWYVDGVEVHNAKTKPREEQYNSTYRVVSVLTVLHQDWLNGKEYKCKVSNKALPAPIEKTISKAKGQPREPQVYTLPPSREEMTKNQVSLTCLVKGFYPSDIAVEWESNGQPENNYKTTPPVLDSDGSFFLYSKLTVDKSRWQQGNVFSCSVMHEALHNHYTQKSLSLSPGK

SEQ ID NO: 169 - protein, 214 aa, synthetic construct
DIQMTQSPSFVSASVGDRVTITCLASEDIYSYLAWYQQKPGKAPKLLIFAANRLQSGVPSRFSGGGSGTGFTLTISSLQPEDFATYFCLQGSKFPYTFGQGTKLEINRTVAAPSVFIFPPSDEQLKSGTASVVCLLNNFYPREAKVQWKVDNALQSGNSQESVTEQDSKDSTYSLSSTLTLSKADYEKHKVYACEVTHQGLSSPVTKSFNRGEC

SEQ ID NO: 170 - protein, 214 aa, synthetic construct
DIQMTQSPSFVSASVGDRVTITCLASEDIYSYLAWYQQKPGKAPKLLIFAANRLQDGVPSRFSGGGSGTGFTLTISSLQPEDFATYFCLQGSKFPYTFGQGTKLEIKRTVAAPSVFIFPPSDEQLKSGTASVVCLLNNFYPREAKVQWKVDNALQSGNSQESVTEQDSKDSTYSLSSTLTLSKADYEKHKVYACEVTHQGLSSPVTKSFNRGEC

SEQ ID NO: 171 - protein, 214 aa, synthetic construct
DIQMTQSPSFVSASVGDRVTITCLASEDIYSYLAWYQQKPGKAPKLLIFAANRLQSGVPSRFSGGGSGTGFTLTISSLQPEDFATYFCLQGSKFPYTFGQGTKLEIKRTVAAPSVFIFPPSDEQLKSGTASVVCLLNNFYPREAKVQWKVDNALQSGNSQESVTEQDSKDSTYSLSSTLTLSKADYEKHKVYACEVTHQGLSSPVTKSFNRGEC

SEQ ID NO: 172 - protein, 465 aa, synthetic construct
DIQMTQSPSFVSASVGDRVTITCLASEDIYSYLAWYQQKPGKAPKLLIFAANRLQDGVPSRFSGGGSGTGFTLTISSLQPEDFATYFCLQGSKFPYTFGQGTKLEINRTVAAPSVFIFPPSDEQLKSGTASVVCLLNNFYPREAKVQWKVDNALQSGNSQESVTEQDSKDSTYSLSSTLTLSKADYEKHKVYACEVTHQGLSSPVTKSFNRGECGGGGSGGGGSQVQLVQSGGGVVQPGRSLRLSCKASGYTFTRYTMHWVRQAPGKGLEWIGYINPSRGYTNYNQKVKDRFTISRDNSKNTAFLQMDSLRPEDTGVYFCARYYDDHYSLDYWGQGTPVTVSSGGGGSGGGGSGGGGSDIQMTQSPSSLSASVGDRVTITCSASSSVSYMNWYQQTPGKAPKRWIYDTSKLASGVPSRFSGSGSGTDYTFTISSLQPEDIATYYCQQWSSNPFTFGQGTKLQITR

SEQ ID NO: 173 - protein, 465 aa, synthetic construct
DIQMTQSPSFVSASVGDRVTITCLASEDIYSYLAWYQQKPGKAPKLLIFAANRLQSGVPSRFSGGGSGTGFTLTISSLQPEDFATYFCLQGSKFPYTFGQGTKLEINRTVAAPSVFIFPPSDEQLKSGTASVVCLLNNFYPREAKVQWKVDNALQSGNSQESVTEQDSKDSTYSLSSTLTLSKADYEKHKVYACEVTHQGLSSPVTKSFNRGECGGGGSGGGGSQVQLVQSGGGVVQPGRSLRLSCKASGYTFTRYTMHWVRQAPGKGLEWIGYINPSRGYTNYNQKVKDRFTISRDNSKNTAFLQMDSLRPEDTGVYFCARYYDDHYSLDYWGQGTPVTVSSGGGGSGGGGSGGGGSDIQMTQSPSSLSASVGDRVTITCSASSSVSYMNWYQQTPGKAPKRWIYDTSKLASGVPSRFSGSGSGTDYTFTISSLQPEDIATYYCQQWSSNPFTFGQGTKLQITR

SEQ ID NO: 174 - protein, 695 aa, synthetic construct
QVQLVQSGAEVKKPGSSVKVSCKASGYTFTRNFIHWIRQAPGQGLEWIGWIFPGDADTEYNQKFSGRATITADKSTSTAYMELSSLRSEDTAVYYCARGNYNYEYFDYWGQGTMVTVSSASTKGPSVFPLAPSSKSTSGGTAALGCLVKDYFPEPVTVSWNSGALTSGVHTFPAVLQSSGLYSLSSVVTVPSSSLGTQTYICNVNHKPSNTKVDKRVEPKSCGGGGSQVQLVQSGGGVVQPGRSLRLSCKASGYTFTRYTMHWVRQAPGKGLEWIGYINPSRGYTNYNQKVKDRFTISRDNSKNTAFLQMDSLRPEDTGVYFCARYYDDHYSLDYWGQGTPVTVSSGGGGSGGGGSGGGGSDIQMTQSPSSLSASVGDRVTITCSASSSVSYMNWYQQTPGKAPKRWIYDTSKLASGVPSRFSGSGSGTDYTFTISSLQPEDIATYYCQQWSSNPFTFGQGTKLQITRDKTHTCPPCPAPEAAGGPSVFLFPPKPKDTLMISRTPEVTCVVVDVSHEDPEVKFNWYVDGVEVHNAKTKPREEQYNSTYRVVSVLTVLHQDWLNGKEYKCKVSNKALPAPIEKTISKAKGQPREPQVYTLPPSREEMTKNQVSLTCLVKGFYPSDIAVEWESNGQPENNYKTTPPVLDSDGSFFLYSKLTVDKSRWQQGNVFSCSVMHEALHNHYTQKSLSLSPGK

SEQ ID NO: 175 - protein, 695 aa, synthetic construct
QVQLVQSGAEVKKPGSSVKVSCKASGYTFTRNFIHWIRQAPGQGLEWIGWIFPGDADTEYNQKFSGRATITADKSTSTAYMELSSLRSEDTAVYYCARGNYNYEYFDYWGQGTMVTVSSASTKGPSVFPLAPSSKSTSGGTAALGCLVKDYFPEPVTVSWNSGALTSGVHTFPAVLQSSGLYSLSSVVTVPSSSLGTQTYICNVNHKPSNTKVDKRVEPKSCGGGGSQVQLVQSGGGVVQPGRSLRLSCKASGYTFTRYTMHWVRQAPGKGLEWIGYINPSRGYTNYNQKVKDRFTISRDNSKNTAFLQMDSLRPEDTGVYFCARYYDDHYSLDYWGQGTPVTVSSGGGGSGGGGSGGGGSDIQMTQSPSSLSASVGDRVTITCSASSSVAYMNWYQQTPGKAPKRWIYDTSKLASGVPSRFSGSGSGTDYTFTISSLQPEDIATYYCQQWSSNPFTFGQGTKLQITRDKTHTCPPCPAPEAAGGPSVFLFPPKPKDTLMISRTPEVTCVVVDVSHEDPEVKFNWYVDGVEVHNAKTKPREEQYNSTYRVVSVLTVLHQDWLNGKEYKCKVSNKALPAPIEKTISKAKGQPREPQVYTLPPSREEMTKNQVSLTCLVKGFYPSDIAVEWESNGQPENNYKTTPPVLDSDGSFFLYSKLTVDKSRWQQGNVFSCSVMHEALHNHYTQKSLSLSPGK

SEQ ID NO: 176 - protein, 695 aa, synthetic construct
QVQLVQSGAEVKKPGSSVKVSCKASGYTFTRNFIHWIRQAPGQGLEWIGWIFPGDADTEYNQKFSGRATITADKSTSTAYMELSSLRSEDTAVYYCARGNYNYEYFDYWGQGTMVTVSSASTKGPSVFPLAPSSKSTSGGTAALGCLVKDYFPEPVTVSWNSGALTSGVHTFPAVLQSSGLYSLSSVVTVPSSSLGTQTYICNVNHKPSNTKVDKRVEPKSCGGGGSQVQLVQSGGGVVQPGRSLRLSCKASGYTFTRYTMHWVRQAPGKGLEWIGYINPSRGYTNYNQKVKDRFTISRDNSKNTAFLQMDSLRPEDTGVYFCARYYDDHYSLDYWGQGTPVTVSSGGGGSGGGGSGGGGSDIQMTQSPSSLSASVGDRVTITCSASSSVSYMNWYQQTPGKAPKRWIYNTSKLASGVPSRFSGSGSGTDYTFTISSLQPEDIATYYCQQWSSNPFTFGQGTKLQITRDKTHTCPPCPAPEAAGGPSVFLFPPKPKDTLMISRTPEVTCVVVDVSHEDPEVKFNWYVDGVEVHNAKTKPREEQYNSTYRVVSVLTVLHQDWLNGKEYKCKVSNKALPAPIEKTISKAKGQPREPQVYTLPPSREEMTKNQVSLTCLVKGFYPSDIAVEWESNGQPENNYKTTPPVLDSDGSFFLYSKLTVDKSRWQQGNVFSCSVMHEALHNHYTQKSLSLSPGK

SEQ ID NO: 177 - protein, 695 aa, synthetic construct
QVQLVQSGAEVKKPGSSVKVSCKASGYTFTRNFIHWIRQAPGQGLEWIGWIFPGDADTEYNQKFSGRATITADKSTSTAYMELSSLRSEDTAVYYCARGNYNYEYFDYWGQGTMVTVSSASTKGPSVFPLAPSSKSTSGGTAALGCLVKDYFPEPVTVSWNSGALTSGVHTFPAVLQSSGLYSLSSVVTVPSSSLGTQTYICNVNHKPSNTKVDKRVEPKSCGGGGSQVQLVQSGGGVVQPGRSLRLSCKASGYTFTRYTMHWVRQAPGKGLEWIGYINPSRGYTNYNQKVKDRFTISRDNSKNTAFLQMDSLRPEDTGVYFCARYYNDHYSLDYWGQGTPVTVSSGGGGSGGGGSGGGGSDIQMTQSPSSLSASVGDRVTITCSASSSVSYMNWYQQTPGKAPKRWIYDTSKLASGVPSRFSGSGSGTDYTFTISSLQPEDIATYYCQQWSSNPFTFGQGTKLQITRDKTHTCPPCPAPEAAGGPSVFLFPPKPKDTLMISRTPEVTCVVVDVSHEDPEVKFNWYVDGVEVHNAKTKPREEQYNSTYRVVSVLTVLHQDWLNGKEYKCKVSNKALPAPIEKTISKAKGQPREPQVYTLPPSREEMTKNQVSLTCLVKGFYPSDIAVEWESNGQPENNYKTTPPVLDSDGSFFLYSKLTVDKSRWQQGNVFSCSVMHEALHNHYTQKSLSLSPGK

SEQ ID NO: 178 - protein, 695 aa, synthetic construct
QVQLVQSGAEVKKPGSSVKVSCKASGYTFTRNFIHWIRQAPGQGLEWIGWIFPGDADTEYNQKFSGRATITADKSTSTAYMELSSLRSEDTAVYYCARGNYNYEYFDYWGQGTMVTVSSASTKGPSVFPLAPSSKSTSGGTAALGCLVKDYFPEPVTVSWNSGALTSGVHTFPAVLQSSGLYSLSSVVTVPSSSLGTQTYICNVNHKPSNTKVDKRVEPKSCGGGGSQVQLVQSGGGVVQPGRSLRLSCKASGYTFTRYTMHWVRQAPGKGLEWIGYINPSRGYTNYNQKVKDRFTISRDNSKNTAFLQMDSLRPEDTGVYFCARYYDDHFSLDYWGQGTPVTVSSGGGGSGGGGSGGGGSDIQMTQSPSSLSASVGDRVTITCSASSSVSYMNWYQQTPGKAPKRWIYDTSKLASGVPSRFSGSGSGTDYTFTISSLQPEDIATYYCQQWSSNPFTFGQGTKLQITRDKTHTCPPCPAPEAAGGPSVFLFPPKPKDTLMISRTPEVTCVVVDVSHEDPEVKFNWYVDGVEVHNAKTKPREEQYNSTYRVVSVLTVLHQDWLNGKEYKCKVSNKALPAPIEKTISKAKGQPREPQVYTLPPSREEMTKNQVSLTCLVKGFYPSDIAVEWESNGQPENNYKTTPPVLDSDGSFFLYSKLTVDKSRWQQGNVFSCSVMHEALHNHYTQKSLSLSPGK

SEQ ID NO: 179 - protein, 695 aa, synthetic construct
QVQLVQSGAEVKKPGSSVKVSCKASGYTFTRNFIHWIRQAPGQGLEWIGWIFPGDADTEYNQKFSGRATITADKSTSTAYMELSSLRSEDTAVYYCARGNYNYEYFDYWGQGTMVTVSSASTKGPSVFPLAPSSKSTSGGTAALGCLVKDYFPEPVTVSWNSGALTSGVHTFPAVLQSSGLYSLSSVVTVPSSSLGTQTYICNVNHKPSNTKVDKRVEPKSCGGGGSQVQLVQSGGGVVQPGRSLRLSCKASGYTFTRYTMHWVRQAPGKGLEWIGYINPSMGATNYNQKVKDRFTISRDNSKNTAFLQMDSLRPEDTGVYFCARYYDDHYSLDYWGQGTPVTVSSGGGGSGGGGSGGGGSDIQMTQSPSSLSASVGDRVTITCSASSSVSYMNWYQQTPGKAPKRWIYDTSKLASGVPSRFSGSGSGTDYTFTISSLQPEDIATYYCQQWSSNPFTFGQGTKLQITRDKTHTCPPCPAPEAAGGPSVFLFPPKPKDTLMISRTPEVTCVVVDVSHEDPEVKFNWYVDGVEVHNAKTKPREEQYNSTYRVVSVLTVLHQDWLNGKEYKCKVSNKALPAPIEKTISKAKGQPREPQVYTLPPSREEMTKNQVSLTCLVKGFYPSDIAVEWESNGQPENNYKTTPPVLDSDGSFFLYSKLTVDKSRWQQGNVFSCSVMHEALHNHYTQKSLSLSPGK

SEQ ID NO: 180 - protein, 695 aa, synthetic construct
QVQLVQSGAEVKKPGSSVKVSCKASGYTFTRNFIHWIRQAPGQGLEWIGWIFPGDADTEYNQKFSGRVTITADKSTSTAYMELSSLRSEDTAVYYCARGNYNYEYFDYWGQGTMVTVSSASTKGPSVFPLAPSSKSTSGGTAALGCLVKDYFPEPVTVSWNSGALTSGVHTFPAVLQSSGLYSLSSVVTVPSSSLGTQTYICNVNHKPSNTKVDKRVEPKSCGGGGSQVQLVQSGGGVVQPGRSLRLSCKASGYTFTRYTMHWVRQAPGKGLEWIGYINPSRGYTNYNQKVKDRFTISRDNSKNTAFLQMDSLRPEDTGVYFCARYYDDHYSLDYWGQGTPVTVSSGGGGSGGGGSGGGGSDIQMTQSPSSLSASVGDRVTITCSASSSVSYMNWYQQTPGKAPKRWIYDTSKLASGVPSRFSGSGSGTDYTFTISSLQPEDIATYYCQQWSSNPFTFGQGTKLQITRDKTHTCPPCPAPEAAGGPSVFLFPPKPKDTLMISRTPEVTCVVVDVSHEDPEVKFNWYVDGVEVHNAKTKPREEQYNSTYRVVSVLTVLHQDWLNGKEYKCKVSNKALPAPIEKTISKAKGQPREPQVYTLPPSREEMTKNQVSLTCLVKGFYPSDIAVEWESNGQPENNYKTTPPVLDSDGSFFLYSKLTVDKSRWQQGNVFSCSVMHEALHNHYTQKSLSLSPGK

SEQ ID NO: 181 - protein, 695 aa, synthetic construct
QVQLVQSGAEVKKPGSSVKVSCKASGYTFTRNFIHWIRQAPGQGLEWIGWIFPGDADTEYNQKFSGRVTITADKSTSTAYMELSSLRSEDTAVYYCARGNYNYEYFDYWGQGTMVTVSSASTKGPSVFPLAPSSKSTSGGTAALGCLVKDYFPEPVTVSWNSGALTSGVHTFPAVLQSSGLYSLSSVVTVPSSSLGTQTYICNVNHKPSNTKVDKRVEPKSCGGGGSQVQLVQSGGGVVQPGRSLRLSCKASGYTFTRYTMHWVRQAPGKGLEWIGYINPSRGYTNYNQKVKDRFTISRDNSKNTAFLQMDSLRPEDTGVYFCARYYDDHYSLDYWGQGTPVTVSSGGGGSGGGGSGGGGSDIQMTQSPSSLSASVGDRVTITCSASSSVAYMNWYQQTPGKAPKRWIYDTSKLASGVPSRFSGSGSGTDYTFTISSLQPEDIATYYCQQWSSNPFTFGQGTKLQITRDKTHTCPPCPAPEAAGGPSVFLFPPKPKDTLMISRTPEVTCVVVDVSHEDPEVKFNWYVDGVEVHNAKTKPREEQYNSTYRVVSVLTVLHQDWLNGKEYKCKVSNKALPAPIEKTISKAKGQPREPQVYTLPPSREEMTKNQVSLTCLVKGFYPSDIAVEWESNGQPENNYKTTPPVLDSDGSFFLYSKLTVDKSRWQQGNVFSCSVMHEALHNHYTQKSLSLSPGK

SEQ ID NO: 182 - protein, 695 aa, synthetic construct
QVQLVQSGAEVKKPGSSVKVSCKASGYTFTRNFIHWIRQAPGQGLEWIGWIFPGDADTEYNQKFSGRVTITADKSTSTAYMELSSLRSEDTAVYYCARGNYNYEYFDYWGQGTMVTVSSASTKGPSVFPLAPSSKSTSGGTAALGCLVKDYFPEPVTVSWNSGALTSGVHTFPAVLQSSGLYSLSSVVTVPSSSLGTQTYICNVNHKPSNTKVDKRVEPKSCGGGGSQVQLVQSGGGVVQPGRSLRLSCKASGYTFTRYTMHWVRQAPGKGLEWIGYINPSRGYTNYNQKVKDRFTISRDNSKNTAFLQMDSLRPEDTGVYFCARYYDDHYSLDYWGQGTPVTVSSGGGGSGGGGSGGGGSDIQMTQSPSSLSASVGDRVTITCSASSSVSYMNWYQQTPGKAPKRWIYNTSKLASGVPSRFSGSGSGTDYTFTISSLQPEDIATYYCQQWSSNPFTFGQGTKLQITRDKTHTCPPCPAPEAAGGPSVFLFPPKPKDTLMISRTPEVTCVVVDVSHEDPEVKFNWYVDGVEVHNAKTKPREEQYNSTYRVVSVLTVLHQDWLNGKEYKCKVSNKALPAPIEKTISKAKGQPREPQVYTLPPSREEMTKNQVSLTCLVKGFYPSDIAVEWESNGQPENNYKTTPPVLDSDGSFFLYSKLTVDKSRWQQGNVFSCSVMHEALHNHYTQKSLSLSPGK

SEQ ID NO: 183 - protein, 695 aa, synthetic construct
QVQLVQSGAEVKKPGSSVKVSCKASGYTFTRNFIHWIRQAPGQGLEWIGWIFPGDADTEYNQKFSGRVTITADKSTSTAYMELSSLRSEDTAVYYCARGNYNYEYFDYWGQGTMVTVSSASTKGPSVFPLAPSSKSTSGGTAALGCLVKDYFPEPVTVSWNSGALTSGVHTFPAVLQSSGLYSLSSVVTVPSSSLGTQTYICNVNHKPSNTKVDKRVEPKSCGGGGSQVQLVQSGGGVVQPGRSLRLSCKASGYTFTRYTMHWVRQAPGKGLEWIGYINPSRGYTNYNQKVKDRFTISRDNSKNTAFLQMDSLRPEDTGVYFCARYYNDHYSLDYWGQGTPVTVSSGGGGSGGGGSGGGGSDIQMTQSPSSLSASVGDRVTITCSASSSVSYMNWYQQTPGKAPKRWIYDTSKLASGVPSRFSGSGSGTDYTFTISSLQPEDIATYYCQQWSSNPFTFGQGTKLQITRDKTHTCPPCPAPEAAGGPSVFLFPPKPKDTLMISRTPEVTCVVVDVSHEDPEVKFNWYVDGVEVHNAKTKPREEQYNSTYRVVSVLTVLHQDWLNGKEYKCKVSNKALPAPIEKTISKAKGQPREPQVYTLPPSREEMTKNQVSLTCLVKGFYPSDIAVEWESNGQPENNYKTTPPVLDSDGSFFLYSKLTVDKSRWQQGNVFSCSVMHEALHNHYTQKSLSLSPGK

SEQ ID NO: 184 - protein, 695 aa, synthetic construct
QVQLVQSGAEVKKPGSSVKVSCKASGYTFTRNFIHWIRQAPGQGLEWIGWIFPGDADTEYNQKFSGRVTITADKSTSTAYMELSSLRSEDTAVYYCARGNYNYEYFDYWGQGTMVTVSSASTKGPSVFPLAPSSKSTSGGTAALGCLVKDYFPEPVTVSWNSGALTSGVHTFPAVLQSSGLYSLSSVVTVPSSSLGTQTYICNVNHKPSNTKVDKRVEPKSCGGGGSQVQLVQSGGGVVQPGRSLRLSCKASGYTFTRYTMHWVRQAPGKGLEWIGYINPSRGYTNYNQKVKDRFTISRDNSKNTAFLQMDSLRPEDTGVYFCARYYDDHFSLDYWGQGTPVTVSSGGGGSGGGGSGGGGSDIQMTQSPSSLSASVGDRVTITCSASSSVSYMNWYQQTPGKAPKRWIYDTSKLASGVPSRFSGSGSGTDYTFTISSLQPEDIATYYCQQWSSNPFTFGQGTKLQITRDKTHTCPPCPAPEAAGGPSVFLFPPKPKDTLMISRTPEVTCVVVDVSHEDPEVKFNWYVDGVEVHNAKTKPREEQYNSTYRVVSVLTVLHQDWLNGKEYKCKVSNKALPAPIEKTISKAKGQPREPQVYTLPPSREEMTKNQVSLTCLVKGFYPSDIAVEWESNGQPENNYKTTPPVLDSDGSFFLYSKLTVDKSRWQQGNVFSCSVMHEALHNHYTQKSLSLSPGK

SEQ ID NO: 185 - protein, 695 aa, synthetic construct
QVQLVQSGAEVKKPGSSVKVSCKASGYTFTRNFIHWIRQAPGQGLEWIGWIFPGDADTEYNQKFSGRVTITADKSTSTAYMELSSLRSEDTAVYYCARGNYNYEYFDYWGQGTMVTVSSASTKGPSVFPLAPSSKSTSGGTAALGCLVKDYFPEPVTVSWNSGALTSGVHTFPAVLQSSGLYSLSSVVTVPSSSLGTQTYICNVNHKPSNTKVDKRVEPKSCGGGGSQVQLVQSGGGVVQPGRSLRLSCKASGYTFTRYTMHWVRQAPGKGLEWIGYINPSMGATNYNQKVKDRFTISRDNSKNTAFLQMDSLRPEDTGVYFCARYYDDHYSLDYWGQGTPVTVSSGGGGSGGGGSGGGGSDIQMTQSPSSLSASVGDRVTITCSASSSVSYMNWYQQTPGKAPKRWIYDTSKLASGVPSRFSGSGSGTDYTFTISSLQPEDIATYYCQQWSSNPFTFGQGTKLQITRDKTHTCPPCPAPEAAGGPSVFLFPPKPKDTLMISRTPEVTCVVVDVSHEDPEVKFNWYVDGVEVHNAKTKPREEQYNSTYRVVSVLTVLHQDWLNGKEYKCKVSNKALPAPIEKTISKAKGQPREPQVYTLPPSREEMTKNQVSLTCLVKGFYPSDIAVEWESNGQPENNYKTTPPVLDSDGSFFLYSKLTVDKSRWQQGNVFSCSVMHEALHNHYTQKSLSLSPGK

SEQ ID NO: 186 - protein, 695 aa, synthetic construct
QVQLVQSGAEVKKPGSSVKVSCKASGYTFTRNFIHWIRQAPGQGLEWIGWIFPGDGDTEYNQKFNGRATITADKSTSTAYMELSSLRSEDTAVYYCARGNYNYEYFDYWGQGTMVTVSSASTKGPSVFPLAPSSKSTSGGTAALGCLVKDYFPEPVTVSWNSGALTSGVHTFPAVLQSSGLYSLSSVVTVPSSSLGTQTYICNVNHKPSNTKVDKRVEPKSCGGGGSQVQLVQSGGGVVQPGRSLRLSCKASGYTFTRYTMHWVRQAPGKGLEWIGYINPSRGYTNYNQKVKDRFTISRDNSKNTAFLQMDSLRPEDTGVYFCARYYDDHYSLDYWGQGTPVTVSSGGGGSGGGGSGGGGSDIQMTQSPSSLSASVGDRVTITCSASSSVSYMNWYQQTPGKAPKRWIYDTSKLASGVPSRFSGSGSGTDYTFTISSLQPEDIATYYCQQWSSNPFTFGQGTKLQITRDKTHTCPPCPAPEAAGGPSVFLFPPKPKDTLMISRTPEVTCVVVDVSHEDPEVKFNWYVDGVEVHNAKTKPREEQYNSTYRVVSVLTVLHQDWLNGKEYKCKVSNKALPAPIEKTISKAKGQPREPQVYTLPPSREEMTKNQVSLTCLVKGFYPSDIAVEWESNGQPENNYKTTPPVLDSDGSFFLYSKLTVDKSRWQQGNVFSCSVMHEALHNHYTQKSLSLSPGK

SEQ ID NO: 187 - protein, 695 aa, synthetic construct
QVQLVQSGAEVKKPGSSVKVSCKASGYTFTRNFIHWIRQAPGQGLEWIGWIFPGDGDTEYNQKFNGRATITADKSTSTAYMELSSLRSEDTAVYYCARGNYNYEYFDYWGQGTMVTVSSASTKGPSVFPLAPSSKSTSGGTAALGCLVKDYFPEPVTVSWNSGALTSGVHTFPAVLQSSGLYSLSSVVTVPSSSLGTQTYICNVNHKPSNTKVDKRVEPKSCGGGGSQVQLVQSGGGVVQPGRSLRLSCKASGYTFTRYTMHWVRQAPGKGLEWIGYINPSRGYTNYNQKVKDRFTISRDNSKNTAFLQMDSLRPEDTGVYFCARYYDDHYSLDYWGQGTPVTVSSGGGGSGGGGSGGGGSDIQMTQSPSSLSASVGDRVTITCSASSSVAYMNWYQQTPGKAPKRWIYDTSKLASGVPSRFSGSGSGTDYTFTISSLQPEDIATYYCQQWSSNPFTFGQGTKLQITRDKTHTCPPCPAPEAAGGPSVFLFPPKPKDTLMISRTPEVTCVVVDVSHEDPEVKFNWYVDGVEVHNAKTKPREEQYNSTYRVVSVLTVLHQDWLNGKEYKCKVSNKALPAPIEKTISKAKGQPREPQVYTLPPSREEMTKNQVSLTCLVKGFYPSDIAVEWESNGQPENNYKTTPPVLDSDGSFFLYSKLTVDKSRWQQGNVFSCSVMHEALHNHYTQKSLSLSPGK

SEQ ID NO: 188 - protein, 695 aa, synthetic construct
QVQLVQSGAEVKKPGSSVKVSCKASGYTFTRNFIHWIRQAPGQGLEWIGWIFPGDGDTEYNQKFNGRATITADKSTSTAYMELSSLRSEDTAVYYCARGNYNYEYFDYWGQGTMVTVSSASTKGPSVFPLAPSSKSTSGGTAALGCLVKDYFPEPVTVSWNSGALTSGVHTFPAVLQSSGLYSLSSVVTVPSSSLGTQTYICNVNHKPSNTKVDKRVEPKSCGGGGSQVQLVQSGGGVVQPGRSLRLSCKASGYTFTRYTMHWVRQAPGKGLEWIGYINPSRGYTNYNQKVKDRFTISRDNSKNTAFLQMDSLRPEDTGVYFCARYYDDHYSLDYWGQGTPVTVSSGGGGSGGGGSGGGGSDIQMTQSPSSLSASVGDRVTITCSASSSVSYMNWYQQTPGKAPKRWIYNTSKLASGVPSRFSGSGSGTDYTFTISSLQPEDIATYYCQQWSSNPFTFGQGTKLQITRDKTHTCPPCPAPEAAGGPSVFLFPPKPKDTLMISRTPEVTCVVVDVSHEDPEVKFNWYVDGVEVHNAKTKPREEQYNSTYRVVSVLTVLHQDWLNGKEYKCKVSNKALPAPIEKTISKAKGQPREPQVYTLPPSREEMTKNQVSLTCLVKGFYPSDIAVEWESNGQPENNYKTTPPVLDSDGSFFLYSKLTVDKSRWQQGNVFSCSVMHEALHNHYTQKSLSLSPGK

SEQ ID NO: 189 - protein, 695 aa, synthetic construct
QVQLVQSGAEVKKPGSSVKVSCKASGYTFTRNFIHWIRQAPGQGLEWIGWIFPGDGDTEYNQKFNGRATITADKSTSTAYMELSSLRSEDTAVYYCARGNYNYEYFDYWGQGTMVTVSSASTKGPSVFPLAPSSKSTSGGTAALGCLVKDYFPEPVTVSWNSGALTSGVHTFPAVLQSSGLYSLSSVVTVPSSSLGTQTYICNVNHKPSNTKVDKRVEPKSCGGGGSQVQLVQSGGGVVQPGRSLRLSCKASGYTFTRYTMHWVRQAPGKGLEWIGYINPSRGYTNYNQKVKDRFTISRDNSKNTAFLQMDSLRPEDTGVYFCARYYNDHYSLDYWGQGTPVTVSSGGGGSGGGGSGGGGSDIQMTQSPSSLSASVGDRVTITCSASSSVSYMNWYQQTPGKAPKRWIYDTSKLASGVPSRFSGSGSGTDYTFTISSLQPEDIATYYCQQWSSNPFTFGQGTKLQITRDKTHTCPPCPAPEAAGGPSVFLFPPKPKDTLMISRTPEVTCVVVDVSHEDPEVKFNWYVDGVEVHNAKTKPREEQYNSTYRVVSVLTVLHQDWLNGKEYKCKVSNKALPAPIEKTISKAKGQPREPQVYTLPPSREEMTKNQVSLTCLVKGFYPSDIAVEWESNGQPENNYKTTPPVLDSDGSFFLYSKLTVDKSRWQQGNVFSCSVMHEALHNHYTQKSLSLSPGK

SEQ ID NO: 190 - protein, 695 aa, synthetic construct
QVQLVQSGAEVKKPGSSVKVSCKASGYTFTRNFIHWIRQAPGQGLEWIGWIFPGDGDTEYNQKFNGRATITADKSTSTAYMELSSLRSEDTAVYYCARGNYNYEYFDYWGQGTMVTVSSASTKGPSVFPLAPSSKSTSGGTAALGCLVKDYFPEPVTVSWNSGALTSGVHTFPAVLQSSGLYSLSSVVTVPSSSLGTQTYICNVNHKPSNTKVDKRVEPKSCGGGGSQVQLVQSGGGVVQPGRSLRLSCKASGYTFTRYTMHWVRQAPGKGLEWIGYINPSRGYTNYNQKVKDRFTISRDNSKNTAFLQMDSLRPEDTGVYFCARYYDDHFSLDYWGQGTPVTVSSGGGGSGGGGSGGGGSDIQMTQSPSSLSASVGDRVTITCSASSSVSYMNWYQQTPGKAPKRWIYDTSKLASGVPSRFSGSGSGTDYTFTISSLQPEDIATYYCQQWSSNPFTFGQGTKLQITRDKTHTCPPCPAPEAAGGPSVFLFPPKPKDTLMISRTPEVTCVVVDVSHEDPEVKFNWYVDGVEVHNAKTKPREEQYNSTYRVVSVLTVLHQDWLNGKEYKCKVSNKALPAPIEKTISKAKGQPREPQVYTLPPSREEMTKNQVSLTCLVKGFYPSDIAVEWESNGQPENNYKTTPPVLDSDGSFFLYSKLTVDKSRWQQGNVFSCSVMHEALHNHYTQKSLSLSPGK

SEQ ID NO: 191 - protein, 695 aa, synthetic construct
QVQLVQSGAEVKKPGSSVKVSCKASGYTFTRNFIHWIRQAPGQGLEWIGWIFPGDGDTEYNQKFNGRATITADKSTSTAYMELSSLRSEDTAVYYCARGNYNYEYFDYWGQGTMVTVSSASTKGPSVFPLAPSSKSTSGGTAALGCLVKDYFPEPVTVSWNSGALTSGVHTFPAVLQSSGLYSLSSVVTVPSSSLGTQTYICNVNHKPSNTKVDKRVEPKSCGGGGSQVQLVQSGGGVVQPGRSLRLSCKASGYTFTRYTMHWVRQAPGKGLEWIGYINPSMGATNYNQKVKDRFTISRDNSKNTAFLQMDSLRPEDTGVYFCARYYDDHYSLDYWGQGTPVTVSSGGGGSGGGGSGGGGSDIQMTQSPSSLSASVGDRVTITCSASSSVSYMNWYQQTPGKAPKRWIYDTSKLASGVPSRFSGSGSGTDYTFTISSLQPEDIATYYCQQWSSNPFTFGQGTKLQITRDKTHTCPPCPAPEAAGGPSVFLFPPKPKDTLMISRTPEVTCVVVDVSHEDPEVKFNWYVDGVEVHNAKTKPREEQYNSTYRVVSVLTVLHQDWLNGKEYKCKVSNKALPAPIEKTISKAKGQPREPQVYTLPPSREEMTKNQVSLTCLVKGFYPSDIAVEWESNGQPENNYKTTPPVLDSDGSFFLYSKLTVDKSRWQQGNVFSCSVMHEALHNHYTQKSLSLSPGK

SEQ ID NO: 192 - protein, 714 aa, synthetic construct
QVQLVQSGGGVVQPGRSLRLSCKASGYTFTRYTMHWVRQAPGKGLEWIGYINPSRGYTNYNQKVKDRFTISRDNSKNTAFLQMDSLRPEDTGVYFCARYYDDHYSLDYWGQGTPVTVSSGGGGSGGGGSGGGGSDIQMTQSPSSLSASVGDRVTITCSASSSVSYMNWYQQTPGKAPKRWIYDTSKLASGVPSRFSGSGSGTDYTFTISSLQPEDIATYYCQQWSSNPFTFGQGTKLQITRGGGGSDIQMTQSPSSLSASVGDRVTITCLASEDIYSYLAWYQQKPGKAPKLLIFAANRLQDGVPSRFSGSGSGTDFTLTISSLQPEDFATYYCLQGSKFPYTFGPGTKVDIKGGGGSGGGGSGGGGSQVQLVQSGAEVKKPGSSVKVSCKASGYTFTRNFIHWIRQAPGQGLEWIGWIFPGDADTEYNQKFSGRATITADKSTSTAYMELSSLRSEDTAVYYCARGNYNYEYFDYWGQGTMVTVSSDKTHTCPPCPAPEAAGGPSVFLFPPKPKDTLMISRTPEVTCVVVDVSHEDPEVKFNWYVDGVEVHNAKTKPREEQYNSTYRVVSVLTVLHQDWLNGKEYKCKVSNKALPAPIEKTISKAKGQPREPQVYTLPPSREEMTKNQVSLTCLVKGFYPSDIAVEWESNGQPENNYKTTPPVLDSDGSFFLYSKLTVDKSRWQQGNVFSCSVMHEALHNHYTQKSLSLSPGK

SEQ ID NO: 193 - protein, 449 aa, synthetic construct
QVQLVQSGAEVKKPGSSVKVSCKASGYTFTRNFIHWIRQAPGQGLEWIGWIFPGDADTEYNQKFSGRATITADKSTSTAYMELSSLRSEDTAVYYCARGNYNYEYFDYWGQGTMVTVSSASTKGPSVFPLAPSSKSTSGGTAALGCLVKDYFPEPVTVSWNSGALTSGVHTFPAVLQSSGLYSLSSVVTVPSSSLGTQTYICNVNHKPSNTKVDKRVEPKSCDKTHTCPPCPAPEAAGGPSVFLFPPKPKDTLMISRTPEVTCVVVDVSHEDPEVKFNWYVDGVEVHNAKTKPREEQYNSTYRVVSVLTVLHQDWLNGKEYKCKVSNKALPAPIEKTISKAKGQPREPQVYTLPPSREEMTKNQVSLTCLVKGFYPSDIAVEWESNGQPENNYKTTPPVLDSDGSFFLYSKLTVDKSRWQQGNVFSCSVMHEALHNHYTQKSLSLSPGK

SEQ ID NO: 194 - protein, 449 aa, synthetic construct
QVQLVQSGAEVKKPGSSVKVSCKASGYTFTRNFIHWIRQAPGQGLEWIGWIFPGDADTEYNQKFSGRVTITADKSTSTAYMELSSLRSEDTAVYYCARGNYNYEYFDYWGQGTMVTVSSASTKGPSVFPLAPSSKSTSGGTAALGCLVKDYFPEPVTVSWNSGALTSGVHTFPAVLQSSGLYSLSSVVTVPSSSLGTQTYICNVNHKPSNTKVDKRVEPKSCDKTHTCPPCPAPEAAGGPSVFLFPPKPKDTLMISRTPEVTCVVVDVSHEDPEVKFNWYVDGVEVHNAKTKPREEQYNSTYRVVSVLTVLHQDWLNGKEYKCKVSNKALPAPIEKTISKAKGQPREPQVYTLPPSREEMTKNQVSLTCLVKGFYPSDIAVEWESNGQPENNYKTTPPVLDSDGSFFLYSKLTVDKSRWQQGNVFSCSVMHEALHNHYTQKSLSLSPGK

SEQ ID NO: 195 - protein, 695 aa, synthetic construct
QVQLVQSGAEVKKPGSSVKVSCKASGYTFTRNFIHWIRQAPGQGLEWIGWIFPGDADTEYNQKFSGRATITADKSTSTAYMELSSLRSEDTAVYYCARGNYNYEYFDYWGQGTMVTVSSASTKGPSVFPLAPSSKSTSGGTAALGCLVKDYFPEPVTVSWNSGALTSGVHTFPAVLQSSGLYSLSSVVTVPSSSLGTQTYICNVNHKPSNTKVDKRVEPKSCGGGGSQVQLVQSGGGVVQPGRSLRLSCKASGYTFTRYTMHWVRQAPGKGLEWIGYINPSRGYTNYNQKVKDRFTISRDNSKNTAFLQMDSLRPEDTGVYFCARYYDDHYSLDYWGQGTPVTVSSGGGGSGGGGSGGGGSDIQMTQSPSSLSASVGDRVTITCSASSSVSYMNWYQQTPGKAPKRWIYDTSKLASGVPSRFSGSGSGTDYTFTISSLQPEDIATYYCQQWSSNPFTFGQGTKLQITRDKTHTCPPCPAPEAAGGPSVFLFPPKPKDTLMISRTPEVTCVVVDVSHEDPEVKFNWYVDGVEVHNAKTKPREEQYNSTYRVVSVLTVLHQDWLNGKEYKCKVSNKALPAPIEKTISKAKGQPREPQVYTLPPCREEMTKNQVSLWCLVKGFYPSDIAVEWESNGQPENNYKTTPPVLDSDGSFFLYSKLTVDKSRWQQGNVFSCSVMHEALHNHYTQKSLSLSPGK

SEQ ID NO: 196 - protein, 705 aa, synthetic construct
QVQLVQSGAEVKKPGSSVKVSCKASGYTFTRNFIHWIRQAPGQGLEWIGWIFPGDADTEYNQKFSGRATITADKSTSTAYMELSSLRSEDTAVYYCARGNYNYEYFDYWGQGTMVTVSSASTKGPSVFPLAPSSKSTSGGTAALGCLVKDYFPEPVTVSWNSGALTSGVHTFPAVLQSSGLYSLSSVVTVPSSSLGTQTYICNVNHKPSNTKVDKRVEPKSCGGGGSQVQLVQSGGGVVQPGRSLRLSCKASGYTFTRYTMHWVRQAPGKGLEWIGYINPSRGYTNYNQKVKDRFTISRDNSKNTAFLQMDSLRPEDTGVYFCARYYDDHYSLDYWGQGTPVTVSSGGGGSGGGGSGGGGSDIQMTQSPSSLSASVGDRVTITCSASSSVSYMNWYQQTPGKAPKRWIYDTSKLASGVPSRFSGSGSGTDYTFTISSLQPEDIATYYCQQWSSNPFTFGQGTKLQITRGGGGSGGGGSDKTHTCPPCPAPEAAGGPSVFLFPPKPKDTLMISRTPEVTCVVVDVSHEDPEVKFNWYVDGVEVHNAKTKPREEQYNSTYRVVSVLTVLHQDWLNGKEYKCKVSNKALPAPIEKTISKAKGQPREPQVYTLPPCREEMTKNQVSLWCLVKGFYPSDIAVEWESNGQPENNYKTTPPVLDSDGSFFLYSKLTVDKSRWQQGNVFSCSVMHEALHNHYTQKSLSLSPGK

SEQ ID NO: 197 - protein, 700 aa, synthetic construct
QVQLVQSGAEVKKPGSSVKVSCKASGYTFTRNFIHWIRQAPGQGLEWIGWIFPGDADTEYNQKFSGRATITADKSTSTAYMELSSLRSEDTAVYYCARGNYNYEYFDYWGQGTMVTVSSASTKGPSVFPLAPSSKSTSGGTAALGCLVKDYFPEPVTVSWNSGALTSGVHTFPAVLQSSGLYSLSSVVTVPSSSLGTQTYICNVNHKPSNTKVDKRVEPKSCGGGGSQVQLVQSGGGVVQPGRSLRLSCKASGYTFTRYTMHWVRQAPGKGLEWIGYINPSRGYTNYNQKVKDRFTISRDNSKNTAFLQMDSLRPEDTGVYFCARYYDDHYSLDYWGQGTPVTVSSGGGGSGGGGSGGGGSDIQMTQSPSSLSASVGDRVTITCSASSSVSYMNWYQQTPGKAPKRWIYDTSKLASGVPSRFSGSGSGTDYTFTISSLQPEDIATYYCQQWSSNPFTFGQGTKLQITREPKSVDKTHTCPPCPAPEAAGGPSVFLFPPKPKDTLMISRTPEVTCVVVDVSHEDPEVKFNWYVDGVEVHNAKTKPREEQYNSTYRVVSVLTVLHQDWLNGKEYKCKVSNKALPAPIEKTISKAKGQPREPQVYTLPPCREEMTKNQVSLWCLVKGFYPSDIAVEWESNGQPENNYKTTPPVLDSDGSFFLYSKLTVDKSRWQQGNVFSCSVMHEALHNHYTQKSLSLSPGK

SEQ ID NO: 198 - protein, 474 aa, synthetic construct
QVQLVQSGAEVKKPGSSVKVSCKASGYTFTRNFIHWIRQAPGQGLEWIGWIFPGDADTEYNQKFSGRATITADKSTSTAYMELSSLRSEDTAVYYCARGNYNYEYFDYWGQGTMVTVSSASTKGPSVFPLAPSSKSTSGGTAALGCLVKDYFPEPVTVSWNSGALTSGVHTFPAVLQSSGLYSLSSVVTVPSSSLGTQTYICNVNHKPSNTKVDKRVEPKSCGGGGSQVQLVQSGGGVVQPGRSLRLSCKASGYTFTRYTMHWVRQAPGKGLEWIGYINPSRGYTNYNQKVKDRFTISRDNSKNTAFLQMDSLRPEDTGVYFCARYYDDHYSLDYWGQGTPVTVSSGGGGSGGGGSGGGGSDIQMTQSPSSLSASVGDRVTITCSASSSVSYMNWYQQTPGKAPKRWIYDTSKLASGVPSRFSGSGSGTDYTFTISSLQPEDIATYYCQQWSSNPFTFGQGTKLQITRHHHHHH

SEQ ID NO: 199 - protein, 449 aa, synthetic construct
QVQLVQSGAEVKKPGSSVKVSCKASGYTFTRNFIHWIRQAPGQGLEWIGWIFPGDADTEYNQKFSGRATITADKSTSTAYMELSSLRSEDTAVYYCARGNYNYEYFDYWGQGTMVTVSSASTKGPSVFPLAPSSKSTSGGTAALGCLVKDYFPEPVTVSWNSGALTSGVHTFPAVLQSSGLYSLSSVVTVPSSSLGTQTYICNVNHKPSNTKVDKRVEPKSCDKTHTCPPCPAPEAAGGPSVFLFPPKPKDTLMISRTPEVTCVVVDVSHEDPEVKFNWYVDGVEVHNAKTKPREEQYNSTYRVVSVLTVLHQDWLNGKEYKCKVSNKALPAPIEKTISKAKGQPREPQVYTLPPCREEMTKNQVSLWCLVKGFYPSDIAVEWESNGQPENNYKTTPPVLDSDGSFFLYSKLTVDKSRWQQGNVFSCSVMHEALHNHYTQKSLSLSPGK

SEQ ID NO: 200 - protein, 483 aa, synthetic construct
DIQMTQSPSSLSASVGDRVTITCLASEDIYSYLAWYQQKPGKAPKLLIFAANRLQSGVPSRFSGSGSGTDFTLTISSLQPEDFATYYCLQGSKFPYTFGPGTKVDIKGGGGSGGGGSGGGGSQVQLVQSGAEVKKPGSSVKVSCKASGYTFTRNFIHWIRQAPGQGLEWIGWIFPGDADTEYNQKFSGRATITADKSTSTAYMELSSLRSEDTAVYYCARGNYNYEYFDYWGQGTMVTVSSGGGGSGGGGSGGGGSDKTHTCPPCPAPEAAGGPSVFLFPPKPKDTLMISRTPEVTCVVVDVSHEDPEVKFNWYVDGVEVHNAKTKPREEQYNSTYRVVSVLTVLHQDWLNGKEYKCKVSNKALPAPIEKTISKAKGQPREPQVCTLPPSREEMTKNQVSLSCAVKGFYPSDIAVEWESNGQPENNYKTTPPVLDSDGSFFLVSKLTVDKSRWQQGNVFSCSVMHEALHNHYTQKSLSLSPGK

SEQ ID NO: 201 - protein, 214 aa, synthetic construct
DIQMTQSPSSLSASVGDRVTITCLASEDIYSYLAWYQQKPGKAPKLLIFAANRLQDGVPSRFSGSGSGTDFTLTISSLQPEDFATYYCLQGSKFPYTFGPGTKVDIKRTVAAPSVFIFPPSDEQLKSGTASVVCLLNNFYPREAKVQWKVDNALQSGNSQESVTEQDSKDSTYSLSSTLTLSKADYEKHKVYACEVTHQGLSSPVTKSFNRGEC

SEQ ID NO: 202 - protein, 214 aa, synthetic construct
DIQMTQSPSSLSASVGDRVTITCLASEDIYSYLAWYQQKPGKAPKLLIFAANRLQSGVPSRFSGSGSGTDFTLTISSLQPEDFATYYCLQGSKFPYTFGPGTKVDIKRTVAAPSVFIFPPSDEQLKSGTASVVCLLNNFYPREAKVQWKVDNALQSGNSQESVTEQDSKDSTYSLSSTLTLSKADYEKHKVYACEVTHQGLSSPVTKSFNRGEC

SEQ ID NO: 203 - protein, 465 aa, synthetic construct
DIQMTQSPSSLSASVGDRVTITCLASEDIYSYLAWYQQKPGKAPKLLIFAANRLQSGVPSRFSGSGSGTDFTLTISSLQPEDFATYYCLQGSKFPYTFGPGTKVDIKRTVAAPSVFIFPPSDEQLKSGTASVVCLLNNFYPREAKVQWKVDNALQSGNSQESVTEQDSKDSTYSLSSTLTLSKADYEKHKVYACEVTHQGLSSPVTKSFNRGECGGGGSGGGGSQVQLVQSGGGVVQPGRSLRLSCKASGYTFTRYTMHWVRQAPGKGLEWIGYINPSRGYTNYNQKVKDRFTISRDNSKNTAFLQMDSLRPEDTGVYFCARYYDDHYSLDYWGQGTPVTVSSGGGGSGGGGSGGGGSDIQMTQSPSSLSASVGDRVTITCSASSSVSYMNWYQQTPGKAPKRWIYDTSKLASGVPSRFSGSGSGTDYTFTISSLQPEDIATYYCQQWSSNPFTFGQGTKLQITR

SEQ ID NO: 204 - protein, 227 aa, synthetic construct
DKTHTCPPCPAPEAAGGPSVFLFPPKPKDTLMISRTPEVTCVVVDVSHEDPEVKFNWYVDGVEVHNAKTKPREEQYNSTYRVVSVLTVLHQDWLNGKEYKCKVSNKALPAPIEKTISKAKGQPREPQVCTLPPSREEMTKNQVSLSCAVKGFYPSDIAVEWESNGQPENNYKTTPPVLDSDGSFFLVSKLTVDKSRWQQGNVFSCSVMHEALHNHYTQKSLSLSPGK

SEQ ID NO: 205 - protein, 483 aa, synthetic construct
QVQLVQSGGGVVQPGRSLRLSCKASGYTFTRYTMHWVRQAPGKGLEWIGYINPSRGYTNYNQKVKDRFTISRDNSKNTAFLQMDSLRPEDTGVYFCARYYDDHYSLDYWGQGTPVTVSSGGGGSGGGGSGGGGSDIQMTQSPSSLSASVGDRVTITCSASSSVSYMNWYQQTPGKAPKRWIYDTSKLASGVPSRFSGSGSGTDYTFTISSLQPEDIATYYCQQWSSNPFTFGQGTKLQITRGGGGSGGGGSGGGGSDKTHTCPPCPAPEAAGGPSVFLFPPKPKDTLMISRTPEVTCVVVDVSHEDPEVKFNWYVDGVEVHNAKTKPREEQYNSTYRVVSVLTVLHQDWLNGKEYKCKVSNKALPAPIEKTISKAKGQPREPQVYTLPPCREEMTKNQVSLWCLVKGFYPSDIAVEWESNGQPENNYKTTPPVLDSDGSFFLYSKLTVDKSRWQQGNVFSCSVMHEALHNHYTQKSLSLSPGK

SEQ ID NO: 206 - protein, 465 aa, synthetic construct
DIQMTQSPSSLSASVGDRVTITCLASEDIYSYLAWYQQKPGKAPKLLIFAANRLQDGVPSRFSGSGSGTDFTLTISSLQPEDFATYYCLQGSKFPYTFGPGTKVDIKRTVAAPSVFIFPPSDEQLKSGTASVVCLLNNFYPREAKVQWKVDNALQSGNSQESVTEQDSKDSTYSLSSTLTLSKADYEKHKVYACEVTHQGLSSPVTKSFNRGECGGGGSGGGGSQVQLVQSGGGVVQPGRSLRLSCKASGYTFTRYTMHWVRQAPGKGLEWIGYINPSRGYTNYNQKVKDRFTISRDNSKNTAFLQMDSLRPEDTGVYFCARYYDDHYSLDYWGQGTPVTVSSGGGGSGGGGSGGGGSDIQMTQSPSSLSASVGDRVTITCSASSSVSYMNWYQQTPGKAPKRWIYDTSKLASGVPSRFSGSGSGTDYTFTISSLQPEDIATYYCQQWSSNPFTFGQGTKLQITR

SEQ ID NO: 207 - protein, 468 aa, synthetic construct
DIQMTQSPSSLSASVGDRVTITCLASEDIYSYLAWYQQKPGKAPKLLIFAANRLQDGVPSRFSGSGSGTDFTLTISSLQPEDFATYYCLQGSKFPYTFGPGTKVDIKGGGGSGGGGSGGGGSQVQLVQSGAEVKKPGSSVKVSCKASGYTFTRNFIHWIRQAPGQGLEWIGWIFPGDADTEYNQKFSGRATITADKSTSTAYMELSSLRSEDTAVYYCARGNYNYEYFDYWGQGTMVTVSSDKTHTCPPCPAPEAAGGPSVFLFPPKPKDTLMISRTPEVTCVVVDVSHEDPEVKFNWYVDGVEVHNAKTKPREEQYNSTYRVVSVLTVLHQDWLNGKEYKCKVSNKALPAPIEKTISKAKGQPREPQVCTLPPSREEMTKNQVSLSCAVKGFYPSDIAVEWESNGQPENNYKTTPPVLDSDGSFFLVSKLTVDKSRWQQGNVFSCSVMHEALHNHYTQKSLSLSPGK

SEQ ID NO: 208 - protein, 119 aa, synthetic construct
QVQLVQSGGGVVQPGRSLRLSCKASGYTFTRYTMHWVRQAPGKGLEWIGYINPSRGYTNYNQKVKDRFTISRDNSKNTAFLQMDSLRPEDTGVYFCARYYNDHYSLDYWGQGTPVTVSS

SEQ ID NO: 209 - protein, 119 aa, synthetic construct
QVQLVQSGGGVVQPGRSLRLSCKASGYTFTRYTMHWVRQAPGKGLEWIGYINPSRGYTNYNQKVKDRFTISRDNSKNTAFLQMDSLRPEDTGVYFCARYYDDHFSLDYWGQGTPVTVSS

SEQ ID NO: 210 - protein, 119 aa, synthetic construct
QVQLVQSGGGVVQPGRSLRLSCKASGYTFTRYTMHWVRQAPGKGLEWIGYINPSMGATNYNQKVKDRFTISRDNSKNTAFLQMDSLRPEDTGVYFCARYYDDHYSLDYWGQGTPVTVSS

SEQ ID NO: 211 - protein, 107 aa, synthetic construct
DIQMTQSPSSLSASVGDRVTITCSASSSVAYMNWYQQTPGKAPKRWIYDTSKLASGVPSRFSGSGSGTDYTFTISSLQPEDIATYYCQQWSSNPFTFGQGTKLQITR

SEQ ID NO: 212 - protein, 107 aa, synthetic construct
DIQMTQSPSSLSASVGDRVTITCSASSSVSYMNWYQQTPGKAPKRWIYNTSKLASGVPSRFSGSGSGTDYTFTISSLQPEDIATYYCQQWSSNPFTFGQGTKLQITR

SEQ ID NO: 213 - protein, 217 aa, synthetic construct
APEAAGGPSVFLFPPKPKDTLMISRTPEVTCVVVDVSHEDPEVKFNWYVDGVEVHNAKTKPREEQYNSTYRVVSVLTVLHQDWLNGKEYKCKVSNKALPAPIEKTISKAKGQPREPQVCTLPPSREEMTKNQVSLSCAVKGFYPSDIAVEWESNGQPENNYKTTPPVLDSDGSFFLVSKLTVDKSRWQQGNVFSCSVMHEALHNHYTQKSLSLSPGK

SEQ ID NO: 214 - protein, 217 aa, synthetic construct
APEAAGGPSVFLFPPKPKDTLMISRTPEVTCVVVDVSHEDPEVKFNWYVDGVEVHNAKTKPREEQYNSTYRVVSVLTVLHQDWLNGKEYKCKVSNKALPAPIEKTISKAKGQPREPQVYTLPPCREEMTKNQVSLWCLVKGFYPSDIAVEWESNGQPENNYKTTPPVLDSDGSFFLYSKLTVDKSRWQQGNVFSCSVMHEALHNHYTQKSLSLSPGK

SEQ ID NO: 215 - protein, 217 aa, synthetic construct
APEAAGGPSVFLFPPKPKDTLMISRTPEVTCVVVDVSHEDPEVKFNWYVDGVEVHNAKTKPREEQYNSTYRVVSVLTVLHQDWLNGKEYKCKVSNKALPAPIEKTISKAKGQPREPQVYTLPPSREEMTKNQVSLTCLVKGFYPSDIAVEWESNGQPENNYKTTPPVLDSDGSFFLYSKLTVDKSRWQQGNVFSCSVMHEALHNHYTQKSLSLSPGK

SEQ ID NO: 216 - protein, 695 aa, synthetic construct
QVQLVQSGAEVKKPGSSVKVSCKASGYTFTRNFIHWIRQAPGQGLEWIGWIFPGDADTEYNQKFSGRVTITADKSTSTAYMELSSLRSEDTAVYYCARGNYNYEYFDYWGQGTMVTVSSASTKGPSVFPLAPSSKSTSGGTAALGCLVKDYFPEPVTVSWNSGALTSGVHTFPAVLQSSGLYSLSSVVTVPSSSLGTQTYICNVNHKPSNTKVDKRVEPKSCGGGGSQVQLVQSGGGVVQPGRSLRLSCKASGYTFTRYTMHWVRQAPGKGLEWIGYINPSRGYTNYNQKVKDRFTISRDNSKNTAFLQMDSLRPEDTGVYFCARYYDDHYSLDYWGQGTPVTVSSGGGGSGGGGSGGGGSDIQMTQSPSSLSASVGDRVTITCSASSSVSYMNWYQQTPGKAPKRWIYDTSKLASGVPSRFSGSGSGTDYTFTISSLQPEDIATYYCQQWSSNPFTFGQGTKLQITRDKTHTCPPCPAPEAAGGPSVFLFPPKPKDTLMISRTPEVTCVVVDVSHEDPEVKFNWYVDGVEVHNAKTKPREEQYNSTYRVVSVLTVLHQDWLNGKEYKCKVSNKALPAPIEKTISKAKGQPREPQVYTLPPCREEMTKNQVSLWCLVKGFYPSDIAVEWESNGQPENNYKTTPPVLDSDGSFFLYSKLTVDKSRWQQGNVFSCSVMHEALHNHYTQKSLSLSPGK

SEQ ID NO: 217 - protein, 122 aa, synthetic construct [sequence omitted]

SEQ ID NO: 218 - protein, 107 aa, synthetic construct [sequence omitted]

SEQ ID NO: 219 - protein, 5 aa, Mus musculus
GYTMN

SEQ ID NO: 220 - protein, 17 aa, Mus musculus
LINPYKGVSTYNQKFKD

SEQ ID NO: 221 - protein, 13 aa, Mus musculus
SGYYGDSDWYFDV

SEQ ID NO: 222 - protein, 11 aa, Mus musculus
RASQDIRNYLN

SEQ ID NO: 223 - protein, 7 aa, Mus musculus
YTSRLES

SEQ ID NO: 224 - protein, 9 aa, Mus musculus
QQGNTLPWT

SEQ ID NO: 225 - protein, 698 aa, synthetic construct
QVQLVQSGAEVKKPGSSVKVSCKASGYTFTRNFIHWIRQAPGQGLEWIGWIFPGDADTEYNQKFSGRVTITADKSTSTAYMELSSLRSEDTAVYYCARGNYNYEYFDYWGQGTMVTVSSASTKGPSVFPLAPSSKSTSGGTAALGCLVKDYFPEPVTVSWNSGALTSGVHTFPAVLQSSGLYSLSSVVTVPSSSLGTQTYICNVNHKPSNTKVDKRVEPKSCGGGGSEVQLVESGGGLVQPGGSLRLSCAASGYSFTGYTMNWVRQAPGKGLEWVALINPYKGVSTYNQKFKDRFTISVDKSKNTAYLQMNSLRAEDTAVYYCARSGYYGDSDWYFDVWGQGTLVTVSSGGGGSGGGGSGGGGSDIQMTQSPSSLSASVGDRVTITCRASQDIRNYLNWYQQKPGKAPKLLIYYTSRLESGVPSRFSGSGSGTDYTLTISSLQPEDFATYYCQQGNTLPWTFGQGTKVEIKDKTHTCPPCPAPEAAGGPSVFLFPPKPKDTLMISRTPEVTCVVVDVSHEDPEVKFNWYVDGVEVHNAKTKPREEQYNSTYRVVSVLTVLHQDWLNGKEYKCKVSNKALPAPIEKTISKAKGQPREPQVYTLPPSREEMTKNQVSLTCLVKGFYPSDIAVEWESNGQPENNYKTTPPVLDSDGSFFLYSKLTVDKSRWQQGNVFSCSVMHEALHNHYTQKSLSLSPGK

SEQ ID NO: 226 - protein, 717 aa, synthetic construct
EVQLVESGGGLVQPGGSLRLSCAASGYSFTGYTMNWVRQAPGKGLEWVALINPYKGVSTYNQKFKDRFTISVDKSKNTAYLQMNSLRAEDTAVYYCARSGYYGDSDWYFDVWGQGTLVTVSSGGGGSGGGGSGGGGSDIQMTQSPSSLSASVGDRVTITCRASQDIRNYLNWYQQKPGKAPKLLIYYTSRLESGVPSRFSGSGSGTDYTLTISSLQPEDFATYYCQQGNTLPWTFGQGTKVEIKGGGGSDIQMTQSPSSLSASVGDRVTITCLASEDIYSYLAWYQQKPGKAPKLLIFAANRLQSGVPSRFSGSGSGTDFTLTISSLQPEDFATYYCLQGSKFPYTFGPGTKVDIKGGGGSGGGGSGGGGSQVQLVQSGAEVKKPGSSVKVSCKASGYTFTRNFIHWIRQAPGQGLEWIGWIFPGDADTEYNQKFSGRVTITADKSTSTAYMELSSLRSEDTAVYYCARGNYNYEYFDYWGQGTMVTVSSDKTHTCPPCPAPEAAGGPSVFLFPPKPKDTLMISRTPEVTCVVVDVSHEDPEVKFNWYVDGVEVHNAKTKPREEQYNSTYRVVSVLTVLHQDWLNGKEYKCKVSNKALPAPIEKTISKAKGQPREPQVYTLPPSREEMTKNQVSLTCLVKGFYPSDIAVEWESNGQPENNYKTTPPVLDSDGSFFLYSKLTVDKSRWQQGNVFSCSVMHEALHNHYTQKSLSLSPGK

SEQ ID NO: 227 - protein, 449 aa, synthetic construct; identical to SEQ ID NO: 194

SEQ ID NO: 228 - protein, 463 aa, synthetic construct
EVQLVESGGGLVQPGGSLRLSCAASGYSFTGYTMNWVRQAPGKGLEWVALINPYKGVSTYNQKFKDRFTISVDKSKNTAYLQMNSLRAEDTAVYYCARSGYYGDSDWYFDVWGQGTLVTVSSGGGGSGGGGSGGGGSDIQMTQSPSSLSASVGDRVTITCRASQDIRNYLNWYQQKPGKAPKLLIYYTSRLESGVPSRFSGSGSGTDYTLTISSLQPEDFATYYCQQGNTLPWTFGQGTKVEIKGGGGSDIQMTQSPSSLSASVGDRVTITCLASEDIYSYLAWYQQKPGKAPKLLIFAANRLQSGVPSRFSGSGSGTDFTLTISSLQPEDFATYYCLQGSKFPYTFGPGTKVDIKRTVAAPSVFIFPPSDEQLKSGTASVVCLLNNFYPREAKVQWKVDNALQSGNSQESVTEQDSKDSTYSLSSTLTLSKADYEKHKVYACEVTHQGLSSPVTKSFNRGEC